European Patent Specification EP 3 303 573 B1, published April 1, 2026. Title: BIOSYNTHESIS OF PHENYLPROPANOID AND DIHYDROPHENYLPROPANOID DERIVATIVES. Applicant: EVOLVA SA Naesby, Michael Simon Vecilla, Ernesto Eichenberger, Michael Lehka, Beata Joanna Bjorn-Yoshimoto, Walden Emil Jensen, Niels Bjerg Dyekjaer, Jane Dannow. The sequence listing filed with the application follows.

SEQUENCE LISTING (109 sequences)

SEQ ID NO: 1 - DNA, 2154 bp, Arabidopsis thaliana
atggaccaaattgaagcaatgctatgcggtggtggtgaaaagaccaaggtggccgtaacgacaaaaactcttgcagatcctttgaattggggtctggcagctgaccagatgaaaggtagccatctggatgaagttaagaagatggttgaggaatacagaagaccagtcgtaaatctaggcggcgagacattgacgataggacaggtagctgctatttcgaccgttggcggttcagtgaaggtagaacttgcagaaacaagtagagccggagttaaggcttcatcagattgggtcatggaaagtatgaacaagggcacagattcctatggcgttaccacaggctttggtgctacctctcatagaagaactaaaaatggcactgctttgcaaacagaactgatcagattccttaacgccggtattttcggtaatacaaaggaaacttgccatacattaccccaatcggcaacaagagctgctatgcttgttagggtgaacactttgttgcaaggttactctggaataaggtttgaaattcttgaggccatcacttcactattgaaccacaacatttctccttcgttgcccttaagaggaacaataactgccagcggtgatttggttcccctttcatatatcgcaggcttattaacgggaagacctaattcaaaggccactggtccagacggagaatccttaaccgctaaggaagcatttgagaaagctggtatttcaactggtttctttgatttgcaacccaaggaaggtttagccctggtgaatggcaccgctgtcggcagcggtatggcatccatggtgttgtttgaagctaacgtacaagcagttttggccgaagttttgtccgcaatttttgccgaagtcatgagtggaaaacctgagtttactgatcacttgacccacaggttaaaacatcacccaggacaaattgaagcagcagctatcatggagcacattttggacggctctagctacatgaagttagcccagaaggttcatgaaatggaccctttgcaaaaacccaaacaagatagatatgctttaaggacatccccacaatggcttggccctcaaattgaagtaattagacaagctacaaagtctatagaaagagagatcaactctgttaacgataatccacttattgatgtgtcgaggaataaggcaatacatggaggcaatttccagggtacacccataggagtcagtatggataataccaggcttgccatagccgcaattggcaaattaatgtttgcccaattttctgaattggtcaatgacttctacaataacggtttgccttcgaatctgaccgcatcttctaaccctagtcttgattatggtttcaaaggtgctgagatagcaatggcaagctattgttcagagctgcaatatctagccaacccagtaacctctcatgtacaatcagccgaacaacacaatcaggatgttaattctttgggcctgatttcatcaagaaaaacaagcgaggccgttgatatccttaaattaatgtccacaacatttttagtgggtatatgccaggccgtagatttgagacacttggaagagaatttgagacagacagtgaaaaataccgtatcacaggttgcaaaaaaggttctaactacaggtatcaatggtgaattgcacccatcaagattctgtgaaaaagatttattaaaagttgtagatagagaacaagtatttacttacgttgacgatccatgtagcgctacttatccattgatgcagagattgagacaagttattgtagatcacgctttatccaatggtgaaactgagaaaaatgccgttacttcaatattccaaaagataggtgcctttgaagaagaactgaaggcagttttaccaaaggaagtcgaagctgctagagccgcatacggaaatggtactgcccctataccaaatagaatcaaagagtgtaggtcgtaccctttgtacagattcgttagagaagagttgggaaccaaattactaactggtgaaaaagtcgttagcccaggtgaagaatttgacaaggtattcacagctatgtgcgagggaaagttgatagatccacttatggattgcttgaaagagtggaatggtgcacctattccaatctgctaa

SEQ ID NO: 2 - DNA, 1521 bp, Ammi majus
atgatggattttgttttgttagaaaaagctcttcttggtttgttcattgcaactatagtagccatcacaatctctaagctaaggggaaagaaacttaagttgcctccaggcccaatccctgtcccagtgtttggtaattggttacaagttggcgacgacttaaaccagaggaatttggtagagtatgctaaaaagttcggcgacttatttctacttaggatgggtcaaagaaacttggtcgtggtttcatcccctgacttagcaaaagacgtactacatacccagggtgtcgagttcggaagtagaactagaaatgttgtgtttgatattttcacaggcaaaggtcaagatatggtttttaccgtatacagcgagcactggaggaaaatgagaagaataatgactgtcccattctttacaaacaaagtggttcaacagtataggttcggatgggaggacgaagccgctagagtagtcgaggatgttaaggcaaatcctgaagccgctaccaacggtattgtgttgaggaatagattacaacttttgatgtacaacaatatgtatagaataatgtttgacaggagatttgaatctgttgatgatccattattcctaaaacttaaggcattgaatggcgagagatcaaggttagctcaatcctttgaatacaacttcggtgacttcattcctatattgaggccattcttgagaggatatcttaagttgtgtcaggaaatcaaggacaaaaggttaaagctattcaaggactacttcgtcgacgagagaaaaaagttggagagtatcaagagcgtaggtaataactccttaaagtgcgccatagatcatattatcgaggcacaagaaaaaggcgagataaacgaggataacgtgttatacatcgtcgagaatatcaacgtggctgccattgaaactacactttggtctattgaatggggtatagcagaactagtgaataaccctgaaatccagaaaaaattgagacacgaattagacaccgtacttggagctggtgttcaaatttgtgaaccagatgttcaaaaattgccttatctacaggccgtgataaaagagactttaaggtacaggatggcaattccattgttagtcccacatatgaatcttcacgaagccaaattggccggctatgatatccctgcagagagcaaaattttggtaaacgcttggtggttagccaataatccagcacattggaacaaacctgatgagtttagaccagaaagatttttggaggaagaatccaaggtcgaggctaatggaaacgactttaagtacatccctttcggtgttggcagaagatcttgcccaggtataattcttgctttaccaatccttggaatagtaattggtaggttggttcaaaacttcgagttacttccacctccaggccaaagcaaaatagatacagccgaaaaaggtggacagttttcattgcaaatcctaaagcattccactattgtgtgtaaacctagaagttcttaa

SEQ ID NO: 3 - DNA, 1671 bp, Arabidopsis thaliana
atgacgacacaagatgtgatagtcaatgatcagaatgatcagaaacagtgtagtaatgacgtcattttccgatcgagattgcctgatatatacatccctaaccacctcccactccacgactacatcttcgaaaatatctcagagttcgccgctaagccatgcttgatcaacggtcccaccggcgaagtatacacctacgccgatgtccacgtaacatctcggaaactcgccgccggtcttcataacctcggcgtgaagcaacacgacgttgtaatgatcctcctcccgaactctcctgaagtagtcctcactttccttgccgcctccttcatcggcgcaatcaccacctccgcgaacccgttcttcactccggcggagatttctaaacaagccaaagcctccgcggcgaaactcatcgtcactcaatcccgttacgtcgataaaatcaagaacctccaaaacgacggcgttttgatcgtcaccaccgactccgacgccatccccgaaaactgcctccgtttctccgagttaactcagtccgaagaaccacgagtggactcaataccggagaagatttcgccagaagacgtcgtggcgcttcctttctcatccggcacgacgggtctccccaaaggagtgatgctaacacacaaaggtctagtcacgagcgtggcgcagcaagtcgacggcgagaatccgaatctttacttcaacagagacgacgtgatcctctgtgtcttgcctatgttccatatatacgctctcaactccatcatgctctgtagtctcagagttggtgccacgatcttgataatgcctaagttcgaaatcactctcttgttagagcagatacaaaggtgtaaagtcacggtggctatggtcgtgccaccgatcgttttagctatcgcgaagtcgccggagacggagaagtatgatctgagctcggttaggatggttaagtctggagcagctcctcttggtaaggagcttgaagatgctattagtgctaagtttcctaacgccaagcttggtcagggctatgggatgacagaagcaggtccggtgctagcaatgtcgttagggtttgctaaagagccgtttccagtgaagtcaggagcatgtggtacggtggtgaggaacgccgagatgaagatacttgatccagacacaggagattctttgcctaggaacaaacccggcgaaatatgcatccgtggcaaccaaatcatgaaaggctatctcaatgaccccttggccacggcatcgacgatcgataaagatggttggcttcacactggagacgtcggatttatcgatgatgacgacgagcttttcattgtggatagattgaaagaactcatcaagtacaaaggatttcaagtggctccagctgagctagagtctctcctcataggtcatccagaaatcaatgatgttgctgtcgtcgccatgaaggaagaagatgctggtgaggttcctgttgcgtttgtggtgagatcgaaagattcaaatatatccgaagatgaaatcaagcaattcgtgtcaaaacaggttgtgttttataagagaatcaacaaagtgttcttcactgactctattcctaaagctccatcagggaagatattgaggaaggatctaagagcaagactagcaaatggattaatgaactag

SEQ ID NO: 4 - DNA, 1200 bp, Hordeum vulgare
atggctgcagtaagattgaaagaagttagaatggcacagagggctgaaggtttagctacagttttagcaatcggtactgccgttccagctaattgtgtttatcaagctacctatccagattattattttagggttactaaaagtgagcacttggcagatttaaaggagaagtttcaaagaatgtgtgacaaatcaatgattagaaagagacacatgcacttgaccgaggaaatattgatcaagaacccaaagatctgtgcacacatggagacctcattggatgctagacacgccatcgcattagttgaagttcccaaattgggccaaggtgcagctgagaaggccattaaggagtggggccaacccttgtctaagattactcatttggtattttgcacaacatccggcgttgacatgcccggtgctgattaccaattaacaaagttgttaggtttgtcccctacagtcaaaaggttaatgatgtaccaacaaggttgctttggtggtgcaactgttttgagattggcaaaagatatcgctgaaaataatagaggtgccagagtgttagtcgtttgttccgagataactgctatggccttcagaggtccatgcaagagtcatttagattccttggtaggtcatgccttgttcggtgatggtgccgctgctgcaattataggcgctgacccagaccaattagacgaacaaccagttttccagttggtatcagcttctcagactatattaccagaatcagaaggtgccatagatggccatttaacagaagctggtttaactatacatttattaaaagatgttcctggtttaatttcagagaacattgaacaggctttggaggatgcctttgaacctttaggtattcataactggaattcaattttctggattgcacatcctggtggccctgccattttagacagagttgaagatagagtaggattggataagaagagaatgagggcttctagggaagtgttatctgaatacggaaatatgtctagtgcctctgtgttgtttgtgttagatgtcatgaggaaaagttctgctaaagacggattggcaaccacaggagaaggaaaagattggggagtgttgtttggattcggaccaggcttgactgtagaaaccttagtgttgcatagtgtcccagtccctgtccctactgcagcttctgcatga

SEQ ID NO: 5 - DNA, 1452 bp, Malus domestica
atgggtgatgtcattgtcttgtatgcttctccaggtatgggtcatatagtttccatggttgaattgggtaaattcatcgttcatagatacggtccacacaagttctctattactatcttgtacacctgtggttccatcgttgatactgcttctattccagtttacatcagaagaatctcccattcccatccattcatctcattcagacaattcccaagagttaccaacaacatcaccagaaacatttccgttccagctattaccttcgacttcatcagacaaaatgatccacatgttagatccgccttgcaagaaatttcaaagtctgctactgttagagccttcatcattgatttgttctgtacttccgctttgccaatcggtaaagaattcaacattccaacctactacttcagaacttctggtgctgctattttggctgctttcttgtacttgccaaagatcgatgaacaaactaagaccaccgaatctttcaaggatttgagagataccgttttcgaatttccaggttggaaatctccattgaaggctactcatatggttcaattggttttggatagaaacgatccagcctactctgatatgatctacttctgttctcatttgccaaagtccaacggtattatcgttaacaccttcgaagaattggaaccaccatctgttttacaagctattgctggtggtttgtgtgttccagatggtccaactccaccagtttattatgttggtccattgatcgaagaagaaaaagaattgtccaaggatgctgatgctgccgaaaaagaagattgcttgtcttggttggataagcaaccatctagatccgttttgttcttgtgttttggttccatgggttcttttccagctgctcaattgaaagaaattgccaatggtttggaagcctctggtcaaagatttttgtgggttgttaagaagccaccagtcgaagaaaaatccaaacaagttcatggtgttgacgacttcgatttgaaaggtgttttgccagaaggtttcttggaaagaactgctgatagaggtatggttgtaaaatcttgggctccacaagttgtcgtcttgaagaaagaatctgttggtggtttcgttactcattgtggttggaattctgttttggaagctgttgttgctggtgttccaatgattgcttggccattatatgctgaacaacacatgaatagaaacgtcttggttaccgatatggaaatcgctattggtgtcgaacaaagagatgaagaaggtggttttgtttccggtgaagaagttgaaagaagagttagagaattgatggaatccgaaggtggtagagttttgagagaaagatgtaaaaagttgggtgaaatggcttctgctgctttaggtgaaactggttcttctactagaaacttggtcaacttcgtttcctccattacctga

SEQ ID NO: 6 - DNA, 2076 bp, Saccharomyces cerevisiae
atgccgtttggaatagacaacaccgacttcactgtcctggcggggctagtgcttgccgtgctactgtacgtaaagagaaactccatcaaggaactgctgatgtccgatgacggagatatcacagctgtcagctcgggcaacagagacattgctcaggtggtgaccgaaaacaacaagaactacttggtgttgtatgcgtcgcagactgggactgccgaggattacgccaaaaagttttccaaggagctggtggccaagttcaacctaaacgtgatgtgcgcagatgttgagaactacgactttgagtcgctaaacgatgtgcccgtcatagtctcgatttttatctctacatatggtgaaggagacttccccgacggggcggtcaactttgaagactttatttgtaatgcggaagcgggtgcactatcgaacctgaggtataatatgtttggtctgggaaattctacttatgaattctttaatggtgccgccaagaaggccgagaagcatctctccgctgcgggcgctatcagactaggcaagctcggtgaagctgatgatggtgcaggaactacagacgaagattacatggcctggaaggactccatcctggaggttttgaaagacgaactgcatttggacgaacaggaagccaagttcacctctcaattccagtacactgtgttgaacgaaatcactgactccatgtcgcttggtgaaccctctgctcactatttgccctcgcatcagttgaaccgcaacgcagacggcatccaattgggtcccttcgatttgtctcaaccgtatattgcacccatcgtgaaatctcgcgaactgttctcttccaatgaccgtaattgcatccactctgaatttgacttgtccggctctaacatcaagtactccactggtgaccatcttgctgtttggccttccaacccattggaaaaggtcgaacagttcttatccatattcaacctggaccctgaaaccatttttgacttgaagcccctggatcccaccgtcaaagtgcccttcccaacgccaactactattggcgctgctattaaacactatttggaaattacaggacctgtctccagacaattgttttcatctttgattcagttcgcccccaacgctgacgtcaaggaaaaattgactctgctttcgaaagacaaggaccaattcgccgtcgagataacctccaaatatttcaacatcgcagatgctctgaaatatttgtctgatggcgccaaatgggacaccgtacccatgcaattcttggtcgaatcagttccccaaatgactcctcgttactactctatctcttcctcttctctgtctgaaaagcaaaccgtccatgtcacctccattgtggaaaactttcctaacccagaattgcctgatgctcctccagttgttggtgttacgactaacttgttaagaaacattcaattggctcaaaacaatgttaacattgccgaaactaacctacctgttcactacgatttaaatggcccacgtaaacttttcgccaattacaaattgcccgtccacgttcgtcgttctaacttcagattgccttccaacccttccaccccagttatcatgatcggtccaggtaccggtgttgccccattccgtgggtttatcagagagcgtgtcgcgttcctcgaatcacaaaagaagggcggtaacaacgtttcgctaggtaagcatatactgttttatggatcccgtaacactgatgatttcttgtaccaggacgaatggccagaatacgccaaaaaattggatggttcgttcgaaatggtcgtggcccattccaggttgccaaacaccaaaaaagtttatgttcaagataaattaaaggattacgaagaccaagtatttgaaatgattaacaacggtgcatttatctacgtctgtggtgatgcaaagggtatggccaagggtgtgtcaaccgcattggttggcatcttatcccgtggtaaatccattaccactgatgaagcaacagagctaatcaagatgctcaagacttcaggtagataccaagaagatgtctggtaa

SEQ ID NO: 7 - DNA, 933 bp, Saccharomyces cerevisiae
atgcctatcaccataaaaagccgctctaaagggttaagggacactgaaattgacttatccaaaaagcctactttagatgatgttttgaaaaaaatctctgctaataaccacaatatcagcaagtacaggataagattaacctacaaaaaggaatctaaacaagttccggttatttcagaatcgttttttcaagaagaggctgatgactcaatggaattcttcatcaaagatttgggtccccaaatttcatggagattagtcttcttttgtgagtatttgggtccagtcttggttcactcccttttttattatctatctaccattcccacagttgttgatagatggcacagtgctagctccgactataatccatttttaaacagggttgcatattttttaattttaggacattatggaaagagattatttgaaaccttatttgttcaccaattctctttagctactatgccaattttcaacctgttcaaaaattgtttccattactgggttctaagcggtctcatttcattcggttactttggctacggcttcccctttgggaatgctaagttattcaaatactattcatatttgaaattggatgacttgagtacattaattggtcttttcgtgctttcagaactatggaacttttattgccacattaaattgcgcctatggggtgactatcaaaagaagcatggtaacgctaagatccgtgtcccattgaatcaaggtattttcaatctttttgttgctcccaactatacttttgaagtttggtcttggatttggtttacttttgtgttcaagttcaatttatttgccgttttatttttgactgtttcaacagctcaaatgtacgcatgggctcaaaagaaaaacaaaaagtatcataccagaagagcattcttgattccatttgtattttga

SEQ ID NO: 8 - DNA, 22283 bp, pPHLO Multi-Expression Plasmid
acgcgtccagtatcccagcagatacgggatatcgacatttctgcaccattccggcgggtataggttttattgatggcctcatccacacgcagcagcgtctgttcatcgtcgtggcggcccataataatctgccggtcaatcagccagctttcctcacccggcccccatccccatacgcgcatttcgtagcggtccagctgggagtcgataccggcggtcaggtaagccacacggtcaggaacgggcgctgaataatgctctttccgctctgccatcacttcagcatccggacgttcgccaattttcgcctcccacgtctcaccgagcgtggtgtttacgaaggttttacgttttcccgtatcccctttcgttttcatccagtctttgacaatctgcacccaggtggtgaacgggctgtacgctgtccagatgtgaaaggtcacactgtcaggtggctcaatctcttcaccggatgacgaaaaccagagaatgccatcacgggtccagatcccggtcttttcgcagatataacgggcatcagtaaagtccagctcctgctggcggatgacgcaggcattatgctcgcagagataaaacacgctggagacgcgttttcccgtctttcagtgccttgttcagttcttcctgacgggcggtatatttctccagcttggcctatgcggccctgtcagaccaagtttacgagctcgcttggactcctgttgatagatccagtaatgacctcagaactccatctggatttgttcagaacgctcggttgccgccgggcgttttttattggtgagaatccaagcactagggacagtaagacgggtaagcctgttgatgataccgctgccttactgggtgcattagccagtctgaatgacctgtcacgggataatccgaagtggtcagactggaaaatcagagggcaggaactgctgaacagcaaaaagtcagatagcaccacatagcagacccgccataaaacgccctgagaagcccgtgacgggcttttcttgtattatgggtagtttccttgcatgaatccataaaaggcgcctgtagtgccatttacccccattcactgccagagccgtgagcgcagcgaactgaatgtcacgaaaaagacagcgactcaggtgcctgatggtcggagacaaaaggaatattcagcgatttgcccgagcttgcgagggtgctacttaagcctttagggttttaaggtctgttttgtagaggagcaaacagcgtttgcgacatccttttgtaatactgcggaactgactaaagtagtgagttatacacagggctgggatctattctttttatctttttttattctttctttattctataaattataaccacttgaatataaacaaaaaaaacacacaaaggtctagcggaatttacagagggtctagcagaatttacaagttttccagcaaaggtctagcagaatttacagatacccacaactcaaaggaaaaggacatgtaattatcattgactagcccatctcaattggtatagtgattaaaatcacctagaccaattgagatgtatgtctgaattagttgttttcaaagcaaatgaactagcgattagtcgctatgacttaacggagcatgaaaccaagctaattttatgctgtgtggcactactcaaccccacgattgaaaaccctacaaggaaagaacggacggtatcgttcacttataaccaatacgctcagatgatgaacatcagtagggaaaatgcttatggtgtattagctaaagcaaccagagagctgatgacgagaactgtggaaatcaggaatcctttggttaaaggctttgagattttccagtggacaaactatgccaagttctcaagcgaaaaattagaattagtttttagtgaagagatattgccttatcttttccagttaaaaaaattcataaaatataatctggaacatgttaagtcttttgaaaacaaatactctatgaggatttatgagtggttattaaaagaactaacacaaaagaaaactcacaaggcaaatatagagattagccttgatgaatttaagttcatgttaatgcttgaaaataactaccatgagtttaaaaggcttaaccaatgggttttgaaaccaataagtaaagatttaaacacttacagcaatatgaaattggtggttgataagcgaggccgcccgactgatacgttgattttccaagttgaactagatagacaaatggatctcgtaaccgaacttgagaacaaccagataaaaatgaatggtgacaaaataccaacaaccattacatcagattcctacctacataacggactaagaaaaacactacacgatgctttaactgcaaaaattcagctcaccagttttgaggcaaaatttttgagtgacatgcaaagtaagtatgatctcaatggttcgttctcatggctcacgcaaaaacaacgaaccacactagagaacatactggctaaatacggaaggatctgaggttcttatggctcttgtatctatcagtgaagcatcaagactaacaaacaaaagtagaacaactgttcaccgttacatatcaaagggaaaactgtccatatgcacagatgaaaacggtgtaaaaaagatagatacatcagagcttttacgagtttttggtgcattcaaagctgttcaccatgaacagatcgacaatgtaacgcggccgcagccaatcaattcttgcggagaactgtgaatgcgcaaaccaacccttggcagaacatatccatcgcgtccgccatctccagcagccgcacgcggcgcatcgggggggggggggggggtttcaattcatcattttttttttattcttttttttgatttcggtttccttgaaatttttttgattcggtaatctccgaacagaaggaagaacgaaggaaggagcacagacttagattggtatatatacgcatatgtagtgttgaagaaacatgaaattgcccagtattcttaacccaactgcacagaacaaaaacctgcaggaaacgaagataaatcatgtcgaaagctacatataaggaacgtgctgctactcatcctagtcctgttgctgccaagctatttaatatcatgcacgaaaagcaaacaaacttgtgtgcttcattggatgttcgtaccaccaaggaattactggagttagttgaagcattaggtcccaaaatttgtttactaaaaacacatgtggatatcttgactgatttttccatggagggcacagttaagccgctaaaggcattatccgccaagtacaattttttactcttcgaagacagaaaatttgctgacattggtaatacagtcaaattgcagtactctgcgggtgtatacagaatagcagaatgggcagacattacgaatgcacacggtgtggtgggcccaggtattgttagcggtttgaagcaggcggcagaagaagtaacaaaggaacctagaggccttttgatgttagcagaattgtcatgcaagggctccctatctactggagaatatactaagggtactgttgacattgcgaagagcgacaaagattttgttatcggctttattgctcaaagagacatgggtggaagagatgaaggttacgattggttgattatgacacccggtgtgggtttagatgacaagggagacgcattgggtcaacagtatagaaccgtggatgatgtggtctctacaggatctgacattattattgttggaagaggactatttgcaaagggaagggatgctaaggtagagggtgaacgttacagaaaagcaggctgggaagcatatttgagaagatgcggccagcaaaactaaaaaactgtattataagtaaatgcatgtatactaaactcacaaattagagcttcaatttaattatatcagttattacccggccgggaatctcggtcgtaatgatttttataatgacgaaaaaaaaaaaattggaaagaaaaccccccccccccccccgcagcgttgggtcctggccacgggtgcgcatgatcgtgctcctgtcgttgaggacccggctaggctggcggggttgccttactggttagcagaatgaatcaccgatacgcgagcgaatgtggcggccgcacgcgttcatcgtccacctccggagaacaggccaccatcacgcatctgtgtctgaatttcatcacgacgcgccttaagggcaccaataactgccttaaaaaaattacgccccgccctgccactcatcgcagtactgttgtaattcattaagcattctgccgacatggaagccatcacagacggcatgatgaacctgaatcgccagcggcatcagcaccttgtcgccttgcgtataatatttgcccatggtgaaaacgggggcgaagaagttgtccatattggccacgtttaaatcaaaactggtgaaactcacccagggattggctgagacgaaaaacatattctcaataaaccctttagggaaataggccaggttttcaccgtaacacgccacatcttgcgaatatatgtgtagaaactgccggaaatcgtcgtggtattcactccagagcgatgaaaacgtttcagtttgctcatggaaaacggtgtaacaagggtgaacactatcccatatcaccagctcaccgtctttcattgccatacggaattccggatgagcattcatcaggcgggcaagaatgtgaataaaggccggataaaacttgtgcttatttttctttacggtctttaaaaaggccgtaatatccagctgaacggtctggttataggtacattgagcaactgactgaaatgcctcaaaatgttctttacgatgccattgggatatatcaacggtggtatatccagtgatttttttctccattttagcttccttagctcctgaaaatctcgataactcaaaaaatacgcccggtagtgatcttatttcattatggtgaaagttggaacctcttacgtgccgatcaacgtctcattttcgccaaaagttggcccagggcttcccggtatcaacagggacaccaggatttatttattctgcgaagtgatcttccgtcacaggtattggaccaccctgtgggtttataagcgcgctgctggcgtgtaaggcggtgacggcgaaggaagggtccttttcatcacgtgctataaaaataattataatttaaattttttaatataaatatataaattaaaaatagaaagtaaaaaaagaaattaaagaaaaaatagtttttgttttccgaagatgtaaaagactctagggggatcgccaacaaatactaccttttatcttgctcttcctgctctcaggtattaatgccgaattgtttcatcttgtctgtgtagaagaccacacacgaaaatcctgtgattttacattttacttatcgttaatcgaatgtatatctatttaatctgcttttcttgtctaataaatatatatgtaaagtacgctttttgttgaaattttttaaacctttgtttatttttttttcttcattccgtaactcttctaccttctttatttactttctaaaatccaaatacaaaacataaaaataaataaacacagagtaaattcccaaattattccatcattaaaagatacgaggcgcgtgtaagttacaggcaagcgatccgtcctaagaaaccattattatcatgacattaacctataaaaataggcgtatcacgaggccctttcgtctcgcgcgtttcggtgatgacggtgaaaacctctgacacatgcagctcccggagacggtcacagcttgtctgtaagcggatgccgggagcagacaagcccgtcagggcgcgtcagcgggtgttggcgggtgtcggggctggcttaactatgcggcatcagagcagattgtactgagagtgcaccacggcgcgtggcacccttgcgggccatgtcatacaccgccttcagagcagccggacctatctgcccgttacgcgccagcttgcaaattaaagccttcgagcgtcccaaaaccttctcaagcaaggttttcagtataatgttacatgcgtacacgcgtctgtacagaaaaaaaagaaaaatttgaaatataaataacgttcttaatactaacataactataaaaaaataaatagggacctagacttcaggttgtctaactccttccttttcggttagagcggatgtggggggagggcgtgaatgtaagcgtgacataactaattacatgatatcgacaaaggaaaagggggacggatctccgaggcctcggacccgtcgggccgccgtcggacgtgccgcggtcatgcagaagctgcagtagggacagggactgggacactatgcaacactaaggtttctacagtcaagcctggtccgaatccaaacaacactccccaatcttttccttctcctgtggttgccaatccgtctttagcagaacttttcctcatgacatctaacacaaacaacacagaggcactagacatatttccgtattcagataacacttccctagaagccctcattctcttcttatccaatcctactctatcttcaactctgtctaaaatggcagggccaccaggatgtgcaatccagaaaattgaattccagttatgaatacctaaaggttcaaaggcatcctccaaagcctgttcaatgttctctgaaattaaaccaggaacatcttttaataaatgtatagttaaaccagcttctgttaaatggccatctatggcaccttctgattctggtaatatagtctgagaagctgataccaactggaaaactggttgttcgtctaattggtctgggtcagcgcctataattgcagcagcggcaccatcaccgaacaaggcatgacctaccaaggaatctaaatgactcttgcatggacctctgaaggccatagcagttatctcggaacaaacgactaacactctggcacctctattattttcagcgatatcttttgccaatctcaaaacagttgcaccaccaaagcaaccttgttggtacatcattaaccttttgactgtaggggacaaacctaacaactttgttaattggtaatcagcaccgggcatgtcaacgccggatgttgtgcaaaataccaaatgagtaatcttagacaagggttggccccactccttaatggccttctcagctgcaccttggcccaatttgggaacttcaactaatgcgatggcgtgtctagcatccaatgaggtctccatgtgtgcacagatctttgggttcttgatcaatatttcctcggtcaagtgcatgtgtctctttctaatcattgatttgtcacacattctttgaaacttctcctttaaatctgccaagtgctcacttttagtaaccctaaaataataatctggataggtagcttgataaacacaattagctggaacggcagtaccgattgctaaaactgtagctaaaccttcagccctctgtgccattctaacttctttcaatcttactgcagccattttaagctttttgtttgtttatgtgtgtttattcgaaactaagttcttggtgttttaaaactaaaaaaaagactaactataaaagtagaatttaagaagtttaagaaatagatttacagaattacaatcaatacctaccgtctttatatacttattagtcaagtaggggaataatttcagggaactggtttcaaccttttttttcagctttttccaaatcagagagagcagaaggtaatagaaggtgtaagaaaatgagatagatacatgcgtgggtcaattgccttgtgtcatcatttactccaggcaggttgcatcactccattgaggttgtgtccgttttttgcctgtttgtgcccctgttctctgtagttgcgctaagagaatggacctatgaactgatggttggtgaagaaaacaatattttggtgctgggattctttttttttctggatgccagcttaaaaagcgggctccattatatttagtggatgccaggaataaactgttcacccagacacctacgatgttatatattctgtgtaacccgccccctattttgggcatgtacgggttacagcagaattaaaaggctaattttttgactaaataaagttaggaaaatcactactattaattatttacgtattctttgaaatggcagtattgataatgataaactcgaactgggcgcgtcgtgccgtcgttgttaatcaccacatggttattctgctcaaacgtcccggacgcctgcgaacgcgccgaaggaaaatgagaaatatcgagggagacgattcagaggagcaggacaaactataaccgactgtttgttggaggatgccgtacataacgaacactgctgaagctaccatgtctacagtttagaggaatgggtacaactcacaggcgagggatggtgttcactcgtgctagcaaacgcggtgggagcaaaaagtagaatattatcttttattcgtgaaacttcgaacactgtcatctaaagatgctatatactaatataggcatacttgataatgaaaactataaatcgtaaagacataagagatccgcggtcaaaatacaaatggaatcaagaatgctcttctggtatgatactttttgtttttcttttgagcccatgcgtacatttgagctgttgaaacagtcaaaaataaaacggcaaataaattgaacttgaacacaaaagtaaaccaaatccaagaccaaacttcaaaagtatagttgggagcaacaaaaagattgaaaataccttgattcaatgggacacggatcttagcgttaccatgcttcttttgatagtcaccccataggcgcaatttaatgtggcaataaaagttccatagttctgaaagcacgaaaagaccaattaatgtactcaagtcatccaatttcaaatatgaatagtatttgaataacttagcattcccaaaggggaagccgtagccaaagtaaccgaatgaaatgagaccgcttagaacccagtaatggaaacaatttttgaacaggttgaaaattggcatagtagctaaagagaattggtgaacaaataaggtttcaaataatctctttccataatgtcctaaaattaaaaaatatgcaaccctgtttaaaaatggattatagtcggagctagcactgtgccatctatcaacaactgtgggaatggtagatagataataaaaaagggagtgaaccaagactggacccaaatactcacaaaagaagactaatctccatgaaatttggggacccaaatctttgatgaagaattccattgagtcatcagcctcttcttgaaaaaacgattctgaaataaccggaacttgtttagattcctttttgtaggttaatcttatcctgtacttgctgatattgtggttattagcagagatttttttcaaaacatcatctaaagtaggctttttggataagtcaatttcagtgtcccttaaccctttagagcggctttttatggtgataggcattttaagctttgttttatatttgttgtaaaaagtagataattacttccttgatgatctgtaaaaaagagaaaaagaaagcatctaagaacttgaaaaactacgaattagaaaagaccaaatatgtatttcttgcattgaccaatttatgcaagtttatatatatgtaaatgtaagtttcacgaggttctactaaactaaaccacccccttggttagaagaaaagagtgtgtgagaacaggctgttgttgtcacacgattcggacaattctgtttgaaagagagagagtaacagtacgatcgaacgaactttgctctggagatcacagtgggcatcatagcatgtggtactaaaccctttcccgccattccagaaccttcgattgcttgttacaaaacctgtgagccgtcgctaggaccttgttgtgtgacgaaattggaagctgcaatcaataggaagacaggaagtcgagcgtgtctgggttttttcagttttgttctttttgcaaacaaatcacgagcgacggtaatttctttctcgataagaggccacgtgctttatgagggtaacatcaattcaagaaggagggaaacacttcctttttctggccctgataatagtatgagggtgaagccaaaataaaggattcgcgcccaaatcggcatctttaaatgcaggtatgcgatagttcctcactctttccttactcacgagtaattcttgcaaatgcctattatgcagatgttataatatctgtgcgtggcgcgtccggctgtctgccatgctgcccggtgtaccgacataaccgccggtggcatagccgcgcatacgcgccatttccttccatcttgtgattcatgctatccatcttttttgagtatccaattaacgaagacgttaccagctgattgaaggttctcaaagtgactgtactccatgttttcttatcatccatgtagttatttttcaaactgcaaattcaagaaaaagccacgcgtgtgcaccttttttttccccttccagtgcattatgcaatagacagcacgagtctttgaaaaagtaacttataaaactgtatcaatttttaaacctaaatagattcataaactattcgttaatataaagtgttctaaactatgatgaaaaaataagcagaaaagactaataattcttagttaaaagcactccctagttcattaatccatttgctagtcttgctcttagatccttcctcaatatcttccctgatggagctttaggaatagagtcagtgaagaacactttgttgattctcttataaaacacaacctgttttgacacgaattgcttgatttcatcttcggatatatttgaatctttcgatctcaccacaaacgcaacaggaacctcaccagcatcttcttccttcatggcgacgacagcaacatcattgatttctggatgacctatgaggagagactctagctcagctggagccacttgaaatcctttgtacttgatgagttctttcaatctatccacaatgaaaagctcgtcgtcatcatcgataaatccgacgtctccagtgtgaagccaaccatctttatcgatcgtcgatgccgtggccaaggggtcattgagatagcctttcatgatttggttgccacggatgcatatttcgccgggtttgttcctaggcaaagaatctcctgtgtctggatcaagtatcttcatctcggcgttcctcaccaccgtaccacatgctcctgacttcactggaaacggctctttagcaaaccctaacgacattgctagcaccggacctgcttctgtcatcccatagccctgaccaagcttggcgttaggaaacttagcactaatagcatcttcaagctccttaccaagaggagctgctccagacttaaccatcctaaccgagctcagatcatacttctccgtctccggcgacttcgcgatagctaaaacgatcggtggcacgaccatagccaccgtgactttacacctttgtatctgctctaacaagagagtgatttcgaacttaggcattatcaagatcgtggcaccaactctgagactacagagcatgatggagttgagagcgtatatatggaacataggcaagacacagaggatcacgtcgtctctgttgaagtaaagattcggattctcgccgtcgacttgctgcgccacgctcgtgactagacctttgtgtgttagcatcactcctttggggagacccgtcgtgccggatgagaaaggaagcgccacgacgtcttctggcgaaatcttctccggtattgagtccactcgtggttcttcggactgagttaactcggagaaacggaggcagttttcggggatggcgtcggagtcggtggtgacgatcaaaacgccgtcgttttggaggttcttgattttatcgacgtaacgggattgagtgacgatgagtttcgccgcggaggctttggcttgtttagaaatctccgccggagtgaagaacgggttcgcggaggtggtgattgcgccgatgaaggaggcggcaaggaaagtgaggactacttcaggagagttcgggaggaggatcattacaacgtcgtgttgcttcacgccgaggttatgaagaccggcggcgagtttccgagatgttacgtggacatcggcgtaggtgtatacttcgccggtgggaccgttgatcaagcatggcttagcggcgaactctgagatattttcgaagatgtagtcgtggagtgggaggtggttagggatgtatatatcaggcaatctcgatcggaaaatgacgtcattactacactgtttctgatcattctgatcattgactatcacatcttgtgtcgtcattttagctttttgtaattaaaacttagattagattgctatgctttctttctaatgagcaagaagtaaaaaaagttgtaatagaacaagaaaaatgaaactgaaacttgagaaattgaagaccgtttattaacttaaatatcaatgggaggtcatcgaaagagaaaaaaatcaaaaaaaaaaattttcaagaaaaagaaacgtgataaaaatttttattgcctttttcgacgaagaaaaagaaacgaggcggtctcttttttcttttccaaacctttagtacgggtaattaacgacaccctagaggaagaaagaggggaaatttagtatgctgtgcttgggtgttttgaagtggtacggcgatgcgcggagtccgagaaaatctggaagagtaaaaaaggagtagaaacattttgaagctaggcgcgtcagccggtaaagattccccacgccaatccggctggttgcctccttcgtgaagacaaactcacgcgcctccaaaatgagctatcaaaaacgatagatcgattaggatgactttgaaatgactccgcagtggactggccgttaatttcaagcgtgagtaaaatagtgcatgacaaaagatgagctaggcttttgtaaaaatatcttacgttgtaaaattttagaaatcattatttccttcatatcattttgtcattgaccttcagaagaaaagagccgaccaataatataaataaataaataaaaataatattccattatttctaaacagattcaatactcattaaaaaactatatcaattaatttgaattaaccgcggttagcagattggaataggtgcaccattccactctttcaagcaatccataagtggatctatcaactttccctcgcacatagctgtgaataccttgtcaaattcttcacctgggctaacgactttttcaccagttagtaatttggttcccaactcttctctaacgaatctgtacaaagggtacgacctacactctttgattctatttggtataggggcagtaccatttccgtatgcggctctagcagcttcgacttcctttggtaaaactgccttcagttcttcttcaaaggcacctatcttttggaatattgaagtaacggcatttttctcagtttcaccattggataaagcgtgatctacaataacttgtctcaatctctgcatcaatggataagtagcgctacatggatcgtcaacgtaagtaaatacttgttctctatctacaacttttaataaatctttttcacagaatcttgatgggtgcaattcaccattgatacctgtagttagaaccttttttgcaacctgtgatacggtatttttcactgtctgtctcaaattctcttccaagtgtctcaaatctacggcctggcatatacccactaaaaatgttgtggacattaatttaaggatatcaacggcctcgcttgtttttcttgatgaaatcaggcccaaagaattaacatcctgattgtgttgttcggctgattgtacatgagaggttactgggttggctagatattgcagctctgaacaatagcttgccattgctatctcagcacctttgaaaccataatcaagactagggttagaagatgcggtcagattcgaaggcaaaccgttattgtagaagtcattgaccaattcagaaaattgggcaaacattaatttgccaattgcggctatggcaagcctggtattatccatactgactcctatgggtgtaccctggaaattgcctccatgtattgccttattcctcgacacatcaataagtggattatcgttaacagagttgatctctctttctatagactttgtagcttgtctaattacttcaatttgagggccaagccattgtggggatgtccttaaagcatatctatcttgtttgggtttttgcaaagggtccatttcatgaaccttctgggctaacttcatgtagctagagccgtccaaaatgtgctccatgatagctgctgcttcaatttgtcctgggtgatgttttaacctgtgggtcaagtgatcagtaaactcaggttttccactcatgacttcggcaaaaattgcggacaaaacttcggccaaaactgcttgtacgttagcttcaaacaacaccatggatgccataccgctgccgacagcggtgccattcaccagggctaaaccttccttgggttgcaaatcaaagaaaccagttgaaataccagctttctcaaatgcttccttagcggttaaggattctccgtctggaccagtggcctttgaattaggtcttcccgttaataagcctgcgatatatgaaaggggaaccaaatcaccgctggcagttattgttcctcttaagggcaacgaaggagaaatgttgtggttcaatagtgaagtgatggcctcaagaatttcaaaccttattccagagtaaccttgcaacaaagtgttcaccctaacaagcatagcagctcttgttgccgattggggtaatgtatggcaagtttcctttgtattaccgaaaataccggcgttaaggaatctgatcagttctgtttgcaaagcagtgccatttttagttcttctatgagaggtagcaccaaagcctgtggtaacgccataggaatctgtgcccttgttcatactttccatgacccaatctgatgaagccttaactccggctctacttgtttctgcaagttctaccttcactgaaccgccaacggtcgaaatagcagctacctgtcctatcgtcaatgtctcgccgcctagatttacgactggtcttctgtattcctcaaccatcttcttaacttcatccagatggctacctttcatctggtcagctgccagaccccaattcaaaggatctgcaagagtttttgtcgttacggccaccttggtcttttcaccaccaccgcatagcattgcttcaatttggtccattttaagctttttgatagatttgactgtgttattttgcgtgaggttatgagtagaaaataataattgagaaaggaatatgacaagaaatatgaaaataaagggaacaaacccaaatctgattgcaaggagagtgaaagagccttgtttatatatttttttttcctatgttcaacgaggacagctaggtttatgcaaaaatgtgccatcaccataagctgattcaaatgagctaaaaaaaaaatagttagaaaataaggtggtgttgaacgatagcaagtagatcaagacaccgtctaacagaaaaaggggcagcggacaatattatgcaattatgaagaaaagtactcaaagggtcggaaaaatattcaaacgatatttgcataaaatcctcaattgattgattattccatagtaaaataccgtaacaacacaaaattgttctcaaattcataaattattcattttttccacgagcctcatcacacgaaaagtcagaagagcatacataatcttttaaatgcataggttatgcattttgcaaatgccaccaggcaacaaaaatatgcgtttagcgggcggaatcgggaaggaagccggaaccaccaaaaactggaagctacgtttttaaggaaggtatgggtgcagtgtgcttatctcaagaaatattagttatgatataaggtgttgaagtttagagataggtaaataaacgcggggtgtgtttattacatgaagaagaagttagtttctgccttgcttgtttatcttgcacatcacatcagcggaacatatgctcacccagtcgcatggcgcgtaccacggtgaacaatccccgctggctcatatttgccgccggttcccgtaaatcctccggtacgcgccgggccgtatacttacatatagtagatgtcaagcgtaggcgcttcccctgccggctgtgagggcgccataaccaaggtatctatagaccgccaatcagcaaactacctccgtacattcatgttgcacccacacatttatacacccagaccgcgacaaattacccataaggttgtttgtgacggcgtcgtacaagagaacgtgggaactttttaggctcaccaaaaaagaaagaaaaaatacgagttgctgacagaagcctcaagaaaaaaaaaattcttcttcgactatgctggaggcagagatgatcgagccggtagttaactatatatagctaaattggttccatcaccttcttttctggtgtcgctccttctagtgctatttctggcttttcctatttttttttttccatttttctttctctctttctaatatataaattctcttgcattttctatttttctctctatctattctacttgtttattcccttcaaggtttttttttaaggagtacttgtttttagaatatacggtcaacgaactataattaactaaacaagcttaaaatgatggattttgttttgttagaaaaagctcttcttggtttgttcattgcaactatagtagccatcacaatctctaagctaaggggaaagaaacttaagttgcctccaggcccaatccctgtcccagtgtttggtaattggttacaagttggcgacgacttaaaccagaggaatttggtagagtatgctaaaaagttcggcgacttatttctacttaggatgggtcaaagaaacttggtcgtggtttcatcccctgacttagcaaaagacgtactacatacccagggtgtcgagttcggaagtagaactagaaatgttgtgtttgatattttcacaggcaaaggtcaagatatggtttttaccgtatacagcgagcactggaggaaaatgagaagaataatgactgtcccattctttacaaacaaagtggttcaacagtataggttcggatgggaggacgaagccgctagagtagtcgaggatgttaaggcaaatcctgaagccgctaccaacggtattgtgttgaggaatagattacaacttttgatgtacaacaatatgtatagaataatgtttgacaggagatttgaatctgttgatgatccattattcctaaaacttaaggcattgaatggcgagagatcaaggttagctcaatcctttgaatacaacttcggtgacttcattcctatattgaggccattcttgagaggatatcttaagttgtgtcaggaaatcaaggacaaaaggttaaagctattcaaggactacttcgtcgacgagagaaaaaagttggagagtatcaagagcgtaggtaataactccttaaagtgcgccatagatcatattatcgaggcacaagaaaaaggcgagataaacgaggataacgtgttatacatcgtcgagaatatcaacgtggctgccattgaaactacactttggtctattgaatggggtatagcagaactagtgaataaccctgaaatccagaaaaaattgagacacgaattagacaccgtacttggagctggtgttcaaatttgtgaaccagatgttcaaaaattgccttatctacaggccgtgataaaagagactttaaggtacaggatggcaattccattgttagtcccacatatgaatcttcacgaagccaaattggccggctatgatatccctgcagagagcaaaattttggtaaacgcttggtggttagccaataatccagcacattggaacaaacctgatgagtttagaccagaaagatttttggaggaagaatccaaggtcgaggctaatggaaacgactttaagtacatccctttcggtgttggcagaagatcttgcccaggtataattcttgctttaccaatccttggaatagtaattggtaggttggttcaaaacttcgagttacttccacctccaggccaaagcaaaatagatacagccgaaaaaggtggacagttttcattgcaaatcctaaagcattccactattgtgtgtaaacctagaagttcttaaccgcggacaaatcgctcttaaatatatacctaaagaacattaaagctatattataagcaaagatacgtaaattttgcttatattattatacacatatcatatttctatatttttaagatttggttatataatgtacgtaatgcaaaggaaataaattttatacattattgaacagcgtccaagtaactacattatgtgcactaatagtttagcgtcgtgaagactttattgtgtcgcgaaaagtaaaaattttaaaaattagagcaccttgaacttgcgaaaaaggttctcatcaactgtttaaaaggaggatatcaggtcctatttctgacaaacaatatacaaatttagtttcaaaggcgcgttgcaaaatggaatttcgccgcagcggcctgaatggctgtaccgcctgacgcggatgcgccacgcgccgcatgccggtagaggtgtggtcaataagagcgacctcatgctatacctgagaaagcaacctgacctacaggaaagagttactcaagaataagaattttcgttttaaaacctaagagtcactttaaaatttgtatacacttattttttttataacttatttaataataaaaatcataaatcataagaaattcgcttatttagaagtgtcaacaacgtatctaccaacgatttgacccttttccatcttttcgtaaatttctggcaaggtagacaagccgacaaccttgattggagacttgaccaaacctctggcgaagaagtccaaagctctagatcaatttaggcctgcggccgcggttaccagacatcttcttggtatctacctgaagtcttgagcatcttgattagctctgttgcttcatcagtggtaatggatttaccacgggataagatgccaaccaatgcggttgacacacccttggccataccctttgcatcaccacagacgtagataaatgcaccgttgttaatcatttcaaatacttggtcttcgtaatcctttaatttatcttgaacataaacttttttggtgtttggcaacctggaatgggccacgaccatttcgaacgaaccatccaattttttggcgtattctggccattcgtcctggtacaagaaatcatcagtgttacgggatccataaaacagtatatgcttacctagcgaaacgttgttaccgcccttcttttgtgattcgaggaacgcgacacgctctctgataaacccacggaatggggcaacaccggtacctggaccgatcatgataactggggtggaagggttggaaggcaatctgaagttagaacgacgaacgtggacgggcaatttgtaattggcgaaaagtttacgtgggccatttaaatcgtagtgaacaggtaggttagtttcggcaatgttaacattgttttgagccaattgaatgtttcttaacaagttagtcgtaacaccaacaactggaggagcatcaggcaattctgggttaggaaagttttccacaatggaggtgacatggacggtttgcttttcagacagagaagaggaagagatagagtagtaacgaggagtcatttggggaactgattcgaccaagaattgcatgggtacggtgtcccatttggcgccatcagacaaatatttcagagcatctgcgatgttgaaatatttggaggttatctcgacggcgaattggtccttgtctttcgaaagcagagtcaatttttccttgacgtcagcgttgggggcgaactgaatcaaagatgaaaacaattgtctggagacaggtcctgtaatttccaaatagtgtttaatagcagcgccaatagtagttggcgttgggaagggcactttgacggtgggatccaggggcttcaagtcaaaaatggtttcagggtccaggttgaatatggataagaactgttcgaccttttccaatgggttggaaggccaaacagcaagatggtcaccagtggagtacttgatgttagagccggacaagtcaaattcagagtggatgcaattacggtcattggaagagaacagttcgcgagatttcacgatgggtgcaatatacggttgagacaaatcgaagggacccaattggatgccgtctgcgttgcggttcaactgatgcgagggcaaatagtgagcagagggttcaccaagcgacatggagtcagtgatttcgttcaacacagtgtactggaattgagaggtgaacttggcttcctgttcgtccaaatgcagttcgtctttcaaaacctccaggatggagtccttccaggccatgtaatcttcgtctgtagttcctgcaccatcatcagcttcaccgagcttgcctagtctgatagcgcccgcagcggagagatgcttctcggccttcttggcggcaccattaaagaattcataagtagaatttcccagaccaaacatattatacctcaggttcgatagtgcacccgcttccgcattacaaataaagtcttcaaagttgaccgccccgtcggggaagtctccttcaccatatgtagagataaaaatcgagactatgacgggcacatcgtttagcgactcaaagtcgtagttctcaacatctgcgcacatcacgtttaggttgaacttggccaccagctccttggaaaactttttggcgtaatcctcggcagtcccagtctgcgacgcatacaacaccaagtagttcttgttgttttcggtcaccacctgagcaatgtctctgttgcccgagctgacagctgtgatatctccgtcatcggacatcagcagttccttgatggagtttctctttacgtacagtagcacggcaagcactagccccgccaggacagtgaagtcggtgttgtctattccaaacggcattttactagtaagctttgtgatgatgttttatttgttttgattggtgtcttgtaaatagaaacaagagagaataataaacaagttaagaataaaaaaccaaaggatgaaaaagaatgaatatgaaaaagagtagagaataactttgaaaggggaccatgatataactggaaaaaagaggttcttggaaatgaaaagttaccaaagagtatttataattcagaaaaaaaagccaacgaatatcgttttgatggcgagcctttttttttttttaggaagacactaaaggtacctagcatcatatgggaaggaaaggaaatcacttggaagacatcacaagcattcatttaccaagagaaaaaatatgcattttagctaagatccattgaacaaagcactcactcaactcaactgaatgaacgaaagaagaaagaacagtagaaaacactttgtgacggtgcggaacacatttacgtagctatcatgctgaattctactatgaaaatctcccaatctgtcgatggcaaaacgacccacgtggcagagttgggtcaagtgccagtttctggattaagtaacagatacagacatcacacgccatagaggaatcccgccgttgcgagagatggaaaacaatagagccgaaattgtggaagcccgatgtctgggtgtacattttttttttttctttctttctctttcaataatctttcctttttccatttagcttgccggaaaaactttcgggtagcgaaaatctttctgccggaaaaattagctatttttttcttccttattatttttttagttctgaagtttgaccagggcgctaccctgaccgtatcacaaccgacgatccggggtcatggcggctatttttttttttttttttttttccttgtgattgtttatttacatttggatcaattctaacaaaaaaaaaataaggggggaaaaataattcacctctttttaatattgttttgtactgagattgatctccaaaatagtagcattggcgcgtgccaccaacagccccgccaatggcgctgccgatactcccgacaatccccaccattgcctg

SEQ ID NO: 9 - DNA, 22010 bp, pPHLON Multi-Expression Plasmid
acgcgtccagtatcccagcagatacgggatatcgacatttctgcaccattccggcgggtataggttttattgatggcctcatccacacgcagcagcgtctgttcatcgtcgtggcggcccataataatctgccggtcaatcagccagctttcctcacccggcccccatccccatacgcgcatttcgtagcggtccagctgggagtcgataccggcggtcaggtaagccacacggtcaggaacgggcgctgaataatgctctttccgctctgccatcacttcagcatccggacgttcgccaattttcgcctcccacgtctcaccgagcgtggtgtttacgaaggttttacgttttcccgtatcccctttcgttttcatccagtctttgacaatctgcacccaggtggtgaacgggctgtacgctgtccagatgtgaaaggtcacactgtcaggtggctcaatctcttcaccggatgacgaaaaccagagaatgccatcacgggtccagatcccggtcttttcgcagatataacgggcatcagtaaagtccagctcctgctggcggatgacgcaggcattatgctcgcagagataaaacacgctggagacgcgttttcccgtctttcagtgccttgttcagttcttcctgacgggcggtatatttctccagcttggcctatgcggccctgtcagaccaagtttacgagctcgcttggactcctgttgatagatccagtaatgacctcagaactccatctggatttgttcagaacgctcggttgccgccgggcgttttttattggtgagaatccaagcactagggacagtaagacgggtaagcctgttgatgataccgctgccttactgggtgcattagccagtctgaatgacctgtcacgggataatccgaagtggtcagactggaaaatcagagggcaggaactgctgaacagcaaaaagtcagatagcaccacatagcagacccgccataaaacgccctgagaagcccgtgacgggcttttcttgtattatgggtagtttccttgcatgaatccataaaaggcgcctgtagtgccatttacccccattcactgccagagccgtgagcgcagcgaactgaatgtcacgaaaaagacagcgactcaggtgcctgatggtcggagacaaaaggaatattcagcgatttgcccgagcttgcgagggtgctacttaagcctttagggttttaaggtctgttttgtagaggagcaaacagcgtttgcgacatccttttgtaatactgcggaactgactaaagtagtgagttatacacagggctgggatctattctttttatctttttttattctttctttattctataaattataaccacttgaatataaacaaaaaaaacacacaaaggtctagcggaatttacagagggtctagcagaatttacaagttttccagcaaaggtctagcagaatttacagatacccacaactcaaaggaaaaggacatgtaattatcattgactagcccatctcaattggtatagtgattaaaatcacctagaccaattgagatgtatgtctgaattagttgttttcaaagcaaatgaactagcgattagtcgctatgacttaacggagcatgaaaccaagctaattttatgctgtgtggcactactcaaccccacgattgaaaaccctacaaggaaagaacggacggtatcgttcacttataaccaatacgctcagatgatgaacatcagtagggaaaatgcttatggtgtattagctaaagcaaccagagagctgatgacgagaactgtggaaatcaggaatcctttggttaaaggctttgagattttccagtggacaaactatgccaagttctcaagcgaaaaattagaattagtttttagtgaagagatattgccttatcttttccagttaaaaaaattcataaaatataatctggaacatgttaagtcttttgaaaacaaatactctatgaggatttatgagtggttattaaaagaactaacacaaaagaaaactcacaaggcaaatatagagattagccttgatgaatttaagttcatgttaatgcttgaaaataactaccatgagtttaaaaggcttaaccaatgggttttgaaaccaataagtaaagatttaaacacttacagcaatatgaaattggtggttgataagcgaggccgcccgactgatacgttgattttccaagttgaactagatagacaaatggatctcgtaaccgaacttgagaacaaccagataaaaatgaatggtgacaaaataccaacaaccattacatcagattcctacctacataacggactaagaaaaacactacacgatgctttaactgcaaaaattcagctcaccagttttgaggcaaaatttttgagtgacatgcaaagtaagtatgatctcaatggttcgttctcatggctcacgcaaaaacaacgaaccacactagagaacatactggctaaatacggaaggatctgaggttcttatggctcttgtatctatcagtgaagcatcaagactaacaaacaaaagtagaacaactgttcaccgttacatatcaaagggaaaactgtccatatgcacagatgaaaacggtgtaaaaaagatagatacatcagagcttttacgagtttttggtgcattcaaagctgttcaccatgaacagatcgacaatgtaacgcggccgcagccaatcaattcttgcggagaactgtgaatgcgcaaaccaacccttggcagaacatatccatcgcgtccgccatctccagcagccgcacgcggcgcatcgggggggggggggggggtttcaattcatcattttttttttattcttttttttgatttcggtttccttgaaatttttttgattcggtaatctccgaacagaaggaagaacgaaggaaggagcacagacttagattggtatatatacgcatatgtagtgttgaagaaacatgaaattgcccagtattcttaacccaactgcacagaacaaaaacctgcaggaaacgaagataaatcatgtcgaaagctacatataaggaacgtgctgctactcatcctagtcctgttgctgccaagctatttaatatcatgcacgaaaagcaaacaaacttgtgtgcttcattggatgttcgtaccaccaaggaattactggagttagttgaagcattaggtcccaaaatttgtttactaaaaacacatgtggatatcttgactgatttttccatggagggcacagttaagccgctaaaggcattatccgccaagtacaattttttactcttcgaagacagaaaatttgctgacattggtaatacagtcaaattgcagtactctgcgggtgtatacagaatagcagaatgggcagacattacgaatgcacacggtgtggtgggcccaggtattgttagcggtttgaagcaggcggcagaagaagtaacaaaggaacctagaggccttttgatgttagcagaattgtcatgcaagggctccctatctactggagaatatactaagggtactgttgacattgcgaagagcgacaaagattttgttatcggctttattgctcaaagagacatgggtggaagagatgaaggttacgattggttgattatgacacccggtgtgggtttagatgacaagggagacgcattgggtcaacagtatagaaccgtggatgatgtggtctctacaggatctgacattattattgttggaagaggactatttgcaaagggaagggatgctaaggtagagggtgaacgttacagaaaagcaggctgggaagcatatttgagaagatgcggccagcaaaactaaaaaactgtattataagtaaatgcatgtatactaaactcacaaattagagcttcaatttaattatatcagttattacccggccgggaatctcggtcgtaatgatttttataatgacgaaaaaaaaaaaattggaaagaaaaccccccccccccccccgcagcgttgggtcctggccacgggtgcgcatgatcgtgctcctgtcgttgaggacccggctaggctggcggggttgccttactggttagcagaatgaatcaccgatacgcgagcgaatgtggcggccgcacgcgttcatcgtccacctccggagaacaggccaccatcacgcatctgtgtctgaatttcatcacgacgcgccttaagggcaccaataactgccttaaaaaaattacgccccgccctgccactcatcgcagtactgttgtaattcattaagcattctgccgacatggaagccatcacagacggcatgatgaacctgaatcgccagcggcatcagcaccttgtcgccttgcgtataatatttgcccatggtgaaaacgggggcgaagaagttgtccatattggccacgtttaaatcaaaactggtgaaactcacccagggattggctgagacgaaaaacatattctcaataaaccctttagggaaataggccaggttttcaccgtaacacgccacatcttgcgaatatatgtgtagaaactgccggaaatcgtcgtggtattcactccagagcgatgaaaacgtttcagtttgctcatggaaaacggtgtaacaagggtgaacactatcccatatcaccagctcaccgtctttcattgccatacggaattccggatgagcattcatcaggcgggcaagaatgtgaataaaggccggataaaacttgtgcttatttttctttacggtctttaaaaaggccgtaatatccagctgaacggtctggttataggtacattgagcaactgactgaaatgcctcaaaatgttctttacgatgccattgggatatatcaacggtggtatatccagtgatttttttctccattttagcttccttagctcctgaaaatctcgataactcaaaaaatacgcccggtagtgatcttatttcattatggtgaaagttggaacctcttacgtgccgatcaacgtctcattttcgccaaaagttggcccagggcttcccggtatcaacagggacaccaggatttatttattctgcgaagtgatcttccgtcacaggtattggaccaccctgtgggtttataagcgcgctgctggcgtgtaaggcggtgacggcgaaggaagggtccttttcatcacgtgctataaaaataattataatttaaattttttaatataaatatataaattaaaaatagaaagtaaaaaaagaaattaaagaaaaaatagtttttgttttccgaagatgtaaaagactctagggggatcgccaacaaatactaccttttatcttgctcttcctgctctcaggtattaatgccgaattgtttcatcttgtctgtgtagaagaccacacacgaaaatcctgtgattttacattttacttatcgttaatcgaatgtatatctatttaatctgcttttcttgtctaataaatatatatgtaaagtacgctttttgttgaaattttttaaacctttgtttatttttttttcttcattccgtaactcttctaccttctttatttactttctaaaatccaaatacaaaacataaaaataaataaacacagagtaaattcccaaattattccatcattaaaagatacgaggcgcgtgtaagttacaggcaagcgatccgtcctaagaaaccattattatcatgacattaacctataaaaataggcgtatcacgaggccctttcgtctcgcgcgtttcggtgatgacggtgaaaacctctgacacatgcagctcccggagacggtcacagcttgtctgtaagcggatgccgggagcagacaagcccgtcagggcgcgtcagcgggtgttggcgggtgtcggggctggcttaactatgcggcatcagagcagattgtactgagagtgcaccacggcgcgtggcacccttgcgggccatgtcatacaccgccttcagagcagccggacctatctgcccgttacgcgccagcttgcaaattaaagccttcgagcgtcccaaaaccttctcaagcaaggttttcagtataatgttacatgcgtacacgcgtctgtacagaaaaaaaagaaaaatttgaaatataaataacgttcttaatactaacataactataaaaaaataaatagggacctagacttcaggttgtctaactccttccttttcggttagagcggatgtggggggagggcgtgaatgtaagcgtgacataactaattacatgatatcgacaaaggaaaagggggacggatctccgaggcctcggacccgtcgggccgccgtcggacgtgccgcggtcatgcagaagctgcagtagggacagggactgggacactatgcaacactaaggtttctacagtcaagcctggtccgaatccaaacaacactccccaatcttttccttctcctgtggttgccaatccgtctttagcagaacttttcctcatgacatctaacacaaacaacacagaggcactagacatatttccgtattcagataacacttccctagaagccctcattctcttcttatccaatcctactctatcttcaactctgtctaaaatggcagggccaccaggatgtgcaatccagaaaattgaattccagttatgaatacctaaaggttcaaaggcatcctccaaagcctgttcaatgttctctgaaattaaaccaggaacatcttttaataaatgtatagttaaaccagcttctgttaaatggccatctatggcaccttctgattctggtaatatagtctgagaagctgataccaactggaaaactggttgttcgtctaattggtctgggtcagcgcctataattgcagcagcggcaccatcaccgaacaaggcatgacctaccaaggaatctaaatgactcttgcatggacctctgaaggccatagcagttatctcggaacaaacgactaacactctggcacctctattattttcagcgatatcttttgccaatctcaaaacagttgcaccaccaaagcaaccttgttggtacatcattaaccttttgactgtaggggacaaacctaacaactttgttaattggtaatcagcaccgggcatgtcaacgccggatgttgtgcaaaataccaaatgagtaatcttagacaagggttggccccactccttaatggccttctcagctgcaccttggcccaatttgggaacttcaactaatgcgatggcgtgtctagcatccaatgaggtctccatgtgtgcacagatctttgggttcttgatcaatatttcctcggtcaagtgcatgtgtctctttctaatcattgatttgtcacacattctttgaaacttctcctttaaatctgccaagtgctcacttttagtaaccctaaaataataatctggataggtagcttgataaacacaattagctggaacggcagtaccgattgctaaaactgtagctaaaccttcagccctctgtgccattctaacttctttcaatcttactgcagccattttaagctttttgtttgtttatgtgtgtttattcgaaactaagttcttggtgttttaaaactaaaaaaaagactaactataaaagtagaatttaagaagtttaagaaatagatttacagaattacaatcaatacctaccgtctttatatacttattagtcaagtaggggaataatttcagggaactggtttcaaccttttttttcagctttttccaaatcagagagagcagaaggtaatagaaggtgtaagaaaatgagatagatacatgcgtgggtcaattgccttgtgtcatcatttactccaggcaggttgcatcactccattgaggttgtgtccgttttttgcctgtttgtgcccctgttctctgtagttgcgctaagagaatggacctatgaactgatggttggtgaagaaaacaatattttggtgctgggattctttttttttctggatgccagcttaaaaagcgggctccattatatttagtggatgccaggaataaactgttcacccagacacctacgatgttatatattctgtgtaacccgccccctattttgggcatgtacgggttacagcagaattaaaaggctaattttttgactaaataaagttaggaaaatcactactattaattatttacgtattctttgaaatggcagtattgataatgataaactcgaactgggcgcgtcgtgccgtcgttgttaatcaccacatggttattctgctcaaacgtcccggacgcctgcgaacgcgccgaaggaaaatgagaaatatcgagggagacgattcagaggagcaggacaaactataaccgactgtttgttggaggatgccgtacataacgaacactgctgaagctaccatgtctacagtttagaggaatgggtacaactcacaggcgagggatggtgttcactcgtgctagcaaacgcggtgggagcaaaaagtagaatattatcttttattcgtgaaacttcgaacactgtcatctaaagatgctatatactaatataggcatacttgataatgaaaactataaatcgtaaagacataagagatccgcggatccccgggtcgagcctgaacggcctcgaggcctgaacggcctcgacgaattcattatttgtagagctcatccatgccatgtgtaatcccagcagcagttacaaactcaagaaggaccatgtggtcacgcttttcgttgggatctttcgaaagggcagattgtgtcgacaggtaatggttgtctggtaaaaggacagggccatcgccaattggagtattttgttgataatggtctgctagttgaacggatccatcttcaatgttgtggcgaattttgaagttagctttgattccattcttttgtttgtctgccgtgatgtatacattgtgtgagttatagttgtactcgagtttgtgtccgagaatgtttccatcttctttaaaatcaataccttttaactcgatacgattaacaagggtatcaccttcaaacttgacttcagcacgcgtcttgtagttcccgtcatctttgaaagatatagtgcgttcctgtacataaccttcgggcatggcactcttgaaaaagtcatgccgtttcatatgatccggataacgggaaaagcattgaacaccataagagaaagtagtgacaagtgttggccatggaacaggtagttttccagtagtgcaaataaatttaagggtaagctggccctgcaggccaagctttgttttatatttgttgtaaaaagtagataattacttccttgatgatctgtaaaaaagagaaaaagaaagcatctaagaacttgaaaaactacgaattagaaaagaccaaatatgtatttcttgcattgaccaatttatgcaagtttatatatatgtaaatgtaagtttcacgaggttctactaaactaaaccacccccttggttagaagaaaagagtgtgtgagaacaggctgttgttgtcacacgattcggacaattctgtttgaaagagagagagtaacagtacgatcgaacgaactttgctctggagatcacagtgggcatcatagcatgtggtactaaaccctttcccgccattccagaaccttcgattgcttgttacaaaacctgtgagccgtcgctaggaccttgttgtgtgacgaaattggaagctgcaatcaataggaagacaggaagtcgagcgtgtctgggttttttcagttttgttctttttgcaaacaaatcacgagcgacggtaatttctttctcgataagaggccacgtgctttatgagggtaacatcaattcaagaaggagggaaacacttcctttttctggccctgataatagtatgagggtgaagccaaaataaaggattcgcgcccaaatcggcatctttaaatgcaggtatgcgatagttcctcactctttccttactcacgagtaattcttgcaaatgcctattatgcagatgttataatatctgtgcgtggcgcgtccggctgtctgccatgctgcccggtgtaccgacataaccgccggtggcatagccgcgcatacgcgccatttccttccatcttgtgattcatgctatccatcttttttgagtatccaattaacgaagacgttaccagctgattgaaggttctcaaagtgactgtactccatgttttcttatcatccatgtagttatttttcaaactgcaaattcaagaaaaagccacgcgtgtgcaccttttttttccccttccagtgcattatgcaatagacagcacgagtctttgaaaaagtaacttataaaactgtatcaatttttaaacctaaatagattcataaactattcgttaatataaagtgttctaaactatgatgaaaaaataagcagaaaagactaataattcttagttaaaagcactccctagttcattaatccatttgctagtcttgctcttagatccttcctcaatatcttccctgatggagctttaggaatagagtcagtgaagaacactttgttgattctcttataaaacacaacctgttttgacacgaattgcttgatttcatcttcggatatatttgaatctttcgatctcaccacaaacgcaacaggaacctcaccagcatcttcttccttcatggcgacgacagcaacatcattgatttctggatgacctatgaggagagactctagctcagctggagccacttgaaatcctttgtacttgatgagttctttcaatctatccacaatgaaaagctcgtcgtcatcatcgataaatccgacgtctccagtgtgaagccaaccatctttatcgatcgtcgatgccgtggccaaggggtcattgagatagcctttcatgatttggttgccacggatgcatatttcgccgggtttgttcctaggcaaagaatctcctgtgtctggatcaagtatcttcatctcggcgttcctcaccaccgtaccacatgctcctgacttcactggaaacggctctttagcaaaccctaacgacattgctagcaccggacctgcttctgtcatcccatagccctgaccaagcttggcgttaggaaacttagcactaatagcatcttcaagctccttaccaagaggagctgctccagacttaaccatcctaaccgagctcagatcatacttctccgtctccggcgacttcgcgatagctaaaacgatcggtggcacgaccatagccaccgtgactttacacctttgtatctgctctaacaagagagtgatttcgaacttaggcattatcaagatcgtggcaccaactctgagactacagagcatgatggagttgagagcgtatatatggaacataggcaagacacagaggatcacgtcgtctctgttgaagtaaagattcggattctcgccgtcgacttgctgcgccacgctcgtgactagacctttgtgtgttagcatcactcctttggggagacccgtcgtgccggatgagaaaggaagcgccacgacgtcttctggcgaaatcttctccggtattgagtccactcgtggttcttcggactgagttaactcggagaaacggaggcagttttcggggatggcgtcggagtcggtggtgacgatcaaaacgccgtcgttttggaggttcttgattttatcgacgtaacgggattgagtgacgatgagtttcgccgcggaggctttggcttgtttagaaatctccgccggagtgaagaacgggttcgcggaggtggtgattgcgccgatgaaggaggcggcaaggaaagtgaggactacttcaggagagttcgggaggaggatcattacaacgtcgtgttgcttcacgccgaggttatgaagaccggcggcgagtttccgagatgttacgtggacatcggcgtaggtgtatacttcgccggtgggaccgttgatcaagcatggcttagcggcgaactctgagatattttcgaagatgtagtcgtggagtgggaggtggttagggatgtatatatcaggcaatctcgatcggaaaatgacgtcattactacactgtttctgatcattctgatcattgactatcacatcttgtgtcgtcattttagctttttgtaattaaaacttagattagattgctatgctttctttctaatgagcaagaagtaaaaaaagttgtaatagaacaagaaaaatgaaactgaaacttgagaaattgaagaccgtttattaacttaaatatcaatgggaggtcatcgaaagagaaaaaaatcaaaaaaaaaaattttcaagaaaaagaaacgtgataaaaatttttattgcctttttcgacgaagaaaaagaaacgaggcggtctcttttttcttttccaaacctttagtacgggtaattaacgacaccctagaggaagaaagaggggaaatttagtatgctgtgcttgggtgttttgaagtggtacggcgatgcgcggagtccgagaaaatctggaagagtaaaaaaggagtagaaacattttgaagctaggcgcgtcagccggtaaagattccccacgccaatccggctggttgcctccttcgtgaagacaaactcacgcgcctccaaaatgagctatcaaaaacgatagatcgattaggatgactttgaaatgactccgcagtggactggccgttaatttcaagcgtgagtaaaatagtgcatgacaaaagatgagctaggcttttgtaaaaatatcttacgttgtaaaattttagaaatcattatttccttcatatcattttgtcattgaccttcagaagaaaagagccgaccaataatataaataaataaataaaaataatattccattatttctaaacagattcaatactcattaaaaaactatatcaattaatttgaattaaccgcggttagcagattggaataggtgcaccattccactctttcaagcaatccataagtggatctatcaactttccctcgcacatagctgtgaataccttgtcaaattcttcacctgggctaacgactttttcaccagttagtaatttggttcccaactcttctctaacgaatctgtacaaagggtacgacctacactctttgattctatttggtataggggcagtaccatttccgtatgcggctctagcagcttcgacttcctttggtaaaactgccttcagttcttcttcaaaggcacctatcttttggaatattgaagtaacggcatttttctcagtttcaccattggataaagcgtgatctacaataacttgtctcaatctctgcatcaatggataagtagcgctacatggatcgtcaacgtaagtaaatacttgttctctatctacaacttttaataaatctttttcacagaatcttgatgggtgcaattcaccattgatacctgtagttagaaccttttttgcaacctgtgatacggtatttttcactgtctgtctcaaattctcttccaagtgtctcaaatctacggcctggcatatacccactaaaaatgttgtggacattaatttaaggatatcaacggcctcgcttgtttttcttgatgaaatcaggcccaaagaattaacatcctgattgtgttgttcggctgattgtacatgagaggttactgggttggctagatattgcagctctgaacaatagcttgccattgctatctcagcacctttgaaaccataatcaagactagggttagaagatgcggtcagattcgaaggcaaaccgttattgtagaagtcattgaccaattcagaaaattgggcaaacattaatttgccaattgcggctatggcaagcctggtattatccatactgactcctatgggtgtaccctggaaattgcctccatgtattgccttattcctcgacacatcaataagtggattatcgttaacagagttgatctctctttctatagactttgtagcttgtctaattacttcaatttgagggccaagccattgtggggatgtccttaaagcatatctatcttgtttgggtttttgcaaagggtccatttcatgaaccttctgggctaacttcatgtagctagagccgtccaaaatgtgctccatgatagctgctgcttcaatttgtcctgggtgatgttttaacctgtgggtcaagtgatcagtaaactcaggttttccactcatgacttcggcaaaaattgcggacaaaacttcggccaaaactgcttgtacgttagcttcaaacaacaccatggatgccataccgctgccgacagcggtgccattcaccagggctaaaccttccttgggttgcaaatcaaagaaaccagttgaaataccagctttctcaaatgcttccttagcggttaaggattctccgtctggaccagtggcctttgaattaggtcttcccgttaataagcctgcgatatatgaaaggggaaccaaatcaccgctggcagttattgttcctcttaagggcaacgaaggagaaatgttgtggttcaatagtgaagtgatggcctcaagaatttcaaaccttattccagagtaaccttgcaacaaagtgttcaccctaacaagcatagcagctcttgttgccgattggggtaatgtatggcaagtttcctttgtattaccgaaaataccggcgttaaggaatctgatcagttctgtttgcaaagcagtgccatttttagttcttctatgagaggtagcaccaaagcctgtggtaacgccataggaatctgtgcccttgttcatactttccatgacccaatctgatgaagccttaactccggctctacttgtttctgcaagttctaccttcactgaaccgccaacggtcgaaatagcagctacctgtcctatcgtcaatgtctcgccgcctagatttacgactggtcttctgtattcctcaaccatcttcttaacttcatccagatggctacctttcatctggtcagctgccagaccccaattcaaaggatctgcaagagtttttgtcgttacggccaccttggtcttttcaccaccaccgcatagcattgcttcaatttggtccattttaagctttttgatagatttgactgtgttattttgcgtgaggttatgagtagaaaataataattgagaaaggaatatgacaagaaatatgaaaataaagggaacaaacccaaatctgattgcaaggagagtgaaagagccttgtttatatatttttttttcctatgttcaacgaggacagctaggtttatgcaaaaatgtgccatcaccataagctgattcaaatgagctaaaaaaaaaatagttagaaaataaggtggtgttgaacgatagcaagtagatcaagacaccgtctaacagaaaaaggggcagcggacaatattatgcaattatgaagaaaagtactcaaagggtcggaaaaatattcaaacgatatttgcataaaatcctcaattgattgattattccatagtaaaataccgtaacaacacaaaattgttctcaaattcataaattattcattttttccacgagcctcatcacacgaaaagtcagaagagcatacataatcttttaaatgcataggttatgcattttgcaaatgccaccaggcaacaaaaatatgcgtttagcgggcggaatcgggaaggaagccggaaccaccaaaaactggaagctacgtttttaaggaaggtatgggtgcagtgtgcttatctcaagaaatattagttatgatataaggtgttgaagtttagagataggtaaataaacgcggggtgtgtttattacatgaagaagaagttagtttctgccttgcttgtttatcttgcacatcacatcagcggaacatatgctcacccagtcgcatggcgcgtaccacggtgaacaatccccgctggctcatatttgccgccggttcccgtaaatcctccggtacgcgccgggccgtatacttacatatagtagatgtcaagcgtaggcgcttcccctgccggctgtgagggcgccataaccaaggtatctatagaccgccaatcagcaaactacctccgtacattcatgttgcacccacacatttatacacccagaccgcgacaaattacccataaggttgtttgtgacggcgtcgtacaagagaacgtgggaactttttaggctcaccaaaaaagaaagaaaaaatacgagttgctgacagaagcctcaagaaaaaaaaaattcttcttcgactatgctggaggcagagatgatcgagccggtagttaactatatatagctaaattggttccatcaccttcttttctggtgtcgctccttctagtgctatttctggcttttcctatttttttttttccatttttctttctctctttctaatatataaattctcttgcattttctatttttctctctatctattctacttgtttattcccttcaaggtttttttttaaggagtacttgtttttagaatatacggtcaacgaactataattaactaaacaagcttaaaatgatggattttgttttgttagaaaaagctcttcttggtttgttcattgcaactatagtagccatcacaatctctaagctaaggggaaagaaacttaagttgcctccaggcccaatccctgtcccagtgtttggtaattggttacaagttggcgacgacttaaaccagaggaatttggtagagtatgctaaaaagttcggcgacttatttctacttaggatgggtcaaagaaacttggtcgtggtttcatcccctgacttagcaaaagacgtactacatacccagggtgtcgagttcggaagtagaactagaaatgttgtgtttgatattttcacaggcaaaggtcaagatatggtttttaccgtatacagcgagcactggaggaaaatgagaagaataatgactgtcccattctttacaaacaaagtggttcaacagtataggttcggatgggaggacgaagccgctagagtagtcgaggatgttaaggcaaatcctgaagccgctaccaacggtattgtgttgaggaatagattacaacttttgatgtacaacaatatgtatagaataatgtttgacaggagatttgaatctgttgatgatccattattcctaaaacttaaggcattgaatggcgagagatcaaggttagctcaatcctttgaatacaacttcggtgacttcattcctatattgaggccattcttgagaggatatcttaagttgtgtcaggaaatcaaggacaaaaggttaaagctattcaaggactacttcgtcgacgagagaaaaaagttggagagtatcaagagcgtaggtaataactccttaaagtgcgccatagatcatattatcgaggcacaagaaaaaggcgagataaacgaggataacgtgttatacatcgtcgagaatatcaacgtggctgccattgaaactacactttggtctattgaatggggtatagcagaactagtgaataaccctgaaatccagaaaaaattgagacacgaattagacaccgtacttggagctggtgttcaaatttgtgaaccagatgttcaaaaattgccttatctacaggccgtgataaaagagactttaaggtacaggatggcaattccattgttagtcccacatatgaatcttcacgaagccaaattggccggctatgatatccctgcagagagcaaaattttggtaaacgcttggtggttagccaataatccagcacattggaacaaacctgatgagtttagaccagaaagatttttggaggaagaatccaaggtcgaggctaatggaaacgactttaagtacatccctttcggtgttggcagaagatcttgcccaggtataattcttgctttaccaatccttggaatagtaattggtaggttggttcaaaacttcgagttacttccacctccaggccaaagcaaaatagatacagccgaaaaaggtggacagttttcattgcaaatcctaaagcattccactattgtgtgtaaacctagaagttcttaaccgcggacaaatcgctcttaaatatatacctaaagaacattaaagctatattataagcaaagatacgtaaattttgcttatattattatacacatatcatatttctatatttttaagatttggttatataatgtacgtaatgcaaaggaaataaattttatacattattgaacagcgtccaagtaactacattatgtgcactaatagtttagcgtcgtgaagactttattgtgtcgcgaaaagtaaaaattttaaaaattagagcaccttgaacttgcgaaaaaggttctcatcaactgtttaaaaggaggatatcaggtcctatttctgacaaacaatatacaaatttagtttcaaaggcgcgttgcaaaatggaatttcgccgcagcggcctgaatggctgtaccgcctgacgcggatgcgccacgcgccgcatgccggtagaggtgtggtcaataagagcgacctcatgctatacctgagaaagcaacctgacctacaggaaagagttactcaagaataagaattttcgttttaaaacctaagagtcactttaaaatttgtatacacttattttttttataacttatttaataataaaaatcataaatcataagaaattcgcttatttagaagtgtcaacaacgtatctaccaacgatttgacccttttccatcttttcgtaaatttctggcaaggtagacaagccgacaaccttgattggagacttgaccaaacctctggcgaagaagtccaaagctctagatcaatttaggcctgcggccgcggttaccagacatcttcttggtatctacctgaagtcttgagcatcttgattagctctgttgcttcatcagtggtaatggatttaccacgggataagatgccaaccaatgcggttgacacacccttggccataccctttgcatcaccacagacgtagataaatgcaccgttgttaatcatttcaaatacttggtcttcgtaatcctttaatttatcttgaacataaacttttttggtgtttggcaacctggaatgggccacgaccatttcgaacgaaccatccaattttttggcgtattctggccattcgtcctggtacaagaaatcatcagtgttacgggatccataaaacagtatatgcttacctagcgaaacgttgttaccgcccttcttttgtgattcgaggaacgcgacacgctctctgataaacccacggaatggggcaacaccggtacctggaccgatcatgataactggggtggaagggttggaaggcaatctgaagttagaacgacgaacgtggacgggcaatttgtaattggcgaaaagtttacgtgggccatttaaatcgtagtgaacaggtaggttagtttcggcaatgttaacattgttttgagccaattgaatgtttcttaacaagttagtcgtaacaccaacaactggaggagcatcaggcaattctgggttaggaaagttttccacaatggaggtgacatggacggtttgcttttcagacagagaagaggaagagatagagtagtaacgaggagtcatttggggaactgattcgaccaagaattgcatgggtacggtgtcccatttggcgccatcagacaaatatttcagagcatctgcgatgttgaaatatttggaggttatctcgacggcgaattggtccttgtctttcgaaagcagagtcaatttttccttgacgtcagcgttgggggcgaactgaatcaaagatgaaaacaattgtctggagacaggtcctgtaatttccaaatagtgtttaatagcagcgccaatagtagttggcgttgggaagggcactttgacggtgggatccaggggcttcaagtcaaaaatggtttcagggtccaggttgaatatggataagaactgttcgaccttttccaatgggttggaaggccaaacagcaagatggtcaccagtggagtacttgatgttagagccggacaagtcaaattcagagtggatgcaattacggtcattggaagagaacagttcgcgagatttcacgatgggtgcaatatacggttgagacaaatcgaagggacccaattggatgccgtctgcgttgcggttcaactgatgcgagggcaaatagtgagcagagggttcaccaagcgacatggagtcagtgatttcgttcaacacagtgtactggaattgagaggtgaacttggcttcctgttcgtccaaatgcagttcgtctttcaaaacctccaggatggagtccttccaggccatgtaatcttcgtctgtagttcctgcaccatcatcagcttcaccgagcttgcctagtctgatagcgcccgcagcggagagatgcttctcggccttcttggcggcaccattaaagaattcataagtagaatttcccagaccaaacatattatacctcaggttcgatagtgcacccgcttccgcattacaaataaagtcttcaaagttgaccgccccgtcggggaagtctccttcaccatatgtagagataaaaatcgagactatgacgggcacatcgtttagcgactcaaagtcgtagttctcaacatctgcgcacatcacgtttaggttgaacttggccaccagctccttggaaaactttttggcgtaatcctcggcagtcccagtctgcgacgcatacaacaccaagtagttcttgttgttttcggtcaccacctgagcaatgtctctgttgcccgagctgacagctgtgatatctccgtcatcggacatcagcagttccttgatggagtttctctttacgtacagtagcacggcaagcactagccccgccaggacagtgaagtcggtgttgtctattccaaacggcattttactagtaagctttgtgatgatgttttatttgttttgattggtgtcttgtaaatagaaacaagagagaataataaacaagttaagaataaaaaaccaaaggatgaaaaagaatgaatatgaaaaagagtagagaataactttgaaaggggaccatgatataactggaaaaaagaggttcttggaaatgaaaagttaccaaagagtatttataattcagaaaaaaaagccaacgaatatcgttttgatggcgagcctttttttttttttaggaagacactaaaggtacctagcatcatatgggaaggaaaggaaatcacttggaagacatcacaagcattcatttaccaagagaaaaaatatgcattttagctaagatccattgaacaaagcactcactcaactcaactgaatgaacgaaagaagaaagaacagtagaaaacactttgtgacggtgcggaacacatttacgtagctatcatgctgaattctactatgaaaatctcccaatctgtcgatggcaaaacgacccacgtggcagagttgggtcaagtgccagtttctggattaagtaacagatacagacatcacacgccatagaggaatcccgccgttgcgagagatggaaaacaatagagccgaaattgtggaagcccgatgtctgggtgtacattttttttttttctttctttctctttcaataatctttcctttttccatttagcttgccggaaaaactttcgggtagcgaaaatctttctgccggaaaaattagctatttttttcttccttattatttttttagttctgaagtttgaccagggcgctaccctgaccgtatcacaaccgacgatccggggtcatggcggctatttttttttttttttttttttccttgtgattgtttatttacatttggatcaattctaacaaaaaaaaaataaggggggaaaaataattcacctctttttaatattgttttgtactgagattgatctccaaaatagtagcattggcgcgtgccaccaacagccccgccaatggcgctgccgatactcccgacaatccccaccattgcctg

SEQ ID NO: 10 - DNA, 24945 bp, pPHLOZ Multi-Expression Plasmid
acgcgcctccaactggcaccgctggcttgaacaacaataccagccttccaacttctgtaaataacggcggtacgccagtgccaccagtaccgttacctttcggtatacctcctttccccatgtttccaatgcccttcatgcctccaacggctactatcacaaatcctcatcaagctgacgcaagccctaagaaatgaataacaatactgacagtactaaataattgcctacttggcttcacatacgttgcatacgtcgatatagataataatgataatgacagcaggattatcgtaatacgtaatagttgaaaatctcaaaaatgtgtgggtcattacgtaaataatgataggaatgggattcttctatttttcctttttccattctagcagccgtcgggaaaacgtggcatcctctctttcgggctcaattggagtcacgctgccgtgagcatcctctctttccatatctaacaactgagcacgtaaccaatggaaaagcatgagcttagcgttgctccaaaaaagtattggatggttaataccatttgtctgttctcttctgactttgactcctcaaaaaaaaaaaatctacaatcaacagatcgcttcaattacgccctcacaaaaacttttttccttcttcttcgcccacgttaaattttatccctcatgttgtctaacggatttctgcacttgatttattataaaaaagacaaagacataatacttctctatcaatttcagttattgttcttccttgcgttattcttctgttcttctttttcttttgtcatatataaccataaccaagtaatacatattcaaaaagcttaaaatgggtgatgtcattgtcttgtatgcttctccaggtatgggtcatatagtttccatggttgaattgggtaaattcatcgttcatagatacggtccacacaagttctctattactatcttgtacacctgtggttccatcgttgatactgcttctattccagtttacatcagaagaatctcccattcccatccattcatctcattcagacaattcccaagagttaccaacaacatcaccagaaacatttccgttccagctattaccttcgacttcatcagacaaaatgatccacatgttagatccgccttgcaagaaatttcaaagtctgctactgttagagccttcatcattgatttgttctgtacttccgctttgccaatcggtaaagaattcaacattccaacctactacttcagaacttctggtgctgctattttggctgctttcttgtacttgccaaagatcgatgaacaaactaagaccaccgaatctttcaaggatttgagagataccgttttcgaatttccaggttggaaatctccattgaaggctactcatatggttcaattggttttggatagaaacgatccagcctactctgatatgatctacttctgttctcatttgccaaagtccaacggtattatcgttaacaccttcgaagaattggaaccaccatctgttttacaagctattgctggtggtttgtgtgttccagatggtccaactccaccagtttattatgttggtccattgatcgaagaagaaaaagaattgtccaaggatgctgatgctgccgaaaaagaagattgcttgtcttggttggataagcaaccatctagatccgttttgttcttgtgttttggttccatgggttcttttccagctgctcaattgaaagaaattgccaatggtttggaagcctctggtcaaagatttttgtgggttgttaagaagccaccagtcgaagaaaaatccaaacaagttcatggtgttgacgacttcgatttgaaaggtgttttgccagaaggtttcttggaaagaactgctgatagaggtatggttgtaaaatcttgggctccacaagttgtcgtcttgaagaaagaatctgttggtggtttcgttactcattgtggttggaattctgttttggaagctgttgttgctggtgttccaatgattgcttggccattatatgctgaacaacacatgaatagaaacgtcttggttaccgatatggaaatcgctattggtgtcgaacaaagagatgaagaaggtggttttgtttccggtgaagaagttgaaagaagagttagagaattgatggaatccgaaggtggtagagttttgagagaaagatgtaaaaagttgggtgaaatggcttctgctgctttaggtgaaactggttcttctactagaaacttggtcaacttcgtttcctccattacctgaccgcggatttaactccttaagttactttaatgatttagtttttattattaataattcatgctcatgacatctcatatacacgtttataaaacttaaatagattgaaaatgtattaaagattcctcagggattcgatttttttggaagtttttgtttttttttccttgagatgctgtagtatttgggaacaattatacaatcgaaagatatatgcttacattcgaccgttttagccgtgatcattatcctatagtaacataacctgaagcataactgacactactatcatcaatacttgtcacatgaggcgcgtcttaagcagaatttctgtcatcatggacagcacggaacgggtgaagctgcgccagttctgacgcgtccagtatcccagcagatacgggatatcgacatttctgcaccattccggcgggtataggttttattgatggcctcatccacacgcagcagcgtctgttcatcgtcgtggcggcccataataatctgccggtcaatcagccagctttcctcacccggcccccatccccatacgcgcatttcgtagcggtccagctgggagtcgataccggcggtcaggtaagccacacggtcaggaacgggcgctgaataatgctctttccgctctgccatcacttcagcatccggacgttcgccaattttcgcctcccacgtctcaccgagcgtggtgtttacgaaggttttacgttttcccgtatcccctttcgttttcatccagtctttgacaatctgcacccaggtggtgaacgggctgtacgctgtccagatgtgaaaggtcacactgtcaggtggctcaatctcttcaccggatgacgaaaaccagagaatgccatcacgggtccagatcccggtcttttcgcagatataacgggcatcagtaaagtccagctcctgctggcggatgacgcaggcattatgctcgcagagataaaacacgctggagacgcgttttcccgtctttcagtgccttgttcagttcttcctgacgggcggtatatttctccagcttggcctatgcggccctgtcagaccaagtttacgagctcgcttggactcctgttgatagatccagtaatgacctcagaactccatctggatttgttcagaacgctcggttgccgccgggcgttttttattggtgagaatccaagcactagggacagtaagacgggtaagcctgttgatgataccgctgccttactgggtgcattagccagtctgaatgacctgtcacgggataatccgaagtggtcagactggaaaatcagagggcaggaactgctgaacagcaaaaagtcagatagcaccacatagcagacccgccataaaacgccctgagaagcccgtgacgggcttttcttgtattatgggtagtttccttgcatgaatccataaaaggcgcctgtagtgccatttacccccattcactgccagagccgtgagcgcagcgaactgaatgtcacgaaaaagacagcgactcaggtgcctgatggtcggagacaaaaggaatattcagcgatttgcccgagcttgcgagggtgctacttaagcctttagggttttaaggtctgttttgtagaggagcaaacagcgtttgcgacatccttttgtaatactgcggaactgactaaagtagtgagttatacacagggctgggatctattctttttatctttttttattctttctttattctataaattataaccacttgaatataaacaaaaaaaacacacaaaggtctagcggaatttacagagggtctagcagaatttacaagttttccagcaaaggtctagcagaatttacagatacccacaactcaaaggaaaaggacatgtaattatcattgactagcccatctcaattggtatagtgattaaaatcacctagaccaattgagatgtatgtctgaattagttgttttcaaagcaaatgaactagcgattagtcgctatgacttaacggagcatgaaaccaagctaattttatgctgtgtggcactactcaaccccacgattgaaaaccctacaaggaaagaacggacggtatcgttcacttataaccaatacgctcagatgatgaacatcagtagggaaaatgcttatggtgtattagctaaagcaaccagagagctgatgacgagaactgtggaaatcaggaatcctttggttaaaggctttgagattttccagtggacaaactatgccaagttctcaagcgaaaaattagaattagtttttagtgaagagatattgccttatcttttccagttaaaaaaattcataaaatataatctggaacatgttaagtcttttgaaaacaaatactctatgaggatttatgagtggttattaaaagaactaacacaaaagaaaactcacaaggcaaatatagagattagccttgatgaatttaagttcatgttaatgcttgaaaataactaccatgagtttaaaaggcttaaccaatgggttttgaaaccaataagtaaagatttaaacacttacagcaatatgaaattggtggttgataagcgaggccgcccgactgatacgttgattttccaagttgaactagatagacaaatggatctcgtaaccgaacttgagaacaaccagataaaaatgaatggtgacaaaataccaacaaccattacatcagattcctacctacataacggactaagaaaaacactacacgatgctttaactgcaaaaattcagctcaccagttttgaggcaaaatttttgagtgacatgcaaagtaagtatgatctcaatggttcgttctcatggctcacgcaaaaacaacgaaccacactagagaacatactggctaaatacggaaggatctgaggttcttatggctcttgtatctatcagtgaagcatcaagactaacaaacaaaagtagaacaactgttcaccgttacatatcaaagggaaaactgtccatatgcacagatgaaaacggtgtaaaaaagatagatacatcagagcttttacgagtttttggtgcattcaaagctgttcaccatgaacagatcgacaatgtaacgcggccgcagccaatcaattcttgcggagaactgtgaatgcgcaaaccaacccttggcagaacatatccatcgcgtccgccatctccagcagccgcacgcggcgcatcgggggggggggggggggtttcaattcatcattttttttttattcttttttttgatttcggtttccttgaaatttttttgattcggtaatctccgaacagaaggaagaacgaaggaaggagcacagacttagattggtatatatacgcatatgtagtgttgaagaaacatgaaattgcccagtattcttaacccaactgcacagaacaaaaacctgcaggaaacgaagataaatcatgtcgaaagctacatataaggaacgtgctgctactcatcctagtcctgttgctgccaagctatttaatatcatgcacgaaaagcaaacaaacttgtgtgcttcattggatgttcgtaccaccaaggaattactggagttagttgaagcattaggtcccaaaatttgtttactaaaaacacatgtggatatcttgactgatttttccatggagggcacagttaagccgctaaaggcattatccgccaagtacaattttttactcttcgaagacagaaaatttgctgacattggtaatacagtcaaattgcagtactctgcgggtgtatacagaatagcagaatgggcagacattacgaatgcacacggtgtggtgggcccaggtattgttagcggtttgaagcaggcggcagaagaagtaacaaaggaacctagaggccttttgatgttagcagaattgtcatgcaagggctccctatctactggagaatatactaagggtactgttgacattgcgaagagcgacaaagattttgttatcggctttattgctcaaagagacatgggtggaagagatgaaggttacgattggttgattatgacacccggtgtgggtttagatgacaagggagacgcattgggtcaacagtatagaaccgtggatgatgtggtctctacaggatctgacattattattgttggaagaggactatttgcaaagggaagggatgctaaggtagagggtgaacgttacagaaaagcaggctgggaagcatatttgagaagatgcggccagcaaaactaaaaaactgtattataagtaaatgcatgtatactaaactcacaaattagagcttcaatttaattatatcagttattacccggccgggaatctcggtcgtaatgatttttataatgacgaaaaaaaaaaaattggaaagaaaaccccccccccccccccgcagcgttgggtcctggccacgggtgcgcatgatcgtgctcctgtcgttgaggacccggctaggctggcggggttgccttactggttagcagaatgaatcaccgatacgcgagcgaatgtggcggccgcacgcgttcatcgtccacctccggagaacaggccaccatcacgcatctgtgtctgaatttcatcacgacgcgccttaagggcaccaataactgccttaaaaaaattacgccccgccctgccactcatcgcagtactgttgtaattcattaagcattctgccgacatggaagccatcacagacggcatgatgaacctgaatcgccagcggcatcagcaccttgtcgccttgcgtataatatttgcccatggtgaaaacgggggcgaagaagttgtccatattggccacgtttaaatcaaaactggtgaaactcacccagggattggctgagacgaaaaacatattctcaataaaccctttagggaaataggccaggttttcaccgtaacacgccacatcttgcgaatatatgtgtagaaactgccggaaatcgtcgtggtattcactccagagcgatgaaaacgtttcagtttgctcatggaaaacggtgtaacaagggtgaacactatcccatatcaccagctcaccgtctttcattgccatacggaattccggatgagcattcatcaggcgggcaagaatgtgaataaaggccggataaaacttgtgcttatttttctttacggtctttaaaaaggccgtaatatccagctgaacggtctggttataggtacattgagcaactgactgaaatgcctcaaaatgttctttacgatgccattgggatatatcaacggtggtatatccagtgatttttttctccattttagcttccttagctcctgaaaatctcgataactcaaaaaatacgcccggtagtgatcttatttcattatggtgaaagttggaacctcttacgtgccgatcaacgtctcattttcgccaaaagttggcccagggcttcccggtatcaacagggacaccaggatttatttattctgcgaagtgatcttccgtcacaggtattggaccaccctgtgggtttataagcgcgctgctggcgtgtaaggcggtgacggcgaaggaagggtccttttcatcacgtgctataaaaataattataatttaaattttttaatataaatatataaattaaaaatagaaagtaaaaaaagaaattaaagaaaaaatagtttttgttttccgaagatgtaaaagactctagggggatcgccaacaaatactaccttttatcttgctcttcctgctctcaggtattaatgccgaattgtttcatcttgtctgtgtagaagaccacacacgaaaatcctgtgattttacattttacttatcgttaatcgaatgtatatctatttaatctgcttttcttgtctaataaatatatatgtaaagtacgctttttgttgaaattttttaaacctttgtttatttttttttcttcattccgtaactcttctaccttctttatttactttctaaaatccaaatacaaaacataaaaataaataaacacagagtaaattcccaaattattccatcattaaaagatacgaggcgcgtgtaagttacaggcaagcgatccgtcctaagaaaccattattatcatgacattaacctataaaaataggcgtatcacgaggccctttcgtctcgcgcgtttcggtgatgacggtgaaaacctctgacacatgcagctcccggagacggtcacagcttgtctgtaagcggatgccgggagcagacaagcccgtcagggcgcgtcagcgggtgttggcgggtgtcggggctggcttaactatgcggcatcagagcagattgtactgagagtgcaccacggcgcgtggcacccttgcgggccatgtcatacaccgccttcagagcagccggacctatctgcccgttacgcgccagcttgcaaattaaagccttcgagcgtcccaaaaccttctcaagcaaggttttcagtataatgttacatgcgtacacgcgtctgtacagaaaaaaaagaaaaatttgaaatataaataacgttcttaatactaacataactataaaaaaataaatagggacctagacttcaggttgtctaactccttccttttcggttagagcggatgtggggggagggcgtgaatgtaagcgtgacataactaattacatgatatcgacaaaggaaaagggggacggatctccgaggcctcggacccgtcgggccgccgtcggacgtgccgcggtcatgcagaagctgcagtagggacagggactgggacactatgcaacactaaggtttctacagtcaagcctggtccgaatccaaacaacactccccaatcttttccttctcctgtggttgccaatccgtctttagcagaacttttcctcatgacatctaacacaaacaacacagaggcactagacatatttccgtattcagataacacttccctagaagccctcattctcttcttatccaatcctactctatcttcaactctgtctaaaatggcagggccaccaggatgtgcaatccagaaaattgaattccagttatgaatacctaaaggttcaaaggcatcctccaaagcctgttcaatgttctctgaaattaaaccaggaacatcttttaataaatgtatagttaaaccagcttctgttaaatggccatctatggcaccttctgattctggtaatatagtctgagaagctgataccaactggaaaactggttgttcgtctaattggtctgggtcagcgcctataattgcagcagcggcaccatcaccgaacaaggcatgacctaccaaggaatctaaatgactcttgcatggacctctgaaggccatagcagttatctcggaacaaacgactaacactctggcacctctattattttcagcgatatcttttgccaatctcaaaacagttgcaccaccaaagcaaccttgttggtacatcattaaccttttgactgtaggggacaaacctaacaactttgttaattggtaatcagcaccgggcatgtcaacgccggatgttgtgcaaaataccaaatgagtaatcttagacaagggttggccccactccttaatggccttctcagctgcaccttggcccaatttgggaacttcaactaatgcgatggcgtgtctagcatccaatgaggtctccatgtgtgcacagatctttgggttcttgatcaatatttcctcggtcaagtgcatgtgtctctttctaatcattgatttgtcacacattctttgaaacttctcctttaaatctgccaagtgctcacttttagtaaccctaaaataataatctggataggtagcttgataaacacaattagctggaacggcagtaccgattgctaaaactgtagctaaaccttcagccctctgtgccattctaacttctttcaatcttactgcagccattttaagctttttgtttgtttatgtgtgtttattcgaaactaagttcttggtgttttaaaactaaaaaaaagactaactataaaagtagaatttaagaagtttaagaaatagatttacagaattacaatcaatacctaccgtctttatatacttattagtcaagtaggggaataatttcagggaactggtttcaaccttttttttcagctttttccaaatcagagagagcagaaggtaatagaaggtgtaagaaaatgagatagatacatgcgtgggtcaattgccttgtgtcatcatttactccaggcaggttgcatcactccattgaggttgtgtccgttttttgcctgtttgtgcccctgttctctgtagttgcgctaagagaatggacctatgaactgatggttggtgaagaaaacaatattttggtgctgggattctttttttttctggatgccagcttaaaaagcgggctccattatatttagtggatgccaggaataaactgttcacccagacacctacgatgttatatattctgtgtaacccgccccctattttgggcatgtacgggttacagcagaattaaaaggctaattttttgactaaataaagttaggaaaatcactactattaattatttacgtattctttgaaatggcagtattgataatgataaactcgaactgggcgcgtcgtgccgtcgttgttaatcaccacatggttattctgctcaaacgtcccggacgcctgcgaacgcgccgaaggaaaatgagaaatatcgagggagacgattcagaggagcaggacaaactataaccgactgtttgttggaggatgccgtacataacgaacactgctgaagctaccatgtctacagtttagaggaatgggtacaactcacaggcgagggatggtgttcactcgtgctagcaaacgcggtgggagcaaaaagtagaatattatcttttattcgtgaaacttcgaacactgtcatctaaagatgctatatactaatataggcatacttgataatgaaaactataaatcgtaaagacataagagatccgcggtcaaaatacaaatggaatcaagaatgctcttctggtatgatactttttgtttttcttttgagcccatgcgtacatttgagctgttgaaacagtcaaaaataaaacggcaaataaattgaacttgaacacaaaagtaaaccaaatccaagaccaaacttcaaaagtatagttgggagcaacaaaaagattgaaaataccttgattcaatgggacacggatcttagcgttaccatgcttcttttgatagtcaccccataggcgcaatttaatgtggcaataaaagttccatagttctgaaagcacgaaaagaccaattaatgtactcaagtcatccaatttcaaatatgaatagtatttgaataacttagcattcccaaaggggaagccgtagccaaagtaaccgaatgaaatgagaccgcttagaacccagtaatggaaacaatttttgaacaggttgaaaattggcatagtagctaaagagaattggtgaacaaataaggtttcaaataatctctttccataatgtcctaaaattaaaaaatatgcaaccctgtttaaaaatggattatagtcggagctagcactgtgccatctatcaacaactgtgggaatggtagatagataataaaaaagggagtgaaccaagactggacccaaatactcacaaaagaagactaatctccatgaaatttggggacccaaatctttgatgaagaattccattgagtcatcagcctcttcttgaaaaaacgattctgaaataaccggaacttgtttagattcctttttgtaggttaatcttatcctgtacttgctgatattgtggttattagcagagatttttttcaaaacatcatctaaagtaggctttttggataagtcaatttcagtgtcccttaaccctttagagcggctttttatggtgataggcattttaagctttgttttatatttgttgtaaaaagtagataattacttccttgatgatctgtaaaaaagagaaaaagaaagcatctaagaacttgaaaaactacgaattagaaaagaccaaatatgtatttcttgcattgaccaatttatgcaagtttatatatatgtaaatgtaagtttcacgaggttctactaaactaaaccacccccttggttagaagaaaagagtgtgtgagaacaggctgttgttgtcacacgattcggacaattctgtttgaaagagagagagtaacagtacgatcgaacgaactttgctctggagatcacagtgggcatcatagcatgtggtactaaaccctttcccgccattccagaaccttcgattgcttgttacaaaacctgtgagccgtcgctaggaccttgttgtgtgacgaaattggaagctgcaatcaataggaagacaggaagtcgagcgtgtctgggttttttcagttttgttctttttgcaaacaaatcacgagcgacggtaatttctttctcgataagaggccacgtgctttatgagggtaacatcaattcaagaaggagggaaacacttcctttttctggccctgataatagtatgagggtgaagccaaaataaaggattcgcgcccaaatcggcatctttaaatgcaggtatgcgatagttcctcactctttccttactcacgagtaattcttgcaaatgcctattatgcagatgttataatatctgtgcgtggcgcgtccggctgtctgccatgctgcccggtgtaccgacataaccgccggtggcatagccgcgcatacgcgccatttccttccatcttgtgattcatgctatccatcttttttgagtatccaattaacgaagacgttaccagctgattgaaggttctcaaagtgactgtactccatgttttcttatcatccatgtagttatttttcaaactgcaaattcaagaaaaagccacgcgtgtgcaccttttttttccccttccagtgcattatgcaatagacagcacgagtctttgaaaaagtaacttataaaactgtatcaatttttaaacctaaatagattcataaactattcgttaatataaagtgttctaaactatgatgaaaaaataagcagaaaagactaataattcttagttaaaagcactccctagttcattaatccatttgctagtcttgctcttagatccttcctcaatatcttccctgatggagctttaggaatagagtcagtgaagaacactttgttgattctcttataaaacacaacctgttttgacacgaattgcttgatttcatcttcggatatatttgaatctttcgatctcaccacaaacgcaacaggaacctcaccagcatcttcttccttcatggcgacgacagcaacatcattgatttctggatgacctatgaggagagactctagctcagctggagccacttgaaatcctttgtacttgatgagttctttcaatctatccacaatgaaaagctcgtcgtcatcatcgataaatccgacgtctccagtgtgaagccaaccatctttatcgatcgtcgatgccgtggccaaggggtcattgagatagcctttcatgatttggttgccacggatgcatatttcgccgggtttgttcctaggcaaagaatctcctgtgtctggatcaagtatcttcatctcggcgttcctcaccaccgtaccacatgctcctgacttcactggaaacggctctttagcaaaccctaacgacattgctagcaccggacctgcttctgtcatcccatagccctgaccaagcttggcgttaggaaacttagcactaatagcatcttcaagctccttaccaagaggagctgctccagacttaaccatcctaaccgagctcagatcatacttctccgtctccggcgacttcgcgatagctaaaacgatcggtggcacgaccatagccaccgtgactttacacctttgtatctgctctaacaagagagtgatttcgaacttaggcattatcaagatcgtggcaccaactctgagactacagagcatgatggagttgagagcgtatatatggaacataggcaagacacagaggatcacgtcgtctctgttgaagtaaagattcggattctcgccgtcgacttgctgcgccacgctcgtgactagacctttgtgtgttagcatcactcctttggggagacccgtcgtgccggatgagaaaggaagcgccacgacgtcttctggcgaaatcttctccggtattgagtccactcgtggttcttcggactgagttaactcggagaaacggaggcagttttcggggatggcgtcggagtcggtggtgacgatcaaaacgccgtcgttttggaggttcttgattttatcgacgtaacgggattgagtgacgatgagtttcgccgcggaggctttggcttgtttagaaatctccgccggagtgaagaacgggttcgcggaggtggtgattgcgccgatgaaggaggcggcaaggaaagtgaggactacttcaggagagttcgggaggaggatcattacaacgtcgtgttgcttcacgccgaggttatgaagaccggcggcgagtttccgagatgttacgtggacatcggcgtaggtgtatacttcgccggtgggaccgttgatcaagcatggcttagcggcgaactctgagatattttcgaagatgtagtcgtggagtgggaggtggttagggatgtatatatcaggcaatctcgatcggaaaatgacgtcattactacactgtttctgatcattctgatcattgactatcacatcttgtgtcgtcattttagctttttgtaattaaaacttagattagattgctatgctttctttctaatgagcaagaagtaaaaaaagttgtaatagaacaagaaaaatgaaactgaaacttgagaaattgaagaccgtttattaacttaaatatcaatgggaggtcatcgaaagagaaaaaaatcaaaaaaaaaaattttcaagaaaaagaaacgtgataaaaatttttattgcctttttcgacgaagaaaaagaaacgaggcggtctcttttttcttttccaaacctttagtacgggtaattaacgacaccctagaggaagaaagaggggaaatttagtatgctgtgcttgggtgttttgaagtggtacggcgatgcgcggagtccgagaaaatctggaagagtaaaaaaggagtagaaacattttgaagctaggcgcgtcagccggtaaagattccccacgccaatccggctggttgcctccttcgtgaagacaaactcacgcgcctccaaaatgagctatcaaaaacgatagatcgattaggatgactttgaaatgactccgcagtggactggccgttaatttcaagcgtgagtaaaatagtgcatgacaaaagatgagctaggcttttgtaaaaatatcttacgttgtaaaattttagaaatcattatttccttcatatcattttgtcattgaccttcagaagaaaagagccgaccaataatataaataaataaataaaaataatattccattatttctaaacagattcaatactcattaaaaaactatatcaattaatttgaattaaccgcggttagcagattggaataggtgcaccattccactctttcaagcaatccataagtggatctatcaactttccctcgcacatagctgtgaataccttgtcaaattcttcacctgggctaacgactttttcaccagttagtaatttggttcccaactcttctctaacgaatctgtacaaagggtacgacctacactctttgattctatttggtataggggcagtaccatttccgtatgcggctctagcagcttcgacttcctttggtaaaactgccttcagttcttcttcaaaggcacctatcttttggaatattgaagtaacggcatttttctcagtttcaccattggataaagcgtgatctacaataacttgtctcaatctctgcatcaatggataagtagcgctacatggatcgtcaacgtaagtaaatacttgttctctatctacaacttttaataaatctttttcacagaatcttgatgggtgcaattcaccattgatacctgtagttagaaccttttttgcaacctgtgatacggtatttttcactgtctgtctcaaattctcttccaagtgtctcaaatctacggcctggcatatacccactaaaaatgttgtggacattaatttaaggatatcaacggcctcgcttgtttttcttgatgaaatcaggcccaaagaattaacatcctgattgtgttgttcggctgattgtacatgagaggttactgggttggctagatattgcagctctgaacaatagcttgccattgctatctcagcacctttgaaaccataatcaagactagggttagaagatgcggtcagattcgaaggcaaaccgttattgtagaagtcattgaccaattcagaaaattgggcaaacattaatttgccaattgcggctatggcaagcctggtattatccatactgactcctatgggtgtaccctggaaattgcctccatgtattgccttattcctcgacacatcaataagtggattatcgttaacagagttgatctctctttctatagactttgtagcttgtctaattacttcaatttgagggccaagccattgtggggatgtccttaaagcatatctatcttgtttgggtttttgcaaagggtccatttcatgaaccttctgggctaacttcatgtagctagagccgtccaaaatgtgctccatgatagctgctgcttcaatttgtcctgggtgatgttttaacctgtgggtcaagtgatcagtaaactcaggttttccactcatgacttcggcaaaaattgcggacaaaacttcggccaaaactgcttgtacgttagcttcaaacaacaccatggatgccataccgctgccgacagcggtgccattcaccagggctaaaccttccttgggttgcaaatcaaagaaaccagttgaaataccagctttctcaaatgcttccttagcggttaaggattctccgtctggaccagtggcctttgaattaggtcttcccgttaataagcctgcgatatatgaaaggggaaccaaatcaccgctggcagttattgttcctcttaagggcaacgaaggagaaatgttgtggttcaatagtgaagtgatggcctcaagaatttcaaaccttattccagagtaaccttgcaacaaagtgttcaccctaacaagcatagcagctcttgttgccgattggggtaatgtatggcaagtttcctttgtattaccgaaaataccggcgttaaggaatctgatcagttctgtttgcaaagcagtgccatttttagttcttctatgagaggtagcaccaaagcctgtggtaacgccataggaatctgtgcccttgttcatactttccatgacccaatctgatgaagccttaactccggctctacttgtttctgcaagttctaccttcactgaaccgccaacggtcgaaatagcagctacctgtcctatcgtcaatgtctcgccgcctagatttacgactggtcttctgtattcctcaaccatcttcttaacttcatccagatggctacctttcatctggtcagctgccagaccccaattcaaaggatctgcaagagtttttgtcgttacggccaccttggtcttttcaccaccaccgcatagcattgcttcaatttggtccattttaagctttttgatagatttgactgtgttattttgcgtgaggttatgagtagaaaataataattgagaaaggaatatgacaagaaatatgaaaataaagggaacaaacccaaatctgattgcaaggagagtgaaagagccttgtttatatatttttttttcctatgttcaacgaggacagctaggtttatgcaaaaatgtgccatcaccataagctgattcaaatgagctaaaaaaaaaatagttagaaaataaggtggtgttgaacgatagcaagtagatcaagacaccgtctaacagaaaaaggggcagcggacaatattatgcaattatgaagaaaagtactcaaagggtcggaaaaatattcaaacgatatttgcataaaatcctcaattgattgattattccatagtaaaataccgtaacaacacaaaattgttctcaaattcataaattattcattttttccacgagcctcatcacacgaaaagtcagaagagcatacataatcttttaaatgcataggttatgcattttgcaaatgccaccaggcaacaaaaatatgcgtttagcgggcggaatcgggaaggaagccggaaccaccaaaaactggaagctacgtttttaaggaaggtatgggtgcagtgtgcttatctcaagaaatattagttatgatataaggtgttgaagtttagagataggtaaataaacgcggggtgtgtttattacatgaagaagaagttagtttctgccttgcttgtttatcttgcacatcacatcagcggaacatatgctcacccagtcgcatggcgcgtaccacggtgaacaatccccgctggctcatatttgccgccggttcccgtaaatcctccggtacgcgccgggccgtatacttacatatagtagatgtcaagcgtaggcgcttcccctgccggctgtgagggcgccataaccaaggtatctatagaccgccaatcagcaaactacctccgtacattcatgttgcacccacacatttatacacccagaccgcgacaaattacccataaggttgtttgtgacggcgtcgtacaagagaacgtgggaactttttaggctcaccaaaaaagaaagaaaaaatacgagttgctgacagaagcctcaagaaaaaaaaaattcttcttcgactatgctggaggcagagatgatcgagccggtagttaactatatatagctaaattggttccatcaccttcttttctggtgtcgctccttctagtgctatttctggcttttcctatttttttttttccatttttctttctctctttctaatatataaattctcttgcattttctatttttctctctatctattctacttgtttattcccttcaaggtttttttttaaggagtacttgtttttagaatatacggtcaacgaactataattaactaaacaagcttaaaatgatggattttgttttgttagaaaaagctcttcttggtttgttcattgcaactatagtagccatcacaatctctaagctaaggggaaagaaacttaagttgcctccaggcccaatccctgtcccagtgtttggtaattggttacaagttggcgacgacttaaaccagaggaatttggtagagtatgctaaaaagttcggcgacttatttctacttaggatgggtcaaagaaacttggtcgtggtttcatcccctgacttagcaaaagacgtactacatacccagggtgtcgagttcggaagtagaactagaaatgttgtgtttgatattttcacaggcaaaggtcaagatatggtttttaccgtatacagcgagcactggaggaaaatgagaagaataatgactgtcccattctttacaaacaaagtggttcaacagtataggttcggatgggaggacgaagccgctagagtagtcgaggatgttaaggcaaatcctgaagccgctaccaacggtattgtgttgaggaatagattacaacttttgatgtacaacaatatgtatagaataatgtttgacaggagatttgaatctgttgatgatccattattcctaaaacttaaggcattgaatggcgagagatcaaggttagctcaatcctttgaatacaacttcggtgacttcattcctatattgaggccattcttgagaggatatcttaagttgtgtcaggaaatcaaggacaaaaggttaaagctattcaaggactacttcgtcgacgagagaaaaaagttggagagtatcaagagcgtaggtaataactccttaaagtgcgccatagatcatattatcgaggcacaagaaaaaggcgagataaacgaggataacgtgttatacatcgtcgagaatatcaacgtggctgccattgaaactacactttggtctattgaatggggtatagcagaactagtgaataaccctgaaatccagaaaaaattgagacacgaattagacaccgtacttggagctggtgttcaaatttgtgaaccagatgttcaaaaattgccttatctacaggccgtgataaaagagactttaaggtacaggatggcaattccattgttagtcccacatatgaatcttcacgaagccaaattggccggctatgatatccctgcagagagcaaaattttggtaaacgcttggtggttagccaataatccagcacattggaacaaacctgatgagtttagaccagaaagatttttggaggaagaatccaaggtcgaggctaatggaaacgactttaagtacatccctttcggtgttggcagaagatcttgcccaggtataattcttgctttaccaatccttggaatagtaattggtaggttggttcaaaacttcgagttacttccacctccaggccaaagcaaaatagatacagccgaaaaaggtggacagttttcattgcaaatcctaaagcattccactattgtgtgtaaacctagaagttcttaaccgcggacaaatcgctcttaaatatatacctaaagaacattaaagctatattataagcaaagatacgtaaattttgcttatattattatacacatatcatatttctatatttttaagatttggttatataatgtacgtaatgcaaaggaaataaattttatacattattgaacagcgtccaagtaactacattatgtgcactaatagtttagcgtcgtgaagactttattgtgtcgcgaaaagtaaaaattttaaaaattagagcaccttgaacttgcgaaaaaggttctcatcaactgtttaaaaggaggatatcaggtcctatttctgacaaacaatatacaaatttagtttcaaaggcgcgttgcaaaatggaatttcgccgcagcggcctgaatggctgtaccgcctgacgcggatgcgccacgcgccgcatgccggtagaggtgtggtcaataagagcgacctcatgctatacctgagaaagcaacctgacctacaggaaagagttactcaagaataagaattttcgttttaaaacctaagagtcactttaaaatttgtatacacttattttttttataacttatttaataataaaaatcataaatcataagaaattcgcttatttagaagtgtcaacaacgtatctaccaacgatttgacccttttccatcttttcgtaaatttctggcaaggtagacaagccgacaaccttgattggagacttgaccaaacctctggcgaagaagtccaaagctctagatcaatttaggcctgcggccgcggttaccagacatcttcttggtatctacctgaagtcttgagcatcttgattagctctgttgcttcatcagtggtaatggatttaccacgggataagatgccaaccaatgcggttgacacacccttggccataccctttgcatcaccacagacgtagataaatgcaccgttgttaatcatttcaaatacttggtcttcgtaatcctttaatttatcttgaacataaacttttttggtgtttggcaacctggaatgggccacgaccatttcgaacgaaccatccaattttttggcgtattctggccattcgtcctggtacaagaaatcatcagtgttacgggatccataaaacagtatatgcttacctagcgaaacgttgttaccgcccttcttttgtgattcgaggaacgcgacacgctctctgataaacccacggaatggggcaacaccggtacctggaccgatcatgataactggggtggaagggttggaaggcaatctgaagttagaacgacgaacgtggacgggcaatttgtaattggcgaaaagtttacgtgggccatttaaatcgtagtgaacaggtaggttagtttcggcaatgttaacattgttttgagccaattgaatgtttcttaacaagttagtcgtaacaccaacaactggaggagcatcaggcaattctgggttaggaaagttttccacaatggaggtgacatggacggtttgcttttcagacagagaagaggaagagatagagtagtaacgaggagtcatttggggaactgattcgaccaagaattgcatgggtacggtgtcccatttggcgccatcagacaaatatttcagagcatctgcgatgttgaaatatttggaggttatctcgacggcgaattggtccttgtctttcgaaagcagagtcaatttttccttgacgtcagcgttgggggcgaactgaatcaaagatgaaaacaattgtctggagacaggtcctgtaatttccaaatagtgtttaatagcagcgccaatagtagttggcgttgggaagggcactttgacggtgggatccaggggcttcaagtcaaaaatggtttcagggtccaggttgaatatggataagaactgttcgaccttttccaatgggttggaaggccaaacagcaagatggtcaccagtggagtacttgatgttagagccggacaagtcaaattcagagtggatgcaattacggtcattggaagagaacagttcgcgagatttcacgatgggtgcaatatacggttgagacaaatcgaagggacccaattggatgccgtctgcgttgcggttcaactgatgcgagggcaaatagtgagcagagggttcaccaagcgacatggagtcagtgatttcgttcaacacagtgtactggaattgagaggtgaacttggcttcctgttcgtccaaatgcagttcgtctttcaaaacctccaggatggagtccttccaggccatgtaatcttcgtctgtagttcctgcaccatcatcagcttcaccgagcttgcctagtctgatagcgcccgcagcggagagatgcttctcggccttcttggcggcaccattaaagaattcataagtagaatttcccagaccaaacatattatacctcaggttcgatagtgcacccgcttccgcattacaaataaagtcttcaaagttgaccgccccgtcggggaagtctccttcaccatatgtagagataaaaatcgagactatgacgggcacatcgtttagcgactcaaagtcgtagttctcaacatctgcgcacatcacgtttaggttgaacttggccaccagctccttggaaaactttttggcgtaatcctcggcagtcccagtctgcgacgcatacaacaccaagtagttcttgttgttttcggtcaccacctgagcaatgtctctgttgcccgagctgacagctgtgatatctccgtcatcggacatcagcagttccttgatggagtttctctttacgtacagtagcacggcaagcactagccccgccaggacagtgaagtcggtgttgtctattccaaacggcattttactagtaagctttgtgatgatgttttatttgttttgattggtgtcttgtaaatagaaacaagagagaataataaacaagttaagaataaaaaaccaaaggatgaaaaagaatgaatatgaaaaagagtagagaataactttgaaaggggaccatgatataactggaaaaaagaggttcttggaaatgaaaagttaccaaagagtatttataattcagaaaaaaaagccaacgaatatcgttttgatggcgagcctttttttttttttaggaagacactaaaggtacctagcatcatatgggaaggaaaggaaatcacttggaagacatcacaagcattcatttaccaagagaaaaaatatgcattttagctaagatccattgaacaaagcactcactcaactcaactgaatgaacgaaagaagaaagaacagtagaaaacactttgtgacggtgcggaacacatttacgtagctatcatgctgaattctactatgaaaatctcccaatctgtcgatggcaaaacgacccacgtggcagagttgggtcaagtgccagtttctggattaagtaacagatacagacatcacacgccatagaggaatcccgccgttgcgagagatggaaaacaatagagccgaaattgtggaagcccgatgtctgggtgtacattttttttttttctttctttctctttcaataatctttcctttttccatttagcttgccggaaaaactttcgggtagcgaaaatctttctgccggaaaaattagctatttttttcttccttattatttttttagttctgaagtttgaccagggcgctaccctgaccgtatcacaaccgacgatccggggtcatggcggctatttttttttttttttttttttccttgtgattgtttatttacatttggatcaattctaacaaaaaaaaaataaggggggaaaaataattcacctctttttaatattgttttgtactgagattgatctccaaaatagtagcattggcgcgtgccaccaacagccccgccaatggcgctgccgatactcccgacaatccccaccattgcctg

SEQ ID NO: 11 - DNA, 3607 bp, Helper fragment
tttcccgtctttcagtgccttgttcagttcttcctgacgggcggtatatttctccagcttggcctatgcggccctgtcagaccaagtttacgagctcgcttggactcctgttgatagatccagtaatgacctcagaactccatctggatttgttcagaacgctcggttgccgccgggcgttttttattggtgagaatccaagcactagggacagtaagacgggtaagcctgttgatgataccgctgccttactgggtgcattagccagtctgaatgacctgtcacgggataatccgaagtggtcagactggaaaatcagagggcaggaactgctgaacagcaaaaagtcagatagcaccacatagcagacccgccataaaacgccctgagaagcccgtgacgggcttttcttgtattatgggtagtttccttgcatgaatccataaaaggcgcctgtagtgccatttacccccattcactgccagagccgtgagcgcagcgaactgaatgtcacgaaaaagacagcgactcaggtgcctgatggtcggagacaaaaggaatattcagcgatttgcccgagcttgcgagggtgctacttaagcctttagggttttaaggtctgttttgtagaggagcaaacagcgtttgcgacatccttttgtaatactgcggaactgactaaagtagtgagttatacacagggctgggatctattctttttatctttttttattctttctttattctataaattataaccacttgaatataaacaaaaaaaacacacaaaggtctagcggaatttacagagggtctagcagaatttacaagttttccagcaaaggtctagcagaatttacagatacccacaactcaaaggaaaaggacatgtaattatcattgactagcccatctcaattggtatagtgattaaaatcacctagaccaattgagatgtatgtctgaattagttgttttcaaagcaaatgaactagcgattagtcgctatgacttaacggagcatgaaaccaagctaattttatgctgtgtggcactactcaaccccacgattgaaaaccctacaaggaaagaacggacggtatcgttcacttataaccaatacgctcagatgatgaacatcagtagggaaaatgcttatggtgtattagctaaagcaaccagagagctgatgacgagaactgtggaaatcaggaatcctttggttaaaggctttgagattttccagtggacaaactatgccaagttctcaagcgaaaaattagaattagtttttagtgaagagatattgccttatcttttccagttaaaaaaattcataaaatataatctggaacatgttaagtcttttgaaaacaaatactctatgaggatttatgagtggttattaaaagaactaacacaaaagaaaactcacaaggcaaatatagagattagccttgatgaatttaagttcatgttaatgcttgaaaataactaccatgagtttaaaaggcttaaccaatgggttttgaaaccaataagtaaagatttaaacacttacagcaatatgaaattggtggttgataagcgaggccgcccgactgatacgttgattttccaagttgaactagatagacaaatggatctcgtaaccgaacttgagaacaaccagataaaaatgaatggtgacaaaataccaacaaccattacatcagattcctacctacataacggactaagaaaaacactacacgatgctttaactgcaaaaattcagctcaccagttttgaggcaaaatttttgagtgacatgcaaagtaagtatgatctcaatggttcgttctcatggctcacgcaaaaacaacgaaccacactagagaacatactggctaaatacggaaggatctgaggttcttatggctcttgtatctatcagtgaagcatcaagactaacaaacaaaagtagaacaactgttcaccgttacatatcaaagggaaaactgtccatatgcacagatgaaaacggtgtaaaaaagatagatacatcagagcttttacgagtttttggtgcattcaaagctgttcaccatgaacagatcgacaatgtaacgcggccgcagccaatcaattcttgcggagaactgtgaatgcgcaaaccaacccttggcagaacatatccatcgcgtccgccatctccagcagccgcacgcggcgcatcgggggggggggggggggtttcaattcatcattttttttttattcttttttttgatttcggtttccttgaaatttttttgattcggtaatctccgaacagaaggaagaacgaaggaaggagcacagacttagattggtatatatacgcatatgtagtgttgaagaaacatgaaattgcccagtattcttaacccaactgcacagaacaaaaacctgcaggaaacgaagataaatcatgtcgaaagctacatataaggaacgtgctgctactcatcctagtcctgttgctgccaagctatttaatatcatgcacgaaaagcaaacaaacttgtgtgcttcattggatgttcgtaccaccaaggaattactggagttagttgaagcattaggtcccaaaatttgtttactaaaaacacatgtggatatcttgactgatttttccatggagggcacagttaagccgctaaaggcattatccgccaagtacaattttttactcttcgaagacagaaaatttgctgacattggtaatacagtcaaattgcagtactctgcgggtgtatacagaatagcagaatgggcagacattacgaatgcacacggtgtggtgggcccaggtattgttagcggtttgaagcaggcggcagaagaagtaacaaaggaacctagaggccttttgatgttagcagaattgtcatgcaagggctccctatctactggagaatatactaagggtactgttgacattgcgaagagcgacaaagattttgttatcggctttattgctcaaagagacatgggtggaagagatgaaggttacgattggttgattatgacacccggtgtgggtttagatgacaagggagacgcattgggtcaacagtatagaaccgtggatgatgtggtctctacaggatctgacattattattgttggaagaggactatttgcaaagggaagggatgctaaggtagagggtgaacgttacagaaaagcaggctgggaagcatatttgagaagatgcggccagcaaaactaaaaaactgtattataagtaaatgcatgtatactaaactcacaaattagagcttcaatttaattatatcagttattacccggccgggaatctcggtcgtaatgatttttataatgacgaaaaaaaaaaaattggaaagaaaaccccccccccccccccgcagcgttgggtcctggccacgggtgcgcatgatcgtgctcctgtcgttgaggacccggctaggctggcggggttgccttactggttagcagaatgaatcaccgatacgcgagcgaatgtggcggccgcacgcgttcatcgtccacctccggagaacaggccaccatcacgcatctgtgtctgaatttcatcacg

SEQ ID NO: 12 - DNA, 1855 bp, Helper fragment
tcatcgtccacctccggagaacaggccaccatcacgcatctgtgtctgaatttcatcacgacgcgccttaagggcaccaataactgccttaaaaaaattacgccccgccctgccactcatcgcagtactgttgtaattcattaagcattctgccgacatggaagccatcacagacggcatgatgaacctgaatcgccagcggcatcagcaccttgtcgccttgcgtataatatttgcccatggtgaaaacgggggcgaagaagttgtccatattggccacgtttaaatcaaaactggtgaaactcacccagggattggctgagacgaaaaacatattctcaataaaccctttagggaaataggccaggttttcaccgtaacacgccacatcttgcgaatatatgtgtagaaactgccggaaatcgtcgtggtattcactccagagcgatgaaaacgtttcagtttgctcatggaaaacggtgtaacaagggtgaacactatcccatatcaccagctcaccgtctttcattgccatacggaattccggatgagcattcatcaggcgggcaagaatgtgaataaaggccggataaaacttgtgcttatttttctttacggtctttaaaaaggccgtaatatccagctgaacggtctggttataggtacattgagcaactgactgaaatgcctcaaaatgttctttacgatgccattgggatatatcaacggtggtatatccagtgatttttttctccattttagcttccttagctcctgaaaatctcgataactcaaaaaatacgcccggtagtgatcttatttcattatggtgaaagttggaacctcttacgtgccgatcaacgtctcattttcgccaaaagttggcccagggcttcccggtatcaacagggacaccaggatttatttattctgcgaagtgatcttccgtcacaggtattggaccaccctgtgggtttataagcgcgctgctggcgtgtaaggcggtgacggcgaaggaagggtccttttcatcacgtgctataaaaataattataatttaaattttttaatataaatatataaattaaaaatagaaagtaaaaaaagaaattaaagaaaaaatagtttttgttttccgaagatgtaaaagactctagggggatcgccaacaaatactaccttttatcttgctcttcctgctctcaggtattaatgccgaattgtttcatcttgtctgtgtagaagaccacacacgaaaatcctgtgattttacattttacttatcgttaatcgaatgtatatctatttaatctgcttttcttgtctaataaatatatatgtaaagtacgctttttgttgaaattttttaaacctttgtttatttttttttcttcattccgtaactcttctaccttctttatttactttctaaaatccaaatacaaaacataaaaataaataaacacagagtaaattcccaaattattccatcattaaaagatacgaggcgcgtgtaagttacaggcaagcgatccgtcctaagaaaccattattatcatgacattaacctataaaaataggcgtatcacgaggccctttcgtctcgcgcgtttcggtgatgacggtgaaaacctctgacacatgcagctcccggagacggtcacagcttgtctgtaagcggatgccgggagcagacaagcccgtcagggcgcgtcagcgggtgttggcgggtgtcggggctggcttaactatgcggcatcagagcagattgtactgagagtgcaccacggcgcgtggcacccttgcgggccatgtcatacaccgccttcagagcagccggacctatctgcccgtt

SEQ ID NO: 13 - DNA, 732 bp, Helper fragment for multi-expression plasmid
gccaccaacagccccgccaatggcgctgccgatactcccgacaatccccaccattgcctgacgcgtccagtatcccagcagatacgggatatcgacatttctgcaccattccggcgggtataggttttattgatggcctcatccacacgcagcagcgtctgttcatcgtcgtggcggcccataataatctgccggtcaatcagccagctttcctcacccggcccccatccccatacgcgcatttcgtagcggtccagctgggagtcgataccggcggtcaggtaagccacacggtcaggaacgggcgctgaataatgctctttccgctctgccatcacttcagcatccggacgttcgccaattttcgcctcccacgtctcaccgagcgtggtgtttacgaaggttttacgttttcccgtatcccctttcgttttcatccagtctttgacaatctgcacccaggtggtgaacgggctgtacgctgtccagatgtgaaaggtcacactgtcaggtggctcaatctcttcaccggatgacgaaaaccagagaatgccatcacgggtccagatcccggtcttttcgcagatataacgggcatcagtaaagtccagctcctgctggcggatgacgcaggcattatgctcgcagagataaaacacgctggagacgcgttttcccgtctttcagtgccttgttcagttcttcctgacgggcggtatatttctccagctt

SEQ ID NO: 14 - DNA, 732 bp, Helper fragment for multi-expression plasmid
cttaagcagaatttctgtcatcatggacagcacggaacgggtgaagctgcgccagttctgacgcgtctccagcgtgttttatctctgcgagcataatgcctgcgtcatccgccagcaggagctggactttactgatgcccgttatatctgcgaaaagaccgggatctggacccgtgatggcattctctggttttcgtcatccggtgaagagattgagccacctgacagtgtgacctttcacatctggacagcgtacagcccgttcaccacctgggtgcagattgtcaaagactggatgaaaacgaaaggggatacgggaaaacgtaaaaccttcgtaaacaccacgctcggtgagacgtgggaggcgaaaattggcgaacgtccggatgctgaagtgatggcagagcggaaagagcattattcagcgcccgttcctgaccgtgtggcttacctgaccgccggtatcgactcccagctggaccgctacgaaatgcgcgtatggggatgggggccgggtgaggaaagctggctgattgaccggcagattattatgggccgccacgacgatgaacagacgctgctgcgtgtggatgaggccatcaataaaacctatacccgccggaatggtgcagaaatgtcgatatcccgtatctgctgggatactggacgcgttttcccgtctttcagtgccttgttcagttcttcctgacgggcggtatatttctccagctt

SEQ ID NO: 15 - DNA, 663 bp, Non-expressed stuffer
ggcctgcagggccagcttacccttaaatttatttgcactactggaaaactacctgttccatggccaacacttgtcactactttctcttatggtgttcaatgcttttcccgttatccggatcatatgaaacggcatgactttttcaagagtgccatgcccgaaggttatgtacaggaacgcactatatctttcaaagatgacgggaactacaagacgcgtgctgaagtcaagtttgaaggtgatacccttgttaatcgtatcgagttaaaaggtattgattttaaagaagatggaaacattctcggacacaaactcgagtacaactataactcacacaatgtatacatcacggcagacaaacaaaagaatggaatcaaagctaacttcaaaattcgccacaacattgaagatggatccgttcaactagcagaccattatcaacaaaatactccaattggcgatggccctgtccttttaccagacaaccattacctgtcgacacaatctgccctttcgaaagatcccaacgaaaagcgtgaccacatggtccttcttgagtttgtaactgctgctgggattacacatggcatggatgagctctacaaataatgaattcgtcgaggccgttcaggcctcgaggccgttcaggctcgacccggggat

SEQ ID NO: 16 - protein, 717 aa, Arabidopsis thaliana
MDQIEAMLCGGGEKTKVAVTTKTLADPLNWGLAADQMKGSHLDEVKKMVEEYRRPVVNLGGETLTIGQVAAISTVGGSVKVELAETSRAGVKASSDWVMESMNKGTDSYGVTTGFGATSHRRTKNGTALQTELIRFLNAGIFGNTKETCHTLPQSATRAAMLVRVNTLLQGYSGIRFEILEAITSLLNHNISPSLPLRGTITASGDLVPLSYIAGLLTGRPNSKATGPDGESLTAKEAFEKAGISTGFFDLQPKEGLALVNGTAVGSGMASMVLFEANVQAVLAEVLSAIFAEVMSGKPEFTDHLTHRLKHHPGQIEAAAIMEHILDGSSYMKLAQKVHEMDPLQKPKQDRYALRTSPQWLGPQIEVIRQATKSIEREINSVNDNPLIDVSRNKAIHGGNFQGTPIGVSMDNTRLAIAAIGKLMFAQFSELVNDFYNNGLPSNLTASSNPSLDYGFKGAEIAMASYCSELQYLANPVTSHVQSAEQHNQDVNSLGLISSRKTSEAVDILKLMSTTFLVGICQAVDLRHLEENLRQTVKNTVSQVAKKVLTTGINGELHPSRFCEKDLLKVVDREQVFTYVDDPCSATYPLMQRLRQVIVDHALSNGETEKNAVTSIFQKIGAFEEELKAVLPKEVEAARAAYGNGTAPIPNRIKECRSYPLYRFVREELGTKLLTGEKVVSPGEEFDKVFTAMCEGKLIDPLMDCLKEWNGAPIPIC

SEQ ID NO: 17 - protein, 506 aa, Ammi majus
MMDFVLLEKALLGLFIATIVAITISKLRGKKLKLPPGPIPVPVFGNWLQVGDDLNQRNLVEYAKKFGDLFLLRMGQRNLVVVSSPDLAKDVLHTQGVEFGSRTRNVVFDIFTGKGQDMVFTVYSEHWRKMRRIMTVPFFTNKVVQQYRFGWEDEAARVVEDVKANPEAATNGIVLRNRLQLLMYNNMYRIMFDRRFESVDDPLFLKLKALNGERSRLAQSFEYNFGDFIPILRPFLRGYLKLCQEIKDKRLKLFKDYFVDERKKLESIKSVGNNSLKCAIDHIIEAQEKGEINEDNVLYIVENINVAAIETTLWSIEWGIAELVNNPEIQKKLRHELDTVLGAGVQICEPDVQKLPYLQAVIKETLRYRMAIPLLVPHMNLHEAKLAGYDIPAESKILVNAWWLANNPAHWNKPDEFRPERFLEEESKVEANGNDFKYIPFGVGRRSCPGIILALPILGIVIGRLVQNFELLPPPGQSKIDTAEKGGQFSLQILKHSTIVCKPRSS

SEQ ID NO: 18 - protein, 556 aa, Arabidopsis thaliana
MTTQDVIVNDQNDQKQCSNDVIFRSRLPDIYIPNHLPLHDYIFENISEFAAKPCLINGPTGEVYTYADVHVTSRKLAAGLHNLGVKQHDVVMILLPNSPEVVLTFLAASFIGAITTSANPFFTPAEISKQAKASAAKLIVTQSRYVDKIKNLQNDGVLIVTTDSDAIPENCLRFSELTQSEEPRVDSIPEKISPEDVVALPFSSGTTGLPKGVMLTHKGLVTSVAQQVDGENPNLYFNRDDVILCVLPMFHIYALNSIMLCSLRVGATILIMPKFEITLLLEQIQRCKVTVAMVVPPIVLAIAKSPETEKYDLSSVRMVKSGAAPLGKELEDAISAKFPNAKLGQGYGMTEAGPVLAMSLGFAKEPFPVKSGACGTVVRNAEMKILDPDTGDSLPRNKPGEICIRGNQIMKGYLNDPLATASTIDKDGWLHTGDVGFIDDDDELFIVDRLKELIKYKGFQVAPAELESLLIGHPEINDVAVVAMKEEDAGEVPVAFVVRSKDSNISEDEIKQFVSKQVVFYKRINKVFFTDSIPKAPSGKILRKDLRARLANGLMN

SEQ ID NO: 19 - protein, 399 aa, Hordeum vulgare
MAAVRLKEVRMAQRAEGLATVLAIGTAVPANCVYQATYPDYYFRVTKSEHLADLKEKFQRMCDKSMIRKRHMHLTEEILIKNPKICAHMETSLDARHAIALVEVPKLGQGAAEKAIKEWGQPLSKITHLVFCTTSGVDMPGADYQLTKLLGLSPTVKRLMMYQQGCFGGATVLRLAKDIAENNRGARVLVVCSEITAMAFRGPCKSHLDSLVGHALFGDGAAAAIIGADPDQLDEQPVFQLVSASQTILPESEGAIDGHLTEAGLTIHLLKDVPGLISENIEQALEDAFEPLGIHNWNSIFWIAHPGGPAILDRVEDRVGLDKKRMRASREVLSEYGNMSSASVLFVLDVMRKSSAKDGLATTGEGKDWGVLFGFGPGLTVETLVLHSVPVPVPTAASA

SEQ ID NO: 20 - protein, 483 aa, Malus domestica
MGDVIVLYASPGMGHIVSMVELGKFIVHRYGPHKFSITILYTCGSIVDTASIPVYIRRISHSHPFISFRQFPRVTNNITRNISVPAITFDFIRQNDPHVRSALQEISKSATVRAFIIDLFCTSALPIGKEFNIPTYYFRTSGAAILAAFLYLPKIDEQTKTTESFKDLRDTVFEFPGWKSPLKATHMVQLVLDRNDPAYSDMIYFCSHLPKSNGIIVNTFEELEPPSVLQAIAGGLCVPDGPTPPVYYVGPLIEEEKELSKDADAAEKEDCLSWLDKQPSRSVLFLCFGSMGSFPAAQLKEIANGLEASGQRFLWVVKKPPVEEKSKQVHGVDDFDLKGVLPEGFLERTADRGMVVKSWAPQVVVLKKESVGGFVTHCGWNSVLEAVVAGVPMIAWPLYAEQHMNRNVLVTDMEIAIGVEQRDEEGGFVSGEEVERRVRELMESEGGRVLRERCKKLGEMASAALGETGSSTRNLVNFVSSIT

SEQ ID NO: 21 - protein, 691 aa, Saccharomyces cerevisiae
MPFGIDNTDFTVLAGLVLAVLLYVKRNSIKELLMSDDGDITAVSSGNRDIAQVVTENNKNYLVLYASQTGTAEDYAKKFSKELVAKFNLNVMCADVENYDFESLNDVPVIVSIFISTYGEGDFPDGAVNFEDFICNAEAGALSNLRYNMFGLGNSTYEFFNGAAKKAEKHLSAAGAIRLGKLGEADDGAGTTDEDYMAWKDSILEVLKDELHLDEQEAKFTSQFQYTVLNEITDSMSLGEPSAHYLPSHQLNRNADGIQLGPFDLSQPYIAPIVKSRELFSSNDRNCIHSEFDLSGSNIKYSTGDHLAVWPSNPLEKVEQFLSIFNLDPETIFDLKPLDPTVKVPFPTPTTIGAAIKHYLEITGPVSRQLFSSLIQFAPNADVKEKLTLLSKDKDQFAVEITSKYFNIADALKYLSDGAKWDTVPMQFLVESVPQMTPRYYSISSSSLSEKQTVHVTSIVENFPNPELPDAPPVVGVTTNLLRNIQLAQNNVNIAETNLPVHYDLNGPRKLFANYKLPVHVRRSNFRLPSNPSTPVIMIGPGTGVAPFRGFIRERVAFLESQKKGGNNVSLGKHILFYGSRNTDDFLYQDEWPEYAKKLDGSFEMVVAHSRLPNTKKVYVQDKLKDYEDQVFEMINNGAFIYVCGDAKGMAKGVSTALVGILSRGKSITTDEATELIKMLKTSGRYQEDVW

SEQ ID NO: 22 - protein, 310 aa, Saccharomyces cerevisiae
MPITIKSRSKGLRDTEIDLSKKPTLDDVLKKISANNHNISKYRIRLTYKKESKQVPVISESFFQEEADDSMEFFIKDLGPQISWRLVFFCEYLGPVLVHSLFYYLSTIPTVVDRWHSASSDYNPFLNRVAYFLILGHYGKRLFETLFVHQFSLATMPIFNLFKNCFHYWVLSGLISFGYFGYGFPFGNAKLFKYYSYLKLDDLSTLIGLFVLSELWNFYCHIKLRLWGDYQKKHGNAKIRVPLNQGIFNLFVAPNYTFEVWSWIWFTFVFKFNLFAVLFLTVSTAQMYAWAQKKNKKYHTRRAFLIPFVF

SEQ ID NO: 23 - DNA, 1182 bp, Pinus densiflora
atgggtggtgttgattttgaaggtttcagaaagttgcaaagagctgacggttttgcttccattttggctattggtactgctaatccaccaaacgctgttgatcaatctacttacccagattactacttcagaatcaccggtaacgaacataacactgaattgaaggacaagttcaagagaatctgcgaaagatccgctatcaagcaaagatatatgtacttgaccgaagaaatcttgaaaaagaacccagatgtttgcgcctttgttgaagttccatctttggatgctagacaagctatgttggctatggaagttccaagattggctaaagaagctgctgaaaaggctatccatgaatggggtcaatctaagtctggtattacccatttgattttctgttctactaccaccccagatttgccaggtgctgatttcgaagttgctaagttgttgggtttacacccatctgttaagagagttggtgttttccaacatggttgttttgctggtggtactgttttgagattagctaaggatttggccgaaaacaatagaggtgctagagttttggttatctgctctgaaactactgctgttacttttagaggtccatctgaaacccatttggattctttggttggtcaagctttgtttggtgatggtgcttctgctttgatagttggtgctgatccaattccacaagttgaaaaagcttgcttcgaaattgtcagaacctctcaaactgttgttccaaattcagatggtgctattggtggtaaggttagagaagttggtttgaccttccaattgaagggtgctgttccagatttgatttccgctaacattgaaaactgcttggttgaagctttctcccaattcaaaatttgcgactggaacaagttgttctgggttgttcatccaggtggtagagctattttggatagagttgaagctaagttgaacttggacccaactaagttgattccaaccagacatgttatgtccgaatacggtaatatgtcctctgcttgcgttcatttcattttggacgaaactagaaaggcctctttgagaaatggttgttctacaactggtgaaggtttggaaatgggtgttttgttcggttttggtccaggtttgactattgaaaccgttgttttgaagtccgtcccattacaatga

SEQ ID NO: 24 - protein, 393 aa, Pinus densiflora
MGGVDFEGFRKLQRADGFASILAIGTANPPNAVDQSTYPDYYFRITGNEHNTELKDKFKRICERSAIKQRYMYLTEEILKKNPDVCAFVEVPSLDARQAMLAMEVPRLAKEAAEKAIHEWGQSKSGITHLIFCSTTTPDLPGADFEVAKLLGLHPSVKRVGVFQHGCFAGGTVLRLAKDLAENNRGARVLVICSETTAVTFRGPSETHLDSLVGQALFGDGASALIVGADPIPQVEKACFEIVRTSQTVVPNSDGAIGGKVREVGLTFQLKGAVPDLISANIENCLVEAFSQFKICDWNKLFWVVHPGGRAILDRVEAKLNLDPTKLIPTRHVMSEYGNMSSACVHFILDETRKASLRNGCSTTGEGLEMGVLFGFGPGLTIETVVLKSVPLQ

SEQ ID NO: 25 - protein, 319 aa, Kluyveromyces lactis
MSASSSIFIKSRSKSLKDVKLEVPTENTLTYQSVLQQISKSNHNISVNRLRLSYLKEGKQVAIGPSELNDVGKKNTFDSVNEWYVKDLGPQISWRLVFFIEYLGPILIHSLVYLLSLNATVRDKFHSKNVPYNDFFNKFIYRLIMVHYLKREFETLFIHSFSLETMPLFNLFKNSFHYWILNGLISLGYFGYGFPFANKTLYRVYSALKISDFRVLTALFGLSEMFNFYIHVALRRWGDEQKRNGVTKRVPLNSGLFKLLVAPNYTFESWAWMFFTLLFKLNLFSVLFLVVSVVQMYLWAQKKNKKYGTKRAFLIPFLF

SEQ ID NO: 26 - protein, 253 aa, Saccharomyces cerevisiae
MYFDEEQLLKYTIYAYRLSFFVGICSLFIAKSCLPEFLQYGKTYRPKENSKYSSILERIKKFTVPKAYFSHFYYLATFLSLVTLYFYPKFPIVWIIFGHSLRRLYETLYVLHYTSNSRMNWSHYLVGIWFYSVLLLILNISLYKNSIPNTLNMNAFIIFCIASWDQYKNHVILANLVKYSLPTGRLFRLVCCPHYLDEIIIYSTLLPYEQEFYLTLVWVITSLTISALETKNYYRHKFKDNHVAPYAIIPFII

SEQ ID NO: 27 - DNA, 1173 bp, Hypericum androsaemum
atggttactgttgaagaagttagaaaagctcaaagggcagaaggtccagccacagtgatggctattggaaccgcagttcctccaaattgtgtagatcaggccacttatcctgactactactttagaataacaaactctgagcataaggctgaattgaaagaaaagttccaaaggatgtgcgacaaatcacagatcaagaaaagatacatgtaccttaatgaggaagtcctaaaggaaaacccaaatatgtgtgcatacatggccccttcccttgacgctagacaagatattgtggttgtagaggtcccaaaattgggcaaggaagcagctgttaaagccataaaggaatggggtcaacctaagagcaaaatcacccaccttgtgttttgcactacaagcggagttgacatgccaggcgcagattatcagctaaccaaacttttgggtttaaggccttctgtaaaaagattgatgatgtaccaacaaggttgtttcgctggaggcactgtcttaagactagccaaggatcttgcagagaacaacaaaggtgctagggtgttggttgtatgctcagaaattacagccgtcacctttagaggaccaactgacactcacttagattccctagttggtcaggcattgtttggcgacggtgctgccgcaataatcattggaagtgatcctattccagaggtggaaaagcctctttttgaacttgttagcgctgcccaaactatattgccagattctgagggtgcaatcgacggccacttaagggaagtaggtctaaccttccatcttttgaaagatgtccctggtttaatttcaaagaacgtggaaaaatccctaacagaggcttttaaaccattgggtataagtgactggaatagcttattctggatcgctcacccaggcggccctgccatacttgaccaggttgaagcaaaattgagcttaaagccagaaaaactaagagctactagacatgtattgtcagagtatggtaacatgtccagtgcctgtgtccttttcattttggatgaaatgaggagaaaaagcaaggaggacggcctaaaaaccacaggtgagggaatcgaatggggtgttctattcggctttggtccaggccttactgtggagacagttgtacttcattcagtcgcaattaattag

SEQ ID NO: 28 - DNA, 1197 bp, Petroselinum crispum
atggctaatcatcataatgctgaaattgaggaaataagaaacagacaaagagcccagggtccagctaatatcttggcaattggaactgccacaccttctaattgtgtttatcaagctgattacccagactattacttcagaatcaccaactcagagcacatgacagacttaaagttgaaattcaagagaatgtgcgaaaagagtatgataagaaagagatacatgcacatcaccgaggagtatttgaaggagaaccctaacgtgtgcgcctacgaggccccaagtttagacgctagacaggacttggtagtcgttgaagtgccaagattaggaaaagaagccgctagtaaggccattaaagaatggggacaaccaaaatctaagatcactcacttaatattctgtacaacctccggtgtcgacatgccaggtgcagactaccaattgacaaagttattgggattaagaccaagtgtgaaaagattcatgatgtatcagcaaggatgcttcgcaggaggtactgttttgagattggcaaaggacttagccgaaaataacgctggtgccagagtattagtggtgtgttctgaaattacagccgtgactttcagaggaccatccgactcccacttggatagtttagttggtcaggctttgtttggtgacggagccgcagccgtgatattaggaagtgaccctgatttgtcagtcgaaagaccattattccagttgatttctgccgcacaaactatcttaccagacagtgatggagctatagacggtcatttgagagaagtgggtttaacatttcatttgttaaaagatgttcctggtttaataagtaagaatattgaaaagtcattgaaggaggctttcggtccaataggaattagtgattggaactccttattttggatagcacacccaggaggtcctgctatattggaccaggtagagttgaagttaggtttaaaggaagagaagatgagagctactagacaagtcttaagtgattacggtaacatgtcatctgcctgtgttttgttcatattagacgaaatgagaaagaaatcaattgaagagggaaaagctaccacaggagaaggattagactggggtgttttgttcggatttggtcctggattgactgttgaaaccgtagtcttacatagtgtgcctgctacattcactcactga

SEQ ID NO: 29 - DNA, 1170 bp, Petunia hybrida
atggttactgttgaagaatatagaaaagctcaaagggcagagggtccagccacagtcatggctattggaaccgcaactcctacaaattgtgtggatcagtctacctacccagactattactttagaataactaactcagaacataagacagatttgaaagaaaagttcaaaaggatgtgcgaaaagtccatgatcaaaaagagatatatgcacttaaccgaggaaattctaaaggagaaccctagtatgtgtgagtacatggccccaagccttgacgctagacaagatatagttgtagtcgaagtgcctaagctaggaaaagaagcagcccagaaggctatcaaagaatggggtcaaccaaagagcaaaattacccacctttttttctgcacaacctcaggagttgacatgcctggctgtgattatcaactaactaaacttttgggtttaaggccatccgtaaagagattgatgatgtaccagcaaggttgctttgcaggaggcacagtcttaagactagctaaagatcttgccgaaaataataagggtgcaagggttttggtggtttgtagtgagataactgctgtaaccttcagaggacctaacgacactcacttagatagcctagtcggtcaagccttgtttggcgacggtgcaggagctatcattattggttctgatccaatacctggcgtggaaaggccattattcgaacttgtttcagccgcacagactttgttacctgattcccatggtgctatcgacggacacctaagagaggtaggtcttacctttcatttgttaaaagatgtccctggtttaattagtaagaatatagagaagagcttggaagaggccttcaagccattaggaatcagcgactggaactcacttttttggattgcacatcctggcggcccagctatacttgaccaagttgaaatcaaattgggcctaaagcctgaaaaattgaaggccacaagaaatgtgttatccgattatggaaacatgagttctgcatgtgttcttttcattttggatgagatgaggaaggcttcagctaaagaaggtctaggcactacaggtgagggcttggagtggggtgtactattcggctttggaccaggccttaccgtcgaaactgtggttttacactctgtagccacataa

SEQ ID NO: 30 - DNA, 1197 bp, Hordeum vulgare
atggctgctacaatgaccgttgaagaagtgagaaatgctcaaagggccgaaggtcccgcaacagtattagccattggcacagctactccagcaaattgtgtttaccaggcagattatccagactattattttaagatcacaaaatcagatcacatggccgacttgaaagaaaagtttaaaagaatgtgtgataagagtcaaatcagaaagaggtatatgcatttgaccgaggaaattttagaggaaaacccaaatatgtgcgcttacatggctccttctttggatgctaggcaagacatagtagttgtggaagttcccaagttgggaaaggcagctgcacagaaggcaataaaagaatggggtcagccaagatctaagataactcatttagtcttctgtactacttcaggtgttgatatgcccggcgctgactatcaattgacaaagatgttgggtttgagaccatcagttaaaaggttgatgatgtaccaacaaggatgttttgccggcggaaccgttttgagattggctaaagacttggctgagaacaatagaggagctagagtattggttgtttgcagtgaaattacagctgttacttttagaggcccacacgaatctcacttggattctttagtaggtcaagcattgtttggtgatggagctgccgcagtcattattggtgcagatccagatttatctgtcgaaagaccattgtttcaattagtctctgcctctcaaacaatattgccagactcagaaggtgctattgacggtcacttgagggaggtgggtttaacttttcatttgttaaaagacgtacctggattaattagtaagaatatagaaagagcattagaagaggctttcaaacctttaggcattgatcattggaattcagtgttctggattgcacatcagggtggtcctgctatcttagatatggttgaagccaaagttaacttaaacaaagaaagaatgagagccaccaggcatgtgttaagtgaatacggcaacatgtcctccgcatgcgtattattcatcatggatgagatgagaaagagatcagcagaggatggtcatgcaacaactggtgaaggaatggattggggtgtattattcggcttcggacctggtttaactgtcgagaccgtcgtcttacattccgtccctatctccgccggtgccactgcttga

SEQ ID NO: 31 - DNA, 1173 bp, Scutellaria baicalensis
atggttactgtcgaagaattccatagggctaccagggctgaaggtccagctaccgttttagccatcggtactgccaaccctcctaactgtgtcgagcaatccacctacgctgactactatttccgtatttgtaagtccgaacacctaaccgacttgaaaaagaagttcgaccgtatgtgtgaaaagtcctgtatcaagaagcgttacatgcacttgaccgaagaatttttaaaagagaatgataacttcactgcttatgaggctccttctttggacgctcgtcaagacatcgtcgttgtcgaaattcctaagttgggtaaggaagctgcccaaaaagctattaaggaatggggtcaaccaaagtctaaaattactcacgttatcttctgtaccacttctggtgttgacatgccaggtgccgactaccaaatcaccaagttattaggtttacgtccttccgtcaagagattcatgatgtaccaacaaggttgcttcgctggtggtaccgtcttaagaatggccaaggatttagccgagaataatgctggtgctagagtcctagttgtctgttccgagatcaccgctattaccttcagaggcccatctgatacccacttagattctttagttggtcaagccttattcggtgacggtgctgctgctgttattgttggttccgatccaatcgtcggtgttgaaagacctttgtttcaattggtttctgctgctcagactattttgccagactctgaaggtgctattgatggtcacgtcagagaagttggtttgactttccatttgttgaaggatgttccaggtttgatctctaaggacattgaaaagtctttgaaagaggctttcgctccattgggtatttccgattggaattccttgttttggattgttcatccaggtggtccagctatcctagatcaagtcggtgaaaagctaggtttgaagcctgaaatcatggtccctactagacacgttttgtctgaatacggtaacatgtcttctgcttgcgtcttgttcgtcatggatgaaatgcgtaaagcctctgctaaagatggttgtaccagcactggtgaaggtaaggactggggtgtcctatttggcttcggtccaggtttgactgttgaaaccgttgttttgcacagcgttcctttaaactaa

SEQ ID NO: 32 - DNA, 1170 bp, Malus domestica
atggtcaccgtcgaagaagttagaaaagctcaaagagctgaaggtccagctactgttttggctattggtactgctactccaccaaattgtgttgatcaagctacttacccagactactacttcagaattaccaactctgaacacaagaccgaattgaaagaaaagttccaaagaatgtgcgacaagtccatgatcaagaccagatatatgtacttgaccgaagaaatcttaaaagaaaacccaaccgtctgcgaatatatggctccatctttggatgctagacaagatatggttgttgttgaagttccaagattgggtaaagaagctgctactaaggctatcaaagaatggggtcaacctaagtctaagatcacccatttggttttctgtactacctctggtgttgatatgccaggtgctgattatcaattgactaagttgttgggtttaagaccatccgtcaagagattgatgatgtaccaacaaggttgttttgctggtggtacagttttgagattggcaaaagatttggccgaaaacaacaaaggtgctagagttttggttgtctgctctgaaattactgctgttacttttagaggtccatccgatactcatttggattctttggttggtcaagccttgtttggtgatggtgctgctgctgttattattggttctgatccagttcctgaagtcgaaaagccattattcgaattggtttctgctgcccaaactatcttgccagattcagatggtgctattgatggtcatttgagagaagttggtttgaccttccatttgttgaaagatgtcccaggtttgatttccaagaacatcgaaaagtctttgaacgaagccttcaagccaattggtatttctgattggaattccttgttctggattgctcatccaggtggtccagcaattttggatcaagttgaatctaagttggccttgaagccagaaaaattggaagctactagacaagtcttgtccgattacggtaatatgtcatctgcttgcgttttgttcatcttggatgaagtcagaagaaagtctgctgaaaagggtttgaaaactactggtgaaggtttggaatggggtgttttgtttggttttggtccaggtttaactgttgaaaccgttgtcttgcattctgttggtgcttaa

SEQ ID NO: 33 - DNA, 1176 bp, Malus domestica
atggttacagtcgaggaagttcgcaaggctcaacgggcggagggtccagccacagtcatggccatcgggacagcaactccttccaactgtgtggatcaggctacctaccccgactactactttcgtatcaccaacagcgagcacaaggttgagctcaaagaaaaattccagcgcatgtgcgacaaatctatgatcaagaaacgttatatgtacttgactgaagaaattttaaaagagaacccaagtgtgtgcgagtacatggctccttcaattgatgcaaggcaggacatggtggttgtggaagtcccaaaacttggcaaagaggctgccaccaaagccatcaaggaatggggacagcccaagtccaaaatcacccacttggtcttttgcaccaccagcggtgtcgacatgcctggcgccgactaccaactcaccaagctcttgggcctccgcccctccgtcaagcgcctcatgatgtaccagcaagggtgcttcgccggtgggacggtcctccgtttggccaaggacttggccgaaaacaacaagggtgcacgtgttcttgttgtgtgctctgagatcaccgcggttaccttccgtgggcctagtgacacccaccttgatagtcttgtgggccaagctttgtttggcgacggtgcagcggccgtaatcattggtgcggatccagtgcccgaagtcgagaagcccttgtttgaattggtgtcggcggcacaaaccattctccccgacagtgatggggctatcgacggacatctccgtgaagtagggcttacatttcaccttctcaaggatgttcccgggcttatttcgaagaacatcgaaaagagccttaatgaggctttcaagcctattgggatttcggactggaactcactcttctggattgcacacccaggtggccctgctattctggaccaagtagaggccaagttggcattgaagccggagaaactagaagcaacaaggcaagtgttgtcggattacggtaacatgtcgagtgcttgtgtgctttttattttggacgaggtcaggaggaagtccgccgagaaaggactcaaaacgaccggggagggactggagtggggtgtgcttttcggatttgggcccggcctcacggtggagaccgtcgtgcttcacagcgtgggtttaacggcttga

SEQ ID NO: 34 - DNA, 1170 bp, Malus domestica
atggtgaccgtcgaggaagttcgcaaggctcagagggctgagggtccggccacagtcttagctattgggactgcaactccttccaattgtgtagaccaggccacataccctgactactactttcgtatcaccaacagcgagcacaagactgagctcaaagaaaaatttcagcgcatgtgtgacaaatctatgatcaagaagcgttacatgtacttgactgaagaaattctgaaagaaaacccgactgtgtgcgagtacatggctccctcactcgatgctcggcaggacatggtggttgttgaagtcccaaggcttggcaaagaagcggccaccaaggcaattaaggaatggggacagcccaagtctaaaatcacccacttggtcttttgcaccaccagcggtgtcgacatgcccggtgccgactaccagctcaccaagctattgggcctccgcccatccgtcaagcgcctcatgatgtaccaacaaggctgttttgctggaggcacggtcctccgtttggccaaggacttggccgaaaacaacaagggtgcacgtgttcttgttgtgtgctctgagatcaccgcggtcaccttccgagggcctagtgacacccaccttgatagtcttgtgggccaagctttgtttggcgacggtgcagcggccgtcatcattggtgcagatccattgcccgaagtcgagaaacccttatttgagctagtgtctgctgcccaaaccatcctccccgacagtgatggggctattgacggacatcttcgtgaagttgggcttacatttcaccttctcaaggatgttcccgggcttatttcgaagaacatcgaaaagagccttaatgaggccttcaagcctataggcatctcggactggaactcgcttttctggattgcacaccctggtggccctgctattctagaccaagtagagtccaagttggcacttaagccggagaaactagaagcaacaaggcaagtgctgtctaattacggcaacatgtcaagtgcgtgtgtcttgtttattttggacgaggtgaggaggaaatccgctgagaaaggactcaaaacaactggagaaggactggagtggggcgtgctcttcggatttgggcctggcctcactgtcgagaccgttgtgcttcacagtgtggctgcttga

SEQ ID NO: 35 - DNA, 1170 bp, Malus domestica
atggtgaccgtcgaagaagttcgcaaggctcaacgggctgagggtccggccactgttttggccattgggacagcaactcctcccaactgtgtggatcaagccacataccccgactattactttcgtatcaccaacagtgagcacaagactgagctcaaagaaaaattccagcgcatgtgtgacaaatctatgatcaagacgcgttacatgtacttgactgaagaaattctgaaagagaacccaactgtgtgcgagtacatggctccctcactcgatgctcggcaggacatggtggttgttgaagtcccaaggcttggcaaagaggctgccaccaaggccattaaggaatggggacagcccaagtccaaaatcacccacttggtcttttgcaccaccagcggtgtcgacatgcccggcgccgactaccaactcaccaagctcttgggcctccgcccctccgtcaagcgcctcatgatgtaccaacaaggttgcttcgccggcgggacggtcctccgtttggccaaggacttggccgagaacaacaagggtgcacgtgttcttgttgtgtgctctgagatcaccgcagtcaccttccgcgggcctagtgacacccaccttgacagtcttgtgggtcaagccttgtttggtgacggcgcagcggccgtcatcattggttcggatccagtgcccgaagtcgagaagcccttgtttgaattggtgtcagcagcacaaaccattcttcccgacagtgatggggctattgacggccatctccgtgaagtagggcttacatttcaccttctcaaggacgttcctgggcttatttccaagaatatcgaaaagagccttaacgaggccttcaagcctataggcatttcagactggaactcgctcttctggattgcacacccaggtggccctgctattctggaccaagtagagtccaagttggcccttaagccggagaaactagaagctacaaggcaagtgctgtctgattacggcaacatgtcgagtgcgtgtgtcttgtttattttggacgaagtgaggaggaagtctgctgagaaaggactcaaaacaactggagaaggactggagtggggcgtactcttcggatttgggcctggcctcactgttgagaccgttgtgcttcacagtgtgggtgcttga

SEQ ID NO: 36 - DNA, 1170 bp, Malus domestica
atggtgactgtccaggaagttcgcaaggctcaacgggctgagggtccggccacagtattcgccattgggacagcaactcctcccaattgtgtggaccaagccacataccccgactattactttcgtatcaccaacagtgagcacaaggctgagctcaaagaaaaattccagcgcatgtgtgacaaatctatgatcaagaagcgttacatgtacttgactgaggaaattctaaaggagaatccaagtgtgtgcgagtacatggcaccatcacttgatgctcggcaggacatggtggttgttgaagtcccaaggcttggcaaagaggctgccaccaaggccatcaaggaatggggacagcccaagtccaaaatcacccacttggtcttttgcaccaccagcggtgtcgacatgcccggcgctgactaccagctcaccaagctattgggcctccgcccctctgttaagcgcctcatgatgtaccaacaaggttgtttcgctggaggcacggttctccgtttggccaaggacttggccgaaaacaacaagggtgcacgtgttcttgttgtgtgctctgagatcaccgcggtcaccttccgtgggcctagtgacacccaccttgacagtcttgtgggtcaagccttgtttggcgacggtgcagcggccgtcatcattggtgccgacccagtgcccgaagtcgagaagcccttgtttgaattggtctcggcggcacaaaccattctcgctgacagtgatggggctatcgacggacatctccgtgaagtagggcttacgtttcaccttttgaaggacgttcccgggcttatttcaaagaacatcgaaaagagccttaacgaggccttcaagcctataggcatttcggactggaactcactcttctggattgcacacccaggtggccctgctattctggaccaagtagaggccaagttggcgttgaagccggagaaattagaagcgacaaggcaagtgttgtcagattacggcaacatgtcgagtgcgtgtgtcttgtttattttggacgaggtgaggaggaagtcagctgagaaaggactggagacaactggagaaggactggaatggggtgtgctatttggatttgggcctggcctcacggtggagaccgtcgtgcttcacagcgtggctgcttga

SEQ ID NO: 37 - DNA, 1179 bp, Vitis pseudoreticulata
atggcctccgttgaagaaattagaaatgctcaaagagctaagggtccagctactattttggctattggtactgctactccagatcattgtgtttaccaatctgattacgccgactactacttcagagttactaagtctgaacacatgaccgaattgaagaaaaagttcaacagaatctgcgacaagtccatgatcaagaagagatatatccacttgaccgaagaaatgttggaagaacatccaaacattggtgcttatatggctccatccttgaacatcagacaagaaattatcactgccgaagttccaaagttgggtaaagaagctgctttgaaggctttgaaagaatggggtcaacctaagtctaagatcacccatttggttttctgtactacctctggtgttgaaatgccaggtgctgattacaaattggctaacttgttgggtttggaaacctctgttagaagagttatgttgtaccatcaaggttgttatgctggtggtactgttttgagaactgctaaagatttggctgaaaacaatgctggtgctagagttttggttgtttgctctgaaattaccgttgttactttcagaggtccatctgaagatgctttggattctttggttggtcaagctttgtttggtgatggttctgctgctgttatagttggttctgatccagatatctccatcgaaagacctttgttccaattggtttcagctgctcaaactttcattccaaattctgctggtgcaattgctggtaacttgagagaagttggtttgacttttcatttgtggccaaacgttccaactttgatctccgaaaacattgaaaactgtttgaccaaggcctttgatccaatcggtatttctgattggaattccttgttctggattgctcatccaggtggtccagcaattttggatgctgttgaagctaaggttggtttggataagcaaaagttgaaggccaccagacacattttgtctgaatacggtaatatgtcctctgcctgcgttttgtttattttggacgaaatgagaaagaagtccttgaaagaaggtaagactactacaggtgaaggtttggattggggtgttttgttcggttttggtccaggtttgactattgaaactgttgtcttgcattccgttggtactgattctaactga

SEQ ID NO: 38 - DNA, 1179 bp, Vitis vinifera
atggcctctgttgaagaattcagaaatgctcaaagagctaaaggtccagctaccattttggctattggtactgctactccagatcattgtgtttaccaatctgattacgccgactactacttcagagttactaagtctgaacacatgaccgaattgaagaaaaagttcaacagaatctgcgacaagtccatgatcaagaagagatatatccacttgaccgaagaaatgttggaagaacatccaaacattggtgcttatatggctccatccttgaacatcagacaagaaattatcactgccgaagttccaagattgggtagagatgctgctttgaaggctttgaaagaatggggtcaacctaagtctaagatcacccatttggttttctgtactacctctggtgttgaaatgccaggtgctgattacaaattggctaacttgttgggtttggaaacttccgttagaagagttatgttgtaccatcaaggttgttatgctggtggtactgttttgagaactgctaaagatttggctgaaaacaatgctggtgctagagttttggttgtttgctctgaaattaccgttgttactttcagaggtccatctgaagatgctttggattctttggttggtcaagctttgtttggtgatggttcttctgctgttatagttggttctgatccagatgtctctatcgaaagacctttgttccaattggtttctgctgctcaaactttcattccaaattctgctggtgcaattgctggtaacttgagagaagttggtttgacttttcatttgtggccaaacgttccaactttgatctccgaaaacattgaaaagtgtttgacccaagctttcgatccattgggtatttctgattggaattccttgttctggattgctcatccaggtggtccagcaattttggatgctgttgaagctaaattgaacttggaaaagaagaagttggaagccaccagacatgttttgtctgaatacggtaatatgtcctctgcttgcgttttgttcattttggacgaaatgagaaaaaagtccttgaagggtgaaaaggctactactggtgaaggtttggattggggtgttttgttcggttttggtccaggtttgactattgaaactgttgtcttgcattctgttccaaccgttaccaattga

SEQ ID NO: 39 - DNA, 1179 bp, Malus domestica
atggctactaccgctgcttcttctttacaaatggcaactgctagaccatgcatctcttcatctagaagagcttttggttcttctaccgctatgttgaatggtaactttaaggttgcttcctggaccaaattatcttccgcttgtcatatctcctctgtccaatcttttcaaagatgcttcacctcctcatctatgaagttggataagttcgttactaaggctatggctggtgcttctgaaaacaaaccagtttctggtttgccaatcaacttgaaaggtaagagagctttcattgctggtgttgctgatgataatggttatggttgggctattgctaaatctttggctgctgctggtgctgaaattttggttggtacttgggttccagccttgaatattttcgaatcctctttgagaagaggtaagttcgacgaatctagaattttgccagatggttccttgatggaaatcactaaggtttatccattggatgccgttttcgataacccagaagatgttccagaagaaatcaagaccaacaaaagatacgctggttcctctaattggactgttcaagaagctgctgaatgcgttaagaatgatttcggttccatcgatgttttggttcactctttggctaatggtccagaagttgttaagcctttgttggaaacttctagaaagggttacttggctgctatttctgcttcatcttactcctacgtcagtttgttgaaacacttcttgccaattatcaacccaggtggttcttccatttctttgacttacattgcctccgaaagaatcattccaggttatggtggtggtatgtcatctgctaaagctgctttggaatctgatacaagagttttggcttttgaagccggtagaaagaagggtattagagttaataccatttccgctggtccattgagatcaagagctgcaaaagctattggtttcatcgatatgatgatcgactactcttctgctaatgccccattggaaaaagaattgtctgctgaagaagttggtaacactgctgcttttttggcttctccattggcttcagctattactggtggtgttatctatgttgacaatggtttgaatgctatgggtgttggtgttgactctccaatcttcgaaaatttgaacattccaaaggcccaacattaa

SEQ ID NO: 40 - DNA, 1179 bp, Malus domestica
atggctactaccgctgcttcttctttacaaatggcaactgctagaccatgcatctcttcatctagaagagcttttggttcctcctccaaaatgttgaacgataactttaaggttgcctcctggtctaagttatcttctacttgtcatacctcctccgtccaatcttttcaaagatcctttacctcctcatccatgaagatggataagttcgttactagagctatggctggtgcttctgaaaacaaaccagtttctggtttgccaatcgatttgaaaggtaagagagctttcattgctggtgttgctgatgataatggttatggttgggctattgctaaatctttggctgctgctggtgctgaaattttggttggtacttgggttccagccttgaatattttcgaatcctctttgagaagaggtaagttcgatgaatctagagttttgccagatggttccttgatggaaattactaaggtttacccattggatgccgttttcgataatccagaagatgttccagaagaaatcaagaccaacaaaagatacgctggttcttctaactggactgttcaagaagctgctgaatgtgttaagaacgatttcggttccattgatatcttggtccattctttggctaatggtccagaagttgttaagcctttgttggaaacttctagaaagggttacttggctgctatttctgcttcatcttactcctacgtcagtttgttgaaacacttcttgccaattatcaacccaggtggttcttccatttctttgacttacattgcctccgaaagaatcattccaggttatggtggtggtatgtcatctgctaaagctgctttggaatctgatacaagagttttggcttttgaagccggtagaagaaagggtattagagttaacacaatttccgctggtccattgagatcaagagctgcaaaagctattggtttcatcgatatgatgatcgactactcttctgctaatgccccattggaaaaagaattgtctgctgatgaagttggtaacactgctgcttttttggcttctccattggcttcagctattactggtggtgttatctatgttgacaatggtttgaatgctatgggtgttggtgttgactctccaatcttcgaaaatttgaacattccaaaggcccaacattaa

SEQ ID NO: 41 - DNA, 1047 bp, Rubus idaeus
atggcttctggtggtgaaatgcaagtctctaacaagcaagttatcttcagagattacgttaccggtttcccaaaagaatccgatatggaattgaccaccagatccattactttgaaattgccacaaggttctaccggtttgttgttgaaaaacttgtacttgtcttgcgacccttacatgagagctagaatgactaatcatcacagattgtcctacgtcgattcttttaaaccaggttccccaattattggttacggtgttgctagagttttggaatctggtaatccaaagtttaacccaggtgatttggtttggggttttactggttgggaagaatactctgttattaccgctactgaatccttgttcaagatccataataccgatgtcccattgtcttactacactggtttgttgggtatgccaggtatgactgcttatgctggtttttacgaaatttgctctccaaaaaagggtgaaaccgtttatgtttctgctgcttcaggtgctgttggtcaattggtcggtcaatttgctaagttgactggttgttatgttgttggttctgccggttctaaagaaaaggttgatttgttgaagaacaagttcggtttcgatgaagccttcaactacaaagaagaagctgatttggacgctgctttgagaagatattttccagatggtatcgacatctacttcgaaaatgttggtggtaagatgttggatgctgttttgccaaatatgagaccaaagggtagaattgctgtttgcggtatgatttcccaatacaacttggaacaaccagaaggtgttagaaacttgatggctttgatcgttaagcaagtcagaatggaaggtttcatggttttctcttactaccacttgtacggtaaattcttggaaactgtcttgccttacatcaagcaaggtaagattacctacgttgaagatgttgttgatggtttggataatgctccagctgctttaattggtttgtactctggtagaaacgtcggtaagcaagttgttgttgtttccagagaatga

SEQ ID NO: 42 - DNA, 2037 bp, Eubacterium ramulus
atggccgaaaagaatcaatacttcccacacttgtttgaaccattgaaggttggttctaagaccatcaagaacagaattgaagctgctccagctttgtttgctttcgaacattacattgaattgaacccagatccattcggttacactactccagttccagaaagagcttttagaatgttggaagctaaagctaaaggtggtgctggtatagtttgtttgggtgaattgtctccaaaccacgaatacgataagagatttccattcgaaccatacttggacttcacttccagatccgataagcaattcgaaatcatgaaagaaaccgccgaaatgatcaaatcttacggtgcttttccaatgggtgaattattgtcttgtggtgaaatcaagaccaacatcggtgatggtattaacccaaaaggtccatctgaaaaggatttgccagatggttctcatgttgaagcctttaccaaagaagaaatcttgtcctgctaccaagattacgttactgcttgtaaatggtttcaagctgctggttgggaaggtattatgattcattgtggtcatggttggttgccagctcaatttttgtctccacaatacaacaagagaaccgatgaatacggtggttcttttgaaaacagagctagattcaccgtcgacttgttgaaaactgttagagaagctatgggtccagatttcgtcattgaaatcagagtctcttcctctgaacatttgcctggtggtttagaattggaagatgctgttaattactgcaagttgtgcgaaccttacatcgatatgatccatgtttcttgcggtcactacttgtcatcttctagatcatgggaattcactactgcttatgctccacatggtccaaatattgaaccagctgctgttatcaagcaaaacgtttctattccagttgctgctgttggtggtatcaattctccagaacaagctgaagaagctattgcctctggtaagattgatatggtttctatgggtagacaattcttcgctgatccagcatttcctaacaaagcaaaagaaggtcacgctgacgaaattagaagatgtttgagatgtggtagatgttacccaggtccatcaggtgaacacgaaactgaaatttggactgttaagttcccaccattggattcttgtaccattaacccatatgatgtttggccagcttctcatcataaggttttaccagatagaatgccaaaaccagaagcctctagaaaggttttggttgtaggtggtggttgcggtggtttacaaactgctattactgcttctgatagaggtcaccaagttatcttgtgtgaaaagtctggtgttttgggtggtttgattaacttcactgatcataccgatcacaaggtcgatatcagaaacttcaaggatttgttgatcagagatgttgaaaaaagaccaatcgaagtcagattgaactgtgaagttaccccagaattgattagagaaattgctccagaagctgttgttttggctgttggttctgatgatttgatcttgccaattgaaggtatcgaaaacgctgttactgctatggatgtttactctaatgatttcgccggtttgggtaaatccactatagtattgggtggtggtttggttggttgtgaagctgctgctgattatattgatcatggtgttgaaaccaccatcgtcgaaatgaagggtgctttgatgccagaaactactggtttgtatagaaccgctgttcacgatttcattgataagaatggtggtaagtacgaagttaacgccaaggttgttaaggttggtaaggattttgttgttgccgaacaagacggtaaagaaattaccattaaggccgattctgttgtcaatgcaatgggtagaagagcacatgctactgaagccttggaaacagctatcaaagaagctggtattccagtctggaaaattggtgattgtgttagagctagacaaatcggtgacgctgtaagagaaggttggactgcagctatggaaattatctga

SEQ ID NO: 43 - DNA, 762 bp, Saccharomyces cerevisiae
atgtactttgatgaagaacaattgctaaaatatactatatatgcctatagattatccttttttgtaggcatttgctcacttttcatagcaaaaagttgtctaccagaatttcttcaatatggtaaaacctaccggcccaaagagaattcaaagtactcaagcattttagaacgaatcaagaagttcacagttccaaaggcgtatttttcccatttttactatttggctacctttctatccttagtcaccttatatttctatcctaaattccccatcgtttggatcatatttggacactcattgcgccgactttatgaaacgctttatgtactacattatacaagcaattctaggatgaattggtcccattatctagtcggtatatggttctattccgtactcttgttaattcttaatatatcactgtacaagaactccattccaaatacgttaaacatgaatgctttcatcatattctgcatagcatcttgggatcagtacaaaaatcatgttattctggccaatctggttaaatattcgctgccaacaggaaggcttttcaggttggtatgctgtcctcattatctcgatgaaataatcatttattctactctgttgccctatgaacaagaattttacctaacactagtttgggtaatcacaagtttgactatatccgcattggaaacaaaaaattattacaggcacaaatttaaagacaatcacgtagccccctacgccataataccttttataatctag

SEQ ID NO: 44 - DNA, 1050 bp, Malus domestica
atggctgcttctaccgaaggtgttatctctaacaagcaagttatcttgaaggattacgttaccggtttcccaaaagaatccgatatgcaattgactactgctaccactaagttgaaattgcctgaaggttctaaaggtgtcttggtcaaaaacttgtacttgtcttgtgacccttacatgagatccagaatgacaaaaagagaaccaggtgcttcttacgttgattcatttgatgctggttctccaatcgttggttatggtgttgctaaagttttggaatctggtgacccaaagtttaagaagggtgatttgatttggggtatgactggttgggaagaatactctgttattacctctaccgaatccttgttcaagatccaacatatcgatgtcccattgtcttactacactggtattttgggtatgccaggtatgacagcttatgctggtttttacgaaatctgcaatccaaaaaagggtgaaaccgtttttgtttctgctgcttctggtgctgttggtcaattggtcggtcaatttgctaagttgttgggttgttatgttgttggttctgccggttccaaagaaaaggttgatttgttgaagaacaagttcggtttcgataacgccttcaactacaaagaagaaccagatttggacgctgctttgaagagatattttccagaaggtatcgacatctacttcgaaaatgttggtggtaagatgttggatgctgttttgccaaatatgagagttcatggtagaattgctgtttgcggtttgatctcccaatacaacattgatgaaccagaaggttgcagaaacttgatgtacttgattatcaagcaagtcagaatgcaaggtttcttggttttctcttactaccacttgtacgaaaagttcttggaaatggttttgccagccatcaaagaaggtaaattgacctacgttgaagatgtcgttgaaggtttagaatctgctccagctgctttaattggtttgtatgctggtagaaacgttggtaagcaagttgttgttgtctccagagaatga

SEQ ID NO: 45 - DNA, 933 bp, Arabidopsis thaliana
atgaaggtcaccgtcgtttctagatcaggtagagaagttttgaaagccccattggatttgccagattctgctactgttgctgacttgcaagaagcctttcataagagagctaagaagttctacccatccagacaaagattgactttgccagttactccaggttctaaagataagccagttgtcttgaactccaagaagtccttgaaagaatactgtgacggtaacaacaactccttgactgttgtttttaaggatttgggtgcccaagtttcttacagaactttgttcttcttcgaatacttgggtcctttgttgatctacccagttttttactacttcccagtctacaagtttttgggttacggtgaagattgcgttatccatccagttcaaacttacgctatgtactactggtgtttccactacttcaagagaatcttggaaaccttcttcgtccacagattttctcatgctacttctccaattggtaacgttttcagaaactgtgcctattactggtctttcggtgcttatattgcttactacgttaaccacccattatacactccagtttcagacttgcaaatgaagattggttttggtttcggtttggtctgtcaagttgctaacttctactgccatatcttgttgaagaacttgagagatccatctggtgctggtggttatcaaattccaagaggttttttgttcaacatcgttacctgtgctaactacactaccgaaatctatcaatggttgggtttcaacattgccactcaaactattgctggttacgtttttttggctgttgccgctttgattatgactaattgggctttgggtaagcactccagattgagaaagattttcgatggtaaagacggtaagccaaagtatccaagaagatgggttattttgccaccattcttgtaa

SEQ ID NO: 46 - DNA, 933 bp, Gossypium hirsutum
atgaaggtcaccttggtcagtagatcaggtagagaattcattaagggtggtttggaattgaacgattctgctactgttgctgacttgcaagaagctattcataagagaactaagaagttctacccatccagacaaagattgactttgccagttccatctggttctagagaaagaccagttatcttgaactacaagaagtccttgaaggattactgtgacggtaacgaaaacactttgaccatcgtttttaaggacttgggtccacaagtttcttacagaactttgttcttcttcgaatatttgggtccattgatcttgtacccagttttctattacttcccagtctacaagtacttcggttacgaagaaaagagagttatccacccagttcaaacttatgccttgtactactggtgtttccactacttcaagagaattatggaaaccttcttcatccacagattctctcatgctacttctccattgtctaacgttttcagaaactgtgcttactactggactttcggttcttatattgcctactacgttaaccacccattatacactccagtttcagacttgcaaatgaagattggttttggtttcggtatcgtttgtcaattggctaacttctactgccacatcatcttgaagaatttgagatcaccagatggttctggtggttaccaaattccaagaggttttttgttcaacatcgttacctgtgctaactacactaccgaaatctatcaatggttgggtttcaacattgctactcaaacagttgctggttacgttttcttggttgttgctacctctattatgactaattgggccttggctaaacacagaagattgaagaaattattcgacggtaaggacggtagaccaaagtatccaagaagatgggttattttgccaccattcttgtaa

SEQ ID NO: 47 - DNA, 933 bp, Malus domestica
atgaaggtcaccgtcgtttctagatcaggtagagaagttgttaagggtggtttggaattgtctgattctgctactgttgctgacttgcaagatgctattcataagagaactaagaagttctacccagccagacaaagattgactttgccagttcaaccaggttctaaagaaagaccagttgtcttgtcttacaagaagtcattgcaagactacatctccggtaactctgataacttgactgttgttttcaaggacttgggtccacaagtttcttacagaactttgttcttcttcgaatatttgggtccattgatcttgtacccaatcttctactacttcccagtttacgattacttgggtttcaagggtgatagagttatccatccagttcaaacttatgccttgtactactggtgtttccactacttcaagagaattatggaaaccttcttcgtccacagattctctcatgctacttctccattgtctaacgttttcagaaactgtgcctactattggtctttcggtgcttttattgcttactacttgaaccacccattatacactccagtttcagacttgcaaatgaagattggtttcggtattggtatcatctgccaaatctctaacttctactgccacatcttgttgagaaacttgagatcaccagatggtaatggtggttaccaaattccaagaggtttcttgttcaacatcgttacctgtgctaactacactaccgaaatctatcaatggttgggttttaacattgccactcaaacagttgccggttacatttttttgatcgttgctgcttctatcatgaccaattgggctttggctaaacacagaagattgaagaaaatcttcgatggtaaggacggtagaccaaagtatccaagaagatgggttattttgccaccattcttgtaa

SEQ ID NO: 48 - DNA, 960 bp, Kluyveromyces lactis
atgtccgcctcctcctccattttcatcaaatctagatccaagtccttgaaggacgttaagttagaagttccaactgaaaacaccttgacctaccaatccgttttacaacaaatctccaagtccaaccacaacatctccgttaatagattgagattgtcctacttgaaagaaggtaagcaagttgctattggtccatccgaattgaatgatgttggtaagaagaacaccttcgactctgttaatgaatggtatgtcaaagacttgggtccacaaattagttggagattggttttcttcatcgaatatttgggtccaatcttgatccactccttggtttatttgttgtctttgaacgctaccgtcagagataagttccattctaagaatgttccatacaacgatttcttcaacaagttcatctacagattgatcatggtccactacttgaagagagaattcgaaaccttgttcatccattccttctcattggaaactatgcctttgttcaacttgttcaaaaactccttccactactggatcttgaacggtttgatttctttgggttacttcggttacggttttccatttgctaacaagaccttgtacagagtttactccgctttgaagatttccgatttcagagttttgactgccttgttcggtttgtctgaaatgtttaacttctacatccacgtcgctttgagaagatggggtgatgaacaaaaaagaaacggtgttactaagagagtcccattgaattctggtttgtttaagttgttggttgccccaaactacacttttgaatcttgggcttggatgttcttcaccttgttgttcaagttgaatttgttctccgtcttgttcttggttgtttccgttgttcaaatgtacttgtgggcccaaaagaaaaacaagaagtacggtacaaagagagccttcttgattccattcttgttctaa

SEQ ID NO: 49 - protein, 390 aa, Hypericum androsaemum
MVTVEEVRKAQRAEGPATVMAIGTAVPPNCVDQATYPDYYFRITNSEHKAELKEKFQRMCDKSQIKKRYMYLNEEVLKENPNMCAYMAPSLDARQDIVVVEVPKLGKEAAVKAIKEWGQPKSKITHLVFCTTSGVDMPGADYQLTKLLGLRPSVKRLMMYQQGCFAGGTVLRLAKDLAENNKGARVLVVCSEITAVTFRGPTDTHLDSLVGQALFGDGAAAIIIGSDPIPEVEKPLFELVSAAQTILPDSEGAIDGHLREVGLTFHLLKDVPGLISKNVEKSLTEAFKPLGISDWNSLFWIAHPGGPAILDQVEAKLSLKPEKLRATRHVLSEYGNMSSACVLFILDEMRRKSKEDGLKTTGEGIEWGVLFGFGPGLTVETVVLHSVAIN

SEQ ID NO: 50 - protein, 398 aa, Petroselinum crispum
MANHHNAEIEEIRNRQRAQGPANILAIGTATPSNCVYQADYPDYYFRITNSEHMTDLKLKFKRMCEKSMIRKRYMHITEEYLKENPNVCAYEAPSLDARQDLVVVEVPRLGKEAASKAIKEWGQPKSKITHLIFCTTSGVDMPGADYQLTKLLGLRPSVKRFMMYQQGCFAGGTVLRLAKDLAENNAGARVLVVCSEITAVTFRGPSDSHLDSLVGQALFGDGAAAVILGSDPDLSVERPLFQLISAAQTILPDSDGAIDGHLREVGLTFHLLKDVPGLISKNIEKSLKEAFGPIGISDWNSLFWIAHPGGPAILDQVELKLGLKEEKMRATRQVLSDYGNMSSACVLFILDEMRKKSIEEGKATTGEGLDWGVLFGFGPGLTVETVVLHSVPATFTH

SEQ ID NO: 51 - protein, 389 aa, Petunia hybrida
MVTVEEYRKAQRAEGPATVMAIGTATPTNCVDQSTYPDYYFRITNSEHKTDLKEKFKRMCEKSMIKKRYMHLTEEILKENPSMCEYMAPSLDARQDIVVVEVPKLGKEAAQKAIKEWGQPKSKITHLFFCTTSGVDMPGCDYQLTKLLGLRPSVKRLMMYQQGCFAGGTVLRLAKDLAENNKGARVLVVCSEITAVTFRGPNDTHLDSLVGQALFGDGAGAIIIGSDPIPGVERPLFELVSAAQTLLPDSHGAIDGHLREVGLTFHLLKDVPGLISKNIEKSLEEAFKPLGISDWNSLFWIAHPGGPAILDQVEIKLGLKPEKLKATRNVLSDYGNMSSACVLFILDEMRKASAKEGLGTTGEGLEWGVLFGFGPGLTVETVVLHSVAT

SEQ ID NO: 52 - protein, 398 aa, Hordeum vulgare
MAATMTVEEVRNAQRAEGPATVLAIGTATPANCVYQADYPDYYFKITKSDHMADLKEKFKRMCDKSQIRKRYMHLTEEILEENPNMCAYMAPSLDARQDIVVVEVPKLGKAAAQKAIKEWGQPRSKITHLVFCTTSGVDMPGADYQLTKMLGLRPSVKRLMMYQQGCFAGGTVLRLAKDLAENNRGARVLVVCSEITAVTFRGPHESHLDSLVGQALFGDGAAAVIIGADPDLSVERPLFQLVSASQTILPDSEGAIDGHLREVGLTFHLLKDVPGLISKNIERALEEAFKPLGIDHWNSVFWIAHQGGPAILDMVEAKVNLNKERMRATRHVLSEYGNMSSACVLFIMDEMRKRSAEDGHATTGEGMDWGVLFGFGPGLTVETVVLHSVPISAGATA

SEQ ID NO: 53 - protein, 390 aa, Scutellaria baicalensis
MVTVEEFHRATRAEGPATVLAIGTANPPNCVEQSTYADYYFRICKSEHLTDLKKKFDRMCEKSCIKKRYMHLTEEFLKENDNFTAYEAPSLDARQDIVVVEIPKLGKEAAQKAIKEWGQPKSKITHVIFCTTSGVDMPGADYQITKLLGLRPSVKRFMMYQQGCFAGGTVLRMAKDLAENNAGARVLVVCSEITAITFRGPSDTHLDSLVGQALFGDGAAAVIVGSDPIVGVERPLFQLVSAAQTILPDSEGAIDGHVREVGLTFHLLKDVPGLISKDIEKSLKEAFAPLGISDWNSLFWIVHPGGPAILDQVGEKLGLKPEIMVPTRHVLSEYGNMSSACVLFVMDEMRKASAKDGCTSTGEGKDWGVLFGFGPGLTVETVVLHSVPLN

SEQ ID NO: 54 - protein, 391 aa, Malus domestica
MVTVEEVRKAQRAEGPATVMAIGTATPSNCVDQATYPDYYFRITNSEHKVELKEKFQRMCDKSMIKKRYMYLTEEILKENPSVCEYMAPSIDARQDMVVVEVPKLGKEAATKAIKEWGQPKSKITHLVFCTTSGVDMPGADYQLTKLLGLRPSVKRLMMYQQGCFAGGTVLRLAKDLAENNKGARVLVVCSEITAVTFRGPSDTHLDSLVGQALFGDGAAAVIIGADPVPEVEKPLFELVSAAQTILPDSDGAIDGHLREVGLTFHLLKDVPGLISKNIEKSLNEAFKPIGISDWNSLFWIAHPGGPAILDQVEAKLALKPEKLEATRQVLSDYGNMSSACVLFILDEVRRKSAEKGLKTTGEGLEWGVLFGFGPGLTVETVVLHSVGLTA

SEQ ID NO: 55 - protein, 389 aa, Malus domestica
MVTVEEVRKAQRAEGPATVLAIGTATPSNCVDQATYPDYYFRITNSEHKTELKEKFQRMCDKSMIKKRYMYLTEEILKENPTVCEYMAPSLDARQDMVVVEVPRLGKEAATKAIKEWGQPKSKITHLVFCTTSGVDMPGADYQLTKLLGLRPSVKRLMMYQQGCFAGGTVLRLAKDLAENNKGARVLVVCSEITAVTFRGPSDTHLDSLVGQALFGDGAAAVIIGADPLPEVEKPLFELVSAAQTILPDSDGAIDGHLREVGLTFHLLKDVPGLISKNIEKSLNEAFKPIGISDWNSLFWIAHPGGPAILDQVESKLALKPEKLEATRQVLSNYGNMSSACVLFILDEVRRKSAEKGLKTTGEGLEWGVLFGFGPGLTVETVVLHSVAA

SEQ ID NO: 56 - protein, 389 aa, Malus domestica
MVTVEEVRKAQRAEGPATVLAIGTATPPNCVDQATYPDYYFRITNSEHKTELKEKFQRMCDKSMIKTRYMYLTEEILKENPTVCEYMAPSLDARQDMVVVEVPRLGKEAATKAIKEWGQPKSKITHLVFCTTSGVDMPGADYQLTKLLGLRPSVKRLMMYQQGCFAGGTVLRLAKDLAENNKGARVLVVCSEITAVTFRGPSDTHLDSLVGQALFGDGAAAVIIGSDPVPEVEKPLFELVSAAQTILPDSDGAIDGHLREVGLTFHLLKDVPGLISKNIEKSLNEAFKPIGISDWNSLFWIAHPGGPAILDQVESKLALKPEKLEATRQVLSDYGNMSSACVLFILDEVRRKSAEKGLKTTGEGLEWGVLFGFGPGLTVETVVLHSVGA

SEQ ID NO: 57 - protein, 389 aa, Malus domestica
MVTVQEVRKAQRAEGPATVFAIGTATPPNCVDQATYPDYYFRITNSEHKAELKEKFQRMCDKSMIKKRYMYLTEEILKENPSVCEYMAPSLDARQDMVVVEVPRLGKEAATKAIKEWGQPKSKITHLVFCTTSGVDMPGADYQLTKLLGLRPSVKRLMMYQQGCFAGGTVLRLAKDLAENNKGARVLVVCSEITAVTFRGPSDTHLDSLVGQALFGDGAAAVIIGADPVPEVEKPLFELVSAAQTILADSDGAIDGHLREVGLTFHLLKDVPGLISKNIEKSLNEAFKPIGISDWNSLFWIAHPGGPAILDQVEAKLALKPEKLEATRQVLSDYGNMSSACVLFILDEVRRKSAEKGLETTGEGLEWGVLFGFGPGLTVETVVLHSVAA

SEQ ID NO: 58 - protein, 392 aa, Vitis pseudoreticulata
MASVEEIRNAQRAKGPATILAIGTATPDHCVYQSDYADYYFRVTKSEHMTELKKKFNRICDKSMIKKRYIHLTEEMLEEHPNIGAYMAPSLNIRQEIITAEVPKLGKEAALKALKEWGQPKSKITHLVFCTTSGVEMPGADYKLANLLGLETSVRRVMLYHQGCYAGGTVLRTAKDLAENNAGARVLVVCSEITVVTFRGPSEDALDSLVGQALFGDGSAAVIVGSDPDISIERPLFQLVSAAQTFIPNSAGAIAGNLREVGLTFHLWPNVPTLISENIENCLTKAFDPIGISDWNSLFWIAHPGGPAILDAVEAKVGLDKQKLKATRHILSEYGNMSSACVLFILDEMRKKSLKEGKTTTGEGLDWGVLFGFGPGLTIETVVLHSVGTDSN

SEQ ID NO: 59 - protein, 392 aa, Vitis vinifera
MASVEEFRNAQRAKGPATILAIGTATPDHCVYQSDYADYYFRVTKSEHMTELKKKFNRICDKSMIKKRYIHLTEEMLEEHPNIGAYMAPSLNIRQEIITAEVPRLGRDAALKALKEWGQPKSKITHLVFCTTSGVEMPGADYKLANLLGLETSVRRVMLYHQGCYAGGTVLRTAKDLAENNAGARVLVVCSEITVVTFRGPSEDALDSLVGQALFGDGSSAVIVGSDPDVSIERPLFQLVSAAQTFIPNSAGAIAGNLREVGLTFHLWPNVPTLISENIEKCLTQAFDPLGISDWNSLFWIAHPGGPAILDAVEAKLNLEKKKLEATRHVLSEYGNMSSACVLFILDEMRKKSLKGEKATTGEGLDWGVLFGFGPGLTIETVVLHSVPTVTN

SEQ ID NO: 60 - protein, 392 aa, Malus domestica
MATTAASSLQMATARPCISSSRRAFGSSTAMLNGNFKVASWTKLSSACHISSVQSFQRCFTSSSMKLDKFVTKAMAGASENKPVSGLPINLKGKRAFIAGVADDNGYGWAIAKSLAAAGAEILVGTWVPALNIFESSLRRGKFDESRILPDGSLMEITKVYPLDAVFDNPEDVPEEIKTNKRYAGSSNWTVQEAAECVKNDFGSIDVLVHSLANGPEVVKPLLETSRKGYLAAISASSYSYVSLLKHFLPIINPGGSSISLTYIASERIIPGYGGGMSSAKAALESDTRVLAFEAGRKKGIRVNTISAGPLRSRAAKAIGFIDMMIDYSSANAPLEKELSAEEVGNTAAFLASPLASAITGGVIYVDNGLNAMGVGVDSPIFENLNIPKAQH

SEQ ID NO: 61 - protein, 392 aa, Malus domestica
MATTAASSLQMATARPCISSSRRAFGSSSKMLNDNFKVASWSKLSSTCHTSSVQSFQRSFTSSSMKMDKFVTRAMAGASENKPVSGLPIDLKGKRAFIAGVADDNGYGWAIAKSLAAAGAEILVGTWVPALNIFESSLRRGKFDESRVLPDGSLMEITKVYPLDAVFDNPEDVPEEIKTNKRYAGSSNWTVQEAAECVKNDFGSIDILVHSLANGPEVVKPLLETSRKGYLAAISASSYSYVSLLKHFLPIINPGGSSISLTYIASERIIPGYGGGMSSAKAALESDTRVLAFEAGRRKGIRVNTISAGPLRSRAAKAIGFIDMMIDYSSANAPLEKELSADEVGNTAAFLASPLASAITGGVIYVDNGLNAMGVGVDSPIFENLNIPKAQH

SEQ ID NO: 62 - protein, 348 aa, Rubus idaeus
MASGGEMQVSNKQVIFRDYVTGFPKESDMELTTRSITLKLPQGSTGLLLKNLYLSCDPYMRARMTNHHRLSYVDSFKPGSPIIGYGVARVLESGNPKFNPGDLVWGFTGWEEYSVITATESLFKIHNTDVPLSYYTGLLGMPGMTAYAGFYEICSPKKGETVYVSAASGAVGQLVGQFAKLTGCYVVGSAGSKEKVDLLKNKFGFDEAFNYKEEADLDAALRRYFPDGIDIYFENVGGKMLDAVLPNMRPKGRIAVCGMISQYNLEQPEGVRNLMALIVKQVRMEGFMVFSYYHLYGKFLETVLPYIKQGKITYVEDVVDGLDNAPAALIGLYSGRNVGKQVVVVSRE

SEQ ID NO: 63 - protein, 678 aa, Eubacterium ramulus
MAEKNQYFPHLFEPLKVGSKTIKNRIEAAPALFAFEHYIELNPDPFGYTTPVPERAFRMLEAKAKGGAGIVCLGELSPNHEYDKRFPFEPYLDFTSRSDKQFEIMKETAEMIKSYGAFPMGELLSCGEIKTNIGDGINPKGPSEKDLPDGSHVEAFTKEEILSCYQDYVTACKWFQAAGWEGIMIHCGHGWLPAQFLSPQYNKRTDEYGGSFENRARFTVDLLKTVREAMGPDFVIEIRVSSSEHLPGGLELEDAVNYCKLCEPYIDMIHVSCGHYLSSSRSWEFTTAYAPHGPNIEPAAVIKQNVSIPVAAVGGINSPEQAEEAIASGKIDMVSMGRQFFADPAFPNKAKEGHADEIRRCLRCGRCYPGPSGEHETEIWTVKFPPLDSCTINPYDVWPASHHKVLPDRMPKPEASRKVLVVGGGCGGLQTAITASDRGHQVILCEKSGVLGGLINFTDHTDHKVDIRNFKDLLIRDVEKRPIEVRLNCEVTPELIREIAPEAVVLAVGSDDLILPIEGIENAVTAMDVYSNDFAGLGKSTIVLGGGLVGCEAAADYIDHGVETTIVEMKGALMPETTGLYRTAVHDFIDKNGGKYEVNAKVVKVGKDFVVAEQDGKEITIKADSVVNAMGRRAHATEALETAIKEAGIPVWKIGDCVRARQIGDAVREGWTAAMEII

SEQ ID NO: 64 - protein, 349 aa, Malus domestica
MAASTEGVISNKQVILKDYVTGFPKESDMQLTTATTKLKLPEGSKGVLVKNLYLSCDPYMRSRMTKREPGASYVDSFDAGSPIVGYGVAKVLESGDPKFKKGDLIWGMTGWEEYSVITSTESLFKIQHIDVPLSYYTGILGMPGMTAYAGFYEICNPKKGETVFVSAASGAVGQLVGQFAKLLGCYVVGSAGSKEKVDLLKNKFGFDNAFNYKEEPDLDAALKRYFPEGIDIYFENVGGKMLDAVLPNMRVHGRIAVCGLISQYNIDEPEGCRNLMYLIIKQVRMQGFLVFSYYHLYEKFLEMVLPAIKEGKLTYVEDVVEGLESAPAALIGLYAGRNVGKQVVVVSRE

SEQ ID NO: 65 - protein, 310 aa, Arabidopsis thaliana
MKVTVVSRSGREVLKAPLDLPDSATVADLQEAFHKRAKKFYPSRQRLTLPVTPGSKDKPVVLNSKKSLKEYCDGNNNSLTVVFKDLGAQVSYRTLFFFEYLGPLLIYPVFYYFPVYKFLGYGEDCVIHPVQTYAMYYWCFHYFKRILETFFVHRFSHATSPIGNVFRNCAYYWSFGAYIAYYVNHPLYTPVSDLQMKIGFGFGLVCQVANFYCHILLKNLRDPSGAGGYQIPRGFLFNIVTCANYTTEIYQWLGFNIATQTIAGYVFLAVAALIMTNWALGKHSRLRKIFDGKDGKPKYPRRWVILPPFL

SEQ ID NO: 66 - protein, 310 aa, Gossypium hirsutum
MKVTLVSRSGREFIKGGLELNDSATVADLQEAIHKRTKKFYPSRQRLTLPVPSGSRERPVILNYKKSLKDYCDGNENTLTIVFKDLGPQVSYRTLFFFEYLGPLILYPVFYYFPVYKYFGYEEKRVIHPVQTYALYYWCFHYFKRIMETFFIHRFSHATSPLSNVFRNCAYYWTFGSYIAYYVNHPLYTPVSDLQMKIGFGFGIVCQLANFYCHIILKNLRSPDGSGGYQIPRGFLFNIVTCANYTTEIYQWLGFNIATQTVAGYVFLVVATSIMTNWALAKHRRLKKLFDGKDGRPKYPRRWVILPPFL

SEQ ID NO: 67 - protein, 310 aa, Malus domestica
MKVTVVSRSGREVVKGGLELSDSATVADLQDAIHKRTKKFYPARQRLTLPVQPGSKERPVVLSYKKSLQDYISGNSDNLTVVFKDLGPQVSYRTLFFFEYLGPLILYPIFYYFPVYDYLGFKGDRVIHPVQTYALYYWCFHYFKRIMETFFVHRFSHATSPLSNVFRNCAYYWSFGAFIAYYLNHPLYTPVSDLQMKIGFGIGIICQISNFYCHILLRNLRSPDGNGGYQIPRGFLFNIVTCANYTTEIYQWLGFNIATQTVAGYIFLIVAASIMTNWALAKHRRLKKIFDGKDGRPKYPRRWVILPPFL

SEQ ID NO: 68 - DNA, 1200 bp, Hordeum vulgare
atggctgcagtaagattgaaagaagttagaatggcacagagggctgaaggtttagctacagttttagcaatcggtactgccgttccagctaattgtgtttatcaagctacctatccagattattattttagggttactaaaagtgagcacttggcagatttaaaggagaagtttcaaagaatgtgtgacaaatcaatgattagaaagagacacatgcacttgaccgaggaaatattgatcaagaacccaaagatctgtgcacacatggagacctcattggatgctagacacgccatcgcattagttgaagttcccaaattgggccaaggtgcagctgagaaggccattaaggagtggggccaacccttgtctaagattactcatttggtattttgcacaacatccggcgttgacatgcccggtgctgattaccaattaacaaagttgttaggtttgtcccctacagtcaaaaggttaatgatgtaccaacaaggttgctttggtggtgcaactgttttgagattggcaaaagatatcgctgaaaataatagaggtgccagagtgttagtcgtttgttccgagataactgctatgaccttcagaggtccatgcaagagtcatttagattccttggtaggtcatgccttgttcggtgatggtgccgctgctgcaattataggcgctgacccagaccaattagacgaacaaccagttttccagttggtatcagcttctcagactatattaccagaatcagaaggtgccatagatggccatttaacagaagctggtttaactatacatttattaaaagatgttcctggtttaatttcagagaacattgaacaggctttggaggatgcctttgaacctttaggtattcataactggaattcaattttctggattgcacatcctggtggccctgccattttagacagagttgaagatagagtaggattggataagaagagaatgagggcttctagggaagtgttatctgaatacggaaatatgtctagtgcctctgtgttgtttgtgttagatgtcatgaggaaaagttctgctaaagacggattggcaaccacaggagaaggaaaagattggggagtgttgtttggattcggaccaggcttgactgtagaaaccttagtgttgcatagtgtcccagtccctgtccctactgcagcttctgcatga

SEQ ID NO: 69 - DNA, 1200 bp, Hordeum vulgare
atggctgcagtaagattgaaagaagttagaatggcacagagggctgaaggtttagctacagttttagcaatcggtactgccgttccagctaattgtgtttatcaagctacctatccagattattattttagggttactaaaagtgagcacttggcagatttaaaggagaagtttcaaagaatgtgtgacaaatcaatgattagaaagagacacatgcacttgaccgaggaaatattgatcaagaacccaaagatctgtgcacacatggagacctcattggatgctagacacgccatcgcattagttgaagttcccaaattgggccaaggtgcagctgagaaggccattaaggagtggggccaacccttgtctaagattactcatttggtattttgcacaacatccggcgttgacatgcccggtgctgattaccaattaacaaagttgttaggtttgtcccctacagtcaaaaggttaatgatgtaccaacaaggttgctttggtggtgcaactgttttgagattggcaaaagatatcgctgaaaataatagaggtgccagagtgttagtcgtttgttccgagataactgctatgaccttcagaggtccatgcaagagtcatttagattccttggtaggtcatgccttgttcggtgatggtgccgctgctgcaattataggcgctgacccagaccaattagacgaacaaccagttttccagttggtatcagcttctcagactatattaccagaatcagaaggtgccatagatggccatttaacagaagctggtttaacttttcatttattaaaagatgttcctggtttaatttcagagaacattgaacaggctttggaggatgcctttgaacctttaggtattcataactggaattcaattttctggattgcacatcctggtggccctgccattttagacagagttgaagatagagtaggattggataagaagagaatgagggcttctagggaagtgttatctgaatacggaaatatgtctagtgcctctgtgttgtttgtgttagatgtcatgaggaaaagttctgctaaagacggattggcaaccacaggagaaggaaaagattggggagtgttgtttggattcggaccaggcttgactgtagaaaccttagtgttgcatagtgtcccagtccctgtccctactgcagcttctgcatga

SEQ ID NO: 70 - DNA, 1200 bp, Hordeum vulgare
atggctgcagtaagattgaaagaagttagaatggcacagagggctgaaggtttagctacagttttagcaatcggtactgccgttccagctaattgtgtttatcaagctacctatccagattattattttagggttactaaaagtgagcacttggcagatttaaaggagaagtttcaaagaatgtgtgacaaatcaatgattagaaagagacacatgcacttgaccgaggaaatattgatcaagaacccaaagatctgtgcacacatggagacctcattggatgctagacacgccatcgcattagttgaagttcccaaattgggccaaggtgcagctgagaaggccattaaggagtggggccaacccttgtctaagattactcatttggtattttgcacaacatccggcgttgacatgcccggtgctgattaccaattaacaaagttgttaggtttgtcccctacagtcaaaaggttaatgatgtaccaacaaggttgctttggtggtgcaactgttttgagattggcaaaagatatcgctgaaaataatagaggtgccagagtgttagtcgtttgttccgagataactgctatggccttcagaggtccatgcaagagtcatttagattccttggtaggtcatgccttgttcggtgatggtgccgctgctgcaattataggcgctgacccagaccaattagacgaacaaccagttttccagttggtatcagcttctcagactatattaccagaatcagaaggtgccatagatggccatttaacagaagctggtttaacttttcatttattaaaagatgttcctggtttaatttcagagaacattgaacaggctttggaggatgcctttgaacctttaggtattcataactggaattcaattttctggattgcacatcctggtggccctgccattttagacagagttgaagatagagtaggattggataagaagagaatgagggcttctagggaagtgttatctgaatacggaaatatgtctagtgcctctgtgttgtttgtgttagatgtcatgaggaaaagttctgctaaagacggattggcaaccacaggagaaggaaaagattggggagtgttgtttggattcggaccaggcttgactgtagaaaccttagtgttgcatagtgtcccagtccctgtccctactgcagcttctgcatga

SEQ ID NO: 71 - protein, 399 aa, Hordeum vulgare
MAAVRLKEVRMAQRAEGLATVLAIGTAVPANCVYQATYPDYYFRVTKSEHLADLKEKFQRMCDKSMIRKRHMHLTEEILIKNPKICAHMETSLDARHAIALVEVPKLGQGAAEKAIKEWGQPLSKITHLVFCTTSGVDMPGADYQLTKLLGLSPTVKRLMMYQQGCFGGATVLRLAKDIAENNRGARVLVVCSEITAMTFRGPCKSHLDSLVGHALFGDGAAAAIIGADPDQLDEQPVFQLVSASQTILPESEGAIDGHLTEAGLTIHLLKDVPGLISENIEQALEDAFEPLGIHNWNSIFWIAHPGGPAILDRVEDRVGLDKKRMRASREVLSEYGNMSSASVLFVLDVMRKSSAKDGLATTGEGKDWGVLFGFGPGLTVETLVLHSVPVPVPTAASA

SEQ ID NO: 72 - protein, 399 aa, Hordeum vulgare
MAAVRLKEVRMAQRAEGLATVLAIGTAVPANCVYQATYPDYYFRVTKSEHLADLKEKFQRMCDKSMIRKRHMHLTEEILIKNPKICAHMETSLDARHAIALVEVPKLGQGAAEKAIKEWGQPLSKITHLVFCTTSGVDMPGADYQLTKLLGLSPTVKRLMMYQQGCFGGATVLRLAKDIAENNRGARVLVVCSEITAMAFRGPCKSHLDSLVGHALFGDGAAAAIIGADPDQLDEQPVFQLVSASQTILPESEGAIDGHLTEAGLTFHLLKDVPGLISENIEQALEDAFEPLGIHNWNSIFWIAHPGGPAILDRVEDRVGLDKKRMRASREVLSEYGNMSSASVLFVLDVMRKSSAKDGLATTGEGKDWGVLFGFGPGLTVETLVLHSVPVPVPTAASA

SEQ ID NO: 73 - protein, 399 aa, Hordeum vulgare
MAAVRLKEVRMAQRAEGLATVLAIGTAVPANCVYQATYPDYYFRVTKSEHLADLKEKFQRMCDKSMIRKRHMHLTEEILIKNPKICAHMETSLDARHAIALVEVPKLGQGAAEKAIKEWGQPLSKITHLVFCTTSGVDMPGADYQLTKLLGLSPTVKRLMMYQQGCFGGATVLRLAKDIAENNRGARVLVVCSEITAMTFRGPCKSHLDSLVGHALFGDGAAAAIIGADPDQLDEQPVFQLVSASQTILPESEGAIDGHLTEAGLTFHLLKDVPGLISENIEQALEDAFEPLGIHNWNSIFWIAHPGGPAILDRVEDRVGLDKKRMRASREVLSEYGNMSSASVLFVLDVMRKSSAKDGLATTGEGKDWGVLFGFGPGLTVETLVLHSVPVPVPTAASA

SEQ ID NO: 74 - DNA, 28 bp, Artificial Sequence
  Forward Primer for restriction enyzme-based cloning
acaaaaagcttaaaatggctgcagtaag

SEQ ID NO: 75 - DNA, 16 bp, Artificial Sequence
  Reverse Primer for restriction enyzme-based cloning
acgtgccgcggtcatg

SEQ ID NO: 76 - DNA, 31 bp, Artificial Sequence
  Reverse Primer
atggacctctgaaggtcatagcagttatctc

SEQ ID NO: 77 - DNA, 31 bp, Artificial Sequence
  Forward primer
gagataactgctatgaccttcagaggtccat

SEQ ID NO: 78 - DNA, 38 bp, Artificial Sequence
  Reverse primer
acatcttttaataaatgaaaagttaaaccagcttctgt

SEQ ID NO: 79 - DNA, 38 bp, Artificial Sequence
  Forward primer
acagaagctggtttaacttttcatttattaaaagatgt

SEQ ID NO: 80 - DNA, 669 bp, Citrus sinensis
atgaatccatctccatctgttactgaattgcaagtagagaacgtcacctttaccccaagtgttcagcctccaggtagtactaaaagccatttcttaggaggcgctggtgaaagaggactagagattgaaggcaagtttgtgaaattcacagcaataggtgtatatcttgaagatgacgccgtccctttgttagctggtaagtggaaaggaaagaccgcagaggaactaactgaatctgtggagtttttcagggatgttgtaacaggcccatttgaaaaattcatgaaggtcaccatgatccttcctttgactggtgcccaatactcagaaaaagttgctgagaattgtattgcaatatggaagtttttcggaatctatacagacgccgaagctaaagcaattgagaagtttaccgaagtgttcaaagatgaaatatttccacctggttccagtatcctttttactcagagcccaggctctttgacaatttcattctccaaggacggtagtattcctaaagatggagttgctgtaatagagtctaacttactaagcgaagccgtccttgaatcaatgatcggtaaaaatggcgtgtccccagcagctaagaaaagtttggccgagagattatctgcactattgaacgttacttcagataagatgaaatga

SEQ ID NO: 81 - DNA, 726 bp, Petunia hybrida
atgtctccaccagtttctgttacaaaaatgcaagtcgaaaattatgcttttgcaccaacagtgaaccctgccggttccaccaatactttgttcttagctggagcaggccatagaggtctagagattgaaggaaagtttgtgaaattcacagccataggcgtataccttgaggaaagtgctatcccatttttggcagaaaagtggaaaggtaagacccctcaggagttaactgatagcgtcgagttctttagggacgtggttacaggtccattcgaaaagtttaccagagtaactatgattctacctcttacaggaaagcaatattctgagaaagtcgccgaaaactgtgttgctcactggaagggcataggtacctacactgatgacgaaggaagggcaatcgagaaattcttggatgtgtttagatcagaaacattcccacctggtgcttccattatgtttactcagagtccattaggcttgttaaccatcagctttgccaaggacgattcagttaccggtactgcaaatgctgtaatcgagaacaaacaactatcagaagccgtccttgaatccattattggaaagcatggtgtgagtcctgcagccaaatgctctgttgccgagagagtagcagaattgttaaaaaagagctatgctgaagaggcctcagtgttcggcaaaccagaaaccgaaaagtccacaatacctgttatcggtgtgtag

SEQ ID NO: 82 - DNA, 663 bp, Petunia hybrida
atgtctccatctgtttctgttactaaagtccaagtggaaaattatgtctttcctccaacagtgaagcctccagctagtaccaaaactttgttcttaggtggagcaggccatagaggtctagatgttgagggaaagtttgtgaaattcacagttattggcgtataccttgaagagagcgccgtccagtttttggctcctaagtggaaaggtaagtctgcagaagaattaatacactcagttgacttctttagggatatcgtgaccggtccattcgagaagtttactagagttaggttcattctacctcttacaggaaagcaattttccgaaaaagtagccgaaaactgtgtcgctcattggaaggcaaccggcacttatagtgacgccggtagcagagctatagagaaattcttgaatgtggttaagtctgaaacatttttaccaggagcatcaatcttgtttacccagtcccctttaggtagtctaactatttctttcacaaaagatgacagcatatccgaagctggcaacgccgtaatcgagaacaaacagtttagtgaggccgtccttgagactattattggtgaacacggagttagtccagctgccaagtgctctatagcagctagaatgtcagaattgttcaaaaacagcttattttga

SEQ ID NO: 83 - DNA, 672 bp, Pisum sativum
atgtgttgttctattttgcatcacagaaatccaaggagggaacatgagtttcctgctgttgtaacttcaccagtcacagaaaaccacatattcttaggtggagcaggcgagagaggtctaaccatcaatggaacttttatcaaattcacatgtataggcgtgtatcttgaagataaggccgacaaatccttggctaccaagtgggaaggcaaattagaggaactactagaaacattggatttttacagagacatcattagtggccctttcgagaagttaataagaaggagcaaaatcaaggaattgtccggtccagaatattcaagaaaagtcatggagaactgcgttgcacacttaaagtccgtaggcacatacggtgatgccgaagtggaggctattcaaaatctacagaaacttagtagaatgttgatttttcacttagttctattgaagaagaacaggcaaagccctgatggaatattaggtctttcttcatccaaagatatcagtattccagaaaaggaggatgcaataatcgagaataaggccgcttctagcgcagtattggagactatgattggcgaacatgctgtctctccagacttaaaaagatgtctagccgcaaggcttccagctttgttaaacgaaggtactttcaaaataggaaattga

SEQ ID NO: 84 - DNA, 675 bp, Pueraria Montana var. lobata
atggctgctgctgctgctgttgctactatttctgccgtacaagtcgaatttttggagttcccagcagtggttacaagccctgcctccggtagaacctattttttaggaggcgctggtgaaaggggactaactatagagggcaaattcatcaagtttacaggtattggtgtataccttgaagataaagcagtcagtagtttggctgccaagtggaaaggaaagccatctgaagagttagtggaaaccctagacttctatagagatataatctcaggcccttttgaaaaacttattaggggttccaagatattgccattaagtggagttgagtacagcaaaaaggtaatggaaaattgtgtcgcacatatgaaatctgttggtacttatggcgacgctgaagccgcagctatcgagaagttcgccgaagcctttaaaaacgtgaatttccagcctggtgctacagttttttacagacaatcaccagatggagtattgggtttatccttcagtgaggacgtcaccattcctgataacgaagccgcagtgattgaaaataaggctgtttctgccgcagtactagagactatgataggcgaacacgctgtcagcccagatcttaaaagatcactagcatccaggcttcctgccgttctaagtcatggtatcattgtgtga

SEQ ID NO: 85 - DNA, 702 bp, Oryza sativa subsp. japonica
atggctgctgtctctgaagttgaagttgacggtgtcgttttccctccagttgctagaccaccaggctctggtcatgctcacttcttggctggtgctggtgtccgtggtgttgaaatcgctggtaatttcatcaagttcaccgctattggcgtctacctagaagaaggtgccgccgttccagctttggctaagaagtgggccggtaagtctgctgatgagttggctgctgatgctgcctttttccgtgacgttgttaccggtgacttcgaaaaattcaccagagtcaccatgatcttgccactaaccggtgagcagtattccgacaaggtcaccgaaaactgtgttgctgcttggaaggccgctggcgtttatactgacgccgaaggtgctgctgctgataaattcaaggaagcctttaaaccacattccttcccaccaggtgcttctatcttgttcactcattctccaccaggtgtcttaaccgttgcctttagcaaagactcctccgtcccagaaggcgctgttgctgctgctgctatcgaaaacagggctttgtgcgaagctgtcctagactccattatcggtgagcatggtgtttctccagctgccaaaagatccatcgctgctcgtgtctctcaattgttgaaagctgaatccaccggcgacgtcgctgctgctgaaccagctcctgtctctgcttaa

SEQ ID NO: 86 - DNA, 669 bp, Medicago sativa
atggctgcttccattaccgctattaccgttgaaaatttggaatacccagctgttgttacttctccagttactggtaagtcttactttttgggtggtgctggtgaaagaggtttgactattgaaggtaacttcattaagttcaccgccatcggtgtttacttggaagatattgctgttgcttctttggctgctaaatggaagggtaaatcctccgaagaattattggaaaccttggacttctacagagacattatttctggtccattcgaaaagttgatcagaggttccaagatcagagaattgtctggtccagaatactccagaaaggttatggaaaattgcgttgcccatttgaagtctgttggtacttatggtgatgctgaagctgaagctatgcaaaaatttgctgaagcctttaagccagttaattttccaccaggtgcttccgttttttacagacaatctccagatggtatcttgggtttgtctttttcaccagatacctccatcccagaaaaagaagctgctttgattgaaaacaaggctgtttcttctgctgtcttggaaactatgattggtgaacatgctgtttccccagatttgaaaagatgtttagctgctagattgcctgccttgttgaatgaaggtgcttttaagattggtaactaa

SEQ ID NO: 87 - protein, 222 aa, Citrus sinensis
MNPSPSVTELQVENVTFTPSVQPPGSTKSHFLGGAGERGLEIEGKFVKFTAIGVYLEDDAVPLLAGKWKGKTAEELTESVEFFRDVVTGPFEKFMKVTMILPLTGAQYSEKVAENCIAIWKFFGIYTDAEAKAIEKFTEVFKDEIFPPGSSILFTQSPGSLTISFSKDGSIPKDGVAVIESNLLSEAVLESMIGKNGVSPAAKKSLAERLSALLNVTSDKMK

SEQ ID NO: 88 - protein, 241 aa, Petunia hybrida
MSPPVSVTKMQVENYAFAPTVNPAGSTNTLFLAGAGHRGLEIEGKFVKFTAIGVYLEESAIPFLAEKWKGKTPQELTDSVEFFRDVVTGPFEKFTRVTMILPLTGKQYSEKVAENCVAHWKGIGTYTDDEGRAIEKFLDVFRSETFPPGASIMFTQSPLGLLTISFAKDDSVTGTANAVIENKQLSEAVLESIIGKHGVSPAAKCSVAERVAELLKKSYAEEASVFGKPETEKSTIPVIGV

SEQ ID NO: 89 - protein, 220 aa, Petunia hybrida
MSPSVSVTKVQVENYVFPPTVKPPASTKTLFLGGAGHRGLDVEGKFVKFTVIGVYLEESAVQFLAPKWKGKSAEELIHSVDFFRDIVTGPFEKFTRVRFILPLTGKQFSEKVAENCVAHWKATGTYSDAGSRAIEKFLNVVKSETFLPGASILFTQSPLGSLTISFTKDDSISEAGNAVIENKQFSEAVLETIIGEHGVSPAAKCSIAARMSELFKNSLF

SEQ ID NO: 90 - protein, 223 aa, Pisum sativum
MCCSILHHRNPRREHEFPAVVTSPVTENHIFLGGAGERGLTINGTFIKFTCIGVYLEDKADKSLATKWEGKLEELLETLDFYRDIISGPFEKLIRRSKIKELSGPEYSRKVMENCVAHLKSVGTYGDAEVEAIQNLQKLSRMLIFHLVLLKKNRQSPDGILGLSSSKDISIPEKEDAIIENKAASSAVLETMIGEHAVSPDLKRCLAARLPALLNEGTFKIGN

SEQ ID NO: 91 - protein, 224 aa, Pueraria montana
MAAAAAVATISAVQVEFLEFPAVVTSPASGRTYFLGGAGERGLTIEGKFIKFTGIGVYLEDKAVSSLAAKWKGKPSEELVETLDFYRDIISGPFEKLIRGSKILPLSGVEYSKKVMENCVAHMKSVGTYGDAEAAAIEKFAEAFKNVNFQPGATVFYRQSPDGVLGLSFSEDVTIPDNEAAVIENKAVSAAVLETMIGEHAVSPDLKRSLASRLPAVLSHGIIV

SEQ ID NO: 92 - protein, 233 aa, Oryza sativa subsp. japonica
MAAVSEVEVDGVVFPPVARPPGSGHAHFLAGAGVRGVEIAGNFIKFTAIGVYLEEGAAVPALAKKWAGKSADELAADAAFFRDVVTGDFEKFTRVTMILPLTGEQYSDKVTENCVAAWKAAGVYTDAEGAAADKFKEAFKPHSFPPGASILFTHSPPGVLTVAFSKDSSVPEGAVAAAAIENRALCEAVLDSIIGEHGVSPAAKRSIAARVSQLLKAESTGDVAAAEPAPVSA

SEQ ID NO: 93 - protein, 222 aa, Medicago sativa
MAASITAITVENLEYPAVVTSPVTGKSYFLGGAGERGLTIEGNFIKFTAIGVYLEDIAVASLAAKWKGKSSEELLETLDFYRDIISGPFEKLIRGSKIRELSGPEYSRKVMENCVAHLKSVGTYGDAEAEAMQKFAEAFKPVNFPPGASVFYRQSPDGILGLSFSPDTSIPEKEAALIENKAVSSAVLETMIGEHAVSPDLKRCLAARLPALLNEGAFKIGN

SEQ ID NO: 94 - DNA, 948 bp, Arabidopsis thaliana
aagcttaaaatgaaggtcaccgtcgtttctagatcaggtagagaagttttgaaagccccattggatttgccagattctgctactgttgctgacttgcaagaagcctttcataagagagctaagaagttctacccatccagacaaagattgactttgccagttactccaggttctaaagataagccagttgtcttgaactccaagaagtccttgaaagaatactgtgacggtaacaacaactccttgactgttgtttttaaggatttgggtgcccaagtttcttacagaactttgttcttcttcgaatacttgggtcctttgttgatctacccagttttttactacttcccagtctacaagtttttgggttacggtgaagattgcgttatccatccagttcaaacttacgctatgtactactggtgtttccactacttcaagagaatcttggaaaccttcttcgtccacagattttctcatgctacttctccaattggtaacgttttcagaaactgtgcctattactggtctttcggtgcttatattgcttactacgttaaccacccattatacactccagtttcagacttgcaaatgaagattggttttggtttcggtttggtctgtcaagttgctaacttctactgccatatcttgttgaagaacttgagagatccatctggtgctggtggttatcaaattccaagaggttttttgttcaacatcgttacctgtgctaactacactaccgaaatctatcaatggttgggtttcaacattgccactcaaactattgctggttacgtttttttggctgttgccgctttgattatgactaattgggctttgggtaagcactccagattgagaaagattttcgatggtaaagacggtaagccaaagtatccaagaagatgggttattttgccaccattcttgtaaccgcgg

SEQ ID NO: 95 - DNA, 948 bp, Gossypium hirsutum
aagcttaaaatgaaggtcaccttggtcagtagatcaggtagagaattcattaagggtggtttggaattgaacgattctgctactgttgctgacttgcaagaagctattcataagagaactaagaagttctacccatccagacaaagattgactttgccagttccatctggttctagagaaagaccagttatcttgaactacaagaagtccttgaaggattactgtgacggtaacgaaaacactttgaccatcgtttttaaggacttgggtccacaagtttcttacagaactttgttcttcttcgaatatttgggtccattgatcttgtacccagttttctattacttcccagtctacaagtacttcggttacgaagaaaagagagttatccacccagttcaaacttatgccttgtactactggtgtttccactacttcaagagaattatggaaaccttcttcatccacagattctctcatgctacttctccattgtctaacgttttcagaaactgtgcttactactggactttcggttcttatattgcctactacgttaaccacccattatacactccagtttcagacttgcaaatgaagattggttttggtttcggtatcgtttgtcaattggctaacttctactgccacatcatcttgaagaatttgagatcaccagatggttctggtggttaccaaattccaagaggttttttgttcaacatcgttacctgtgctaactacactaccgaaatctatcaatggttgggtttcaacattgctactcaaacagttgctggttacgttttcttggttgttgctacctctattatgactaattgggccttggctaaacacagaagattgaagaaattattcgacggtaaggacggtagaccaaagtatccaagaagatgggttattttgccaccattcttgtaaccgcgg

SEQ ID NO: 96 - DNA, 933 bp, Malus domestica; identical to SEQ ID NO: 47

SEQ ID NO: 97 - DNA, 3702 bp, Arabidopsis thaliana
atggatttgttattgctggaaaagtcacttattgctgtatttgtggcagttattctagccacggttatttctaaattaagaggtaagaaactaaaactacctcctggtcccatccccataccaatttttggtaattggttgcaagtgggcgatgatttgaatcacagaaatttggtagactatgctaagaagttcggtgaccttttcttgcttagaatgggtcaaaggaatttggtagtggttagctcacctgatttgactaaggaggtcttattaacgcaaggcgttgagtttggctccagaactagaaatgttgtgtttgatattttcactggtaaaggtcaagatatggtttttacagtttacggtgagcactggagaaaaatgagaagaatcatgaccgtaccattctttactaacaaggttgttcaacaaaatagagaaggttgggagtttgaggcagcttccgtagtggaagacgtaaagaaaaatccagattcggccacaaagggtatagtactaagaaaaagactacaattgatgatgtacaacaatatgttcagaattatgtttgacagaagatttgaaagtgaagatgaccctttgttcctgagacttaaggctttgaatggtgaaagatcgagattggctcaaagtttcgaatataattacggtgactttattccaatcttaagaccatttttgagaggctatttgaaaatttgccaagacgtcaaggataggaggatcgctcttttcaagaagtactttgtggacgagagaaagcaaatagcttcttccaagcccacaggttcggaaggtttaaaatgtgcaattgatcatattttagaagctgaacaaaaaggtgaaattaacgaagataatgttttgtacattgtagaaaatatcaatgtggctgcaatagaaacaaccttatggtcaatagaatggggtattgctgaattggtgaatcacccagaaatacaatctaaactgagaaacgagctagataccgttttaggtccaggtgtccaagttacagaacctgatttgcataagttaccctacttgcaagctgtggttaaagaaaccttgagattgagaatggctattcctcttctagttcctcatatgaacctacatgatgctaaactggccggttatgatattccagcagaaagtaagattttagtaaatgcatggtggttggccaacaatccaaacagttggaaaaagcctgaagaattcagacctgaaagattcttcgaagaggaatctcatgttgaagccaacggaaatgacttcagatatgtaccttttggcgttggcagaagatcgtgtccaggaataatactagccttaccaatattgggtatcacaattggtaggatggttcaaaattttgagttgctaccaccacccggacaatcgaaagtcgatacttcagagaaaggaggacaattctcattgcatattttgaatcattccattatagtcatgaaacccagaaattgtagcgctgaagctgcagcaaaagaagctgcagcuaaagaagctgcagcaaaagcttccagtagctcttcctcctcaacctcgatgatcgacttaatggctgctattataaaaggagaaccagttatagttagtgaccctgctaacgcaagcgcttacgaatccgttgcagccgagttgtcaagtatgcttatagaaaatagacagtttgctatgattgtaacgaccagcatcgccgttttaattggttgcatcgtgatgttggtgtggaggaggagcggttcgggcaattcaaagagggttgaaccactaaagccattagttatcaaacctagagaagaggaaattgacgatggaaggaagaaagtcactatattcttcggcacccaaacaggtacagctgaaggttttgctaaggctctaggagaagaagcaaaagctagatatgaaaagacgagattcaaaattgtcgatctggatgactatgccgccgatgatgacgaatacgaagaaaaattgaagaaagaagatgtcgcatttttcttccttgccacctacggcgacggtgaaccaacagataatgccgcaaggttttacaagtggtttactgaaggtaatgacagaggagaatggctgaagaatttgaaatatggtgtgttcggccttggtaacagacagtacgagcattttaataaggtcgctaaggttgtagatgatatacttgttgaacaaggtgctcaaaggttagtgcaggtgggcttgggtgacgatgatcaatgtattgaagatgactttactgcttggagagaagccttgtggcctgaattagatactatccttagagaagaaggtgacactgctgttgctaccccctacactgcagcagtcctagaatatagagtctcaatccatgattcagaagacgccaaattcaatgatattaacatggccaacggtaacggttacaccgtttttgacgcacaacatccatacaaagctaatgttgctgttaaaagggaacttcacaccccagaaagtgacaggtcatgtatacatttggaatttgatatcgctggtagtggtttgacttacgaaacaggtgaccatgtcggagtactttgcgataatttgtcagaaactgttgatgaagctttgaggttattggatatgtcaccagatacttacttctcattgcatgcagaaaaagaagacggaactccaatatcaagctcgcttccccctccattccctccctgtaacttaagaacagccctaactagatatgcttgtttactgtcttctccaaagaaaagtgctttggttgcattggcagcccacgcatccgatcctaccgaagctgagagattaaagcatttggcttcaccagccggtaaagatgaatacagtaagtgggtagtggagagccaaagatcgcttttagaagtgatggctgagtttccaagtgctaaacctcctctgggtgtatttttcgctggtgtggccccaagattgcagcctagattttattccatatcctcatctccaaaaattgccgaaaccagaattcacgtgacatgtgctctggtctacgaaaagatgccaacaggtaggattcacaagggtgtctgttctacctggatgaaaaatgctgtaccctatgaaaaatccgaaaattgttctagtgcaccaattttcgtaagacaatctaatttcaagttaccaagcgattctaaagtacccattattatgatcggtccaggtactggtttggccccattcagaggcttcttgcaagaaagattggctttagtggagagtggagttgaattgggtccttcagttttattctttggttgtagaaacagaagaatggactttatctacgaagaagaattgcagagatttgttgaaagtggtgcattggccgaattgagtgttgcattcagcagggaaggtccaaccaaagaatacgttcaacacaagatgatggacaaggcttctgatatctggaatatgatttcccaaggtgcttatttgtatgtttgtggtgacgctaaaggaatggctagagatgttcatagatcactgcatacaatcgcacaagaacaaggtagcatggattcaacaaaagcagagggctttgtaaagaatcttcagacaagcggtagatatctgagagatgtatggtaa

SEQ ID NO: 98 - DNA, 2178 bp, Arabidopsis thaliana
atggagattaacggggcacacaagagcaacggaggaggagtggacgctatgttatgcggcggagacatcaagacaaagaacatggtgatcaacgcggaggatcctctcaactggggagctgcagcggagcaaatgaaaggtagccatttggatgaagtgaagagaatggttgctgagtttaggaagccagttgtgaatcttggtggtgagactctgaccattggacaagtggctgcgatctcaactattggtaacagtgtgaaggtggagctatcggagacagctagagccggtgtgaatgctagtagtgattgggttatggagagtatgaacaaaggcactgatagttatggtgttactactggttttggtgctacttctcatcggagaaccaaaaacggtgtcgcacttcagaaggaacttattagattccttaacgccggaatattcggaagcacgaaagaaacaagccacacattgccacactccgccacaagagccgccatgcttgtacgaatcaacactctcctccaaggattttccggtatccgatttgagattctcgaagcaattaccagtttcctcaacaacaacatcactccatctctccccctccgtggtacaatcaccgcctccggagatctcgttcctctctcctacatcgccggacttctcaccggtcgtcccaattccaaagctactggtcccaacggtgaagctttaacagcagaggaagctttcaaattagcaggaatcagctccggattctttgatctccagcctaaggaaggtctcgcgctagtcaatggcacggcggttggatctggaatggcgtcaatggtgttattcgaaacgaatgttctctctgttttggctgagattttgtcggcggttttcgcagaggtgatgagtggtaagcctgagttcaccgatcatctcactcacagacttaaacatcatcccggtcaaatcgaagcggcggcgataatggagcatatcctcgacggaagctcgtacatgaaattagctcagaagcttcacgagatggatccgttacagaaacctaaacaagatcgttacgctcttcgtacttctcctcaatggttaggtcctcaaatcgaagtgatccgttacgcaacgaaatcgatcgagcgtgagattaactccgtcaacgataatccgttgatcgatgtttcgaggaacaaggcgattcacggtggtaacttccaaggaacaccaatcggagtttcaatggataacacgagattggcgatagcagcgattggtaaactcatgtttgctcaattctcagagcttgtgaatgatttctacaacaatggtttaccctcgaatctaaccgcttcgaggaatccaagtttggattatggattcaagggagctgagattgcaatggcttcttattgttcagagcttcaatacttagctaatcctgtgactagccatgttcaatcagcagagcaacataaccaagatgtcaactctttgggactaatctcgtctcgcaaaacttctgaagctgttgatattctcaagcttatgtcaacaacgttcctcgttgcgatttgtcaagctgtggatttgagacatttggaggagaatttgagacagactgtgaagaacactgtctctcaagtggcgaagaaagttcttactactggagtcaatggtgagcttcatccttctcgcttctgcgaaaaggatttactcaaagttgtagaccgtgaacaagtctacacatacgcggatgatccttgtagcgcaacgtacccgttgattcagaagctgagacaagttattgttgaccatgctttgatcaatggtgagagtgagaagaatgcagtgacttcaatcttccataagattggagctttcgaggaggagcttaaggcagtgctaccgaaagaagtggaagcagcaagagcagcctacgataacggaacatcggctatcccgaacaggatcaaggaatgtaggtcgtatccattgtatagattcgtgagggaagagcttggaacagagcttttgaccggagagaaagtgacgtcgcctggagaagagttcgacaaggttttcacggcgatttgtgaaggtaaaatcattgatccgatgatggaatgtctcaacgagtggaacggagctcccattccaatatgttaa

SEQ ID NO: 99 - DNA, 2154 bp, Arabidopsis thaliana
atggatcaaatcgaagctatgttgtgtggtggtggtgaaaaaacaaaagttgctgttactactaagaccttggctgatccattgaattggggtttggctgctgatcaaatgaagggttctcatttggatgaagtcaagaagatggtcgaagaatacagaagaccagttgttaatttgggtggtgaaactttgactattggtcaagttgctgctatttctactgttggtggttctgttaaggttgaattggctgaaacttcaagagctggtgttaaggcttcttctgattgggttatggaatctatgaacaagggtactgattcttacggtgttactacaggttttggtgctacttctcatagaagaactaagaatggtactgccttgcaaaccgaattgatcagatttttgaacgccggtattttcggtaacaccaaagaaacttgtcataccttgccacaatctgctactagagctgctatgttggttagagttaacactttgttgcaaggttactccggtatcagattcgaaattttggaagctatcacctccttgttgaaccataacatttctccatctttgccattgagaggtactattactgcttctggtgatttggttccattgtcttatattgctggtttgttgactggtagaccaaactctaaagctactggtccagatggtgaatcattgactgctaaagaagcctttgaaaaggctggtatctctactggttttttcgacttgcaacctaaagaaggtttggctttggttaatggtacagctgttggttctggtatggcttctatggttttgtttgaagctaacgttcaagctgttttggccgaagttttgtctgctatttttgctgaagttatgtccggtaagccagaattcactgatcatttgacccatagattgaaacatcacccaggtcaaattgaagctgctgcaattatggaacatatcttggatggttcctcttacatgaagttggctcaaaaagttcacgaaatggacccattgcaaaagccaaaacaagatagatacgctttgagaacttctccacaatggttgggtccacaaatagaagttattagacaagccaccaagtccatcgaaagagaaatcaattctgttaacgacaacccattgatcgacgtcagtagaaacaaagctattcatggtggtaacttccaaggtactccaattggtgtttctatggacaacactagattggctattgctgccattggtaaattgatgttcgctcaattctccgaattggtcaacgatttttacaacaacggtttgccttctaacttgaccgcttcttctaatccatcattggattacggttttaagggtgctgaaattgctatggcttcatactgttctgaattgcaatacttggctaacccagttacctctcatgttcaatctgctgaacaacacaatcaagacgttaactccttgggtttgatctcttccagaaaaacttctgaagccgttgacattttgaagttgatgtctactaccttcttggtcggtatttgtcaagcagttgatttgagacacttggaagaaaacttgagacaaaccgttaagaacaccgtttcccaagttgctaaaaaggttttgactaccggtattaacggtgaattgcatccatccagattctgcgaaaaagatttgttgaaggtcgttgacagagaacaagttttcacctatgttgatgatccatgttctgctacctatccattgatgcaaagattgagacaagtcatcgttgatcatgctttgtctaatggtgaaaccgaaaagaacgctgttacctccattttccaaaagattggtgctttcgaagaagaattgaaggccgttttgccaaaagaagttgaagcagctagagcagcttacggtaacggtactgctccaattccaaatagaatcaaagaatgcagatcctacccattatacagattcgttagagaagaattaggtactaagttgttgaccggtgaaaaggttgtttctccaggtgaagaattcgataaggttttcactgctatgtgcgaaggtaaattgatcgatccattgatggactgcttgaaagaatggaatggtgctcctattcctatctgctaa

SEQ ID NO: 100 - DNA, 2112 bp, Aspergillus niger
atgttggacaagcacatcccagacggtcacttagaaaccactagcgcccactggagggatttaaaccaagttgttcaaaacggtgaattatctattgacggttactccttgtccttggccgatgttgttgctgtcgctaagtatggttgccaaccaagattgactgacaagccagagactattgatgctattaacggttctgtcatcgccttggctgaatgtttaagggatggtcatcacatttacggtgttaacactggttttggtggttctgccgattccagaaccaaccagaccactactttgcaaagctccttgttgcaattgttgcaatccggtatcttaactgcttctgacactaccaatgaaggtttgcagttgaacttgcaaggtcaaagcagccattctatgccatctgagtgggttaaagctaccatgttggttcgttctaactctgtcgctagaggccattctgctgtcagcttgccagctatttccgccattttgagattgatcagagaagatatcgtcccagttattccattgagaggtactatctccgcttccggtgacttgatgccattggcttacgttgtcggtgccattgaaggttctccaggtatttacgttagagtcaaggatggttctgaacatcaagtcgttaccgctcaaaaggccctacaaactatcggtgctaagggtgttactttgggccctaaagagggtttaggtttggtcaatggtactgctgcttctggtgccttagctggtttggttttgtatgaggctcatcaattggccgtcttggctcaagctgtcaccgccttaactgtcgaagctattcaaggttctaccgaatcctttcacccttttatcgctcaagtccgtccacatgaaggtcagatcgaggctgctgaaaacatcctatctctattaaaaggtagcttgttggccagaggtagctctactacccaaaccagaaccggtctagtccaagacagatactccttgagaactgcttctcaatggatcggtcctcaattggaagatttattgttggccgacagacaggtccaagtcgaactaaattctaccagcgacaacccattaatcgatactggttctaaaactttctacactggtggtaacttccaagctaccagcattacctccgctatggaaaagactaggttggctttgcaaatgttcggtaagatgttattcgtccaatgtaatgaaatgatcgacccaaacttgaacaacggtctacctaccaacttggttgctgatgacccatccttgtccttcaccatgaaaggcgtcgatatcaacatggctgcttatatgtctgaattggcttacttggctaatccagtctcctcccacgttcaaactgctgaaatgcaaaaccaagccttgaactccttggctttcgttagcgctaggtatactatgaaagctgttgatatcgtctctatgatgggtgcttgtgctttgtatgtcgcttgtcaagccttagacttgagggtcttgcaattgcgtttcttccaaagagtccaaggtgtcgctaaagaaatcgctcacggtgcctttggtaaggccttggaacctttcgaaatcgaccaggttgctgatcacttgtctgaagctattcaaaactcctggccatctacctctaggttggacttgagagacagatgcaaaagggttgctgaaatgtttatcccagtcttgttcggtgctttgttgcaaattatcccacagaacagacaaacctctgatttattcaccgccatctctgcttgtaagatgatttccgtttttaagttggaaggcgtttacagagaagttttcgctgaattttgcacttcccaacctaccgctgactttttgggtaccggtactaaggaaatctacaccttcatcagacacgacttgagagtcccattccaccagggtttcgtcgaacatccatccgcctctcaaaccgacttaccagaaactatcaacggtagagttaaaaagaccgtcggtggttggatttctgtcgtttacgaagccttgagaaatggtaccttaagcggtactattttgaactccttccaacaataa

SEQ ID NO: 101 - DNA, 2151 bp, Rhodosporidium toruloides
atggctccatcattggattctatttctcattcttttgcaaacggtgttgcatctgcaaaacaagctgttaatggtgcatctactaatttggcagttgctggttctcatttaccaactacccaagttacacaagttgatattgttgaaaagatgttagcagcacctactgattctaccttggaattggatggttactctttaaatttaggtgatgttgtttctgcagctagaaagggtagaccagttagagttaaagattctgatgaaattagatctaaaattgataaatctgttgaatttttgagatctcaattatcaatgtcagtttatggtgttacaactggtttcggtggttcagctgatactagaactgaagatgcaatttctttacaaaaggcattgttggaacatcaattatgtggtgttttgccttcatcattcgattcttttagattaggtagaggtttagaaaactctttgccattagaagttgttagaggtgcaatgacaattagagttaattctttaacaagaggtcattctgctgttagattggttgttttagaagctttgactaactttttgaaccatggtattactccaattgttccattaagaggtacaatttctgcatctggtgatttgtctcctttgtcttatattgcagctgctatttcaggtcatccagattcaaaggttcatgttgttcatgaaggtaaggaaaagattttatatgcaagagaagctatggctttatttaatttagaaccagttgttttaggtcctaaggaaggtttaggtttagttaacggtacagctgtttcagcatctatggctaccttagctttgcatgatgctcatatgttatctttgttatctcaatcattaacagctatgactgttgaagctatggttggtcatgctggttcttttcatccattcttgcatgatgttaccagacctcatccaacacaaattgaagttgctggtaatattagaaagttgttagaaggttctagattcgcagttcatcatgaagaagaagttaaagttaaggatgatgaaggtattttgagacaagatagatacccattgagaacttcaccacaatggttgggtccattggtttctgatttgattcatgctcatgcagttttgaccattgaagcaggtcaatctacaacagataatccattgattgatgttgaaaacaaaacatcacatcatggtggtaattttcaagcagctgctgttgctaatacaatggaaaagacaagattaggtttggcacaaattggtaagttaaatttcacacaattaactgaaatgttgaatgcaggtatgaatagaggtttgccatcttgtttggcagctgaagatccttcattatcttatcattgtaaaggtttggatattgcagcagcagcttatacttcagaattaggtcatttagcaaatccagttactacacatgttcaaccagctgaaatggctaatcaagctgttaattctttagcattgatttcagctagaagaaccactgaatcaaacgatgttttgtcattattattagctactcatttatattgtgttttacaagctattgatttgagagcaattgaatttgaatttaaaaagcaatttggtccagctattgtttcattaattgatcaacattttggttctgcaatgactggttcaaatttgagagatgaattagttgaaaaggttaacaagaccttggctaaaagattagaacaaactaactcttacgatttggttccaagatggcatgatgctttttcttttgctgcaggtacagttgttgaagttttgtcatctacctcattgtctttggcagctgttaacgcttggaaagttgctgctgctgaatcagctatttcattaactagacaagttagagaaactttttggtctgctgcttcaacttcttcacctgctttgtcttacttgtctccaagaactcaaattttgtacgctttcgttagagaagaattgggtgttaaagctagaagaggtgatgttttcttaggtaagcaagaagttactattggttctaatgtttctaaaatttacgaagctattaaatcaggtagaattaataacgttttgttgaagatgttagcataa

SEQ ID NO: 102 - DNA, 1173 bp, Hypericum androsaemum
atggttacagtcgaagaagtgagaaaggctcaaagagccgagggaccagctactgtcatggcaattggtaccgctgtacctcctaactgtgtcgatcaagctacataccctgactattactttagaattacaaattcagaacacaaagccgaactgaaggaaaaatttcaaagaatgtgcgacaaatctcagatcaaaaagagatacatgtatttaaacgaggaggttctaaaagagaatccaaatatgtgcgcgtacatggcaccctcactggatgcaagacaagacatagtcgttgttgaagtaccaaagcttggtaaggaggccgccgttaaggctattaaggaatggggccaacctaaatctaaaattacacatttggtcttctgtacaaccagtggcgtggatatgcccggtgctgactaccaactaaccaagttgcttggtttaaggccctccgttaaaagattaatgatgtatcaacagggttgtttcgctggaggaacagttctaagattagctaaagatttagcagaaaacaacaaaggcgctagggtacttgtagtatgttcagaaatcactgctgtaacttttcgtggtccaaccgacactcatttagattccttagttggacaggctctatttggagatggggccgccgccatcattatcggttctgatccgatcccagaggtagagaaaccattgttcgaattggtttccgctgctcaaacaattctgcctgactccgaaggtgccatagacggtcacttgagagaggtcggattgacctttcatttattaaaggatgtgcccggtttgataagtaaaaacgtcgagaaatccttaactgaagcattcaaaccattagggatatccgattggaacagtttattctggatcgctcatccaggcggtccagccatcctagatcaagtagaagctaaattatcattaaaacctgaaaagttaagagcaacgagacatgtcttgtcagaatatggtaatatgtctagcgcgtgtgttcttttcatcttggatgaaatgcgtagaaaatctaaagaagacggtttgaagacgactggtgaaggtattgaatggggtgttttgttcggctttggtccgggtctaaccgtcgaaactgtggtattgcactccgttgccataaattaa

SEQ ID NO: 103 - DNA, 1170 bp, Hypericum androsaemum
gttaccgtagaagaggtacgtaaagctcagagagcagaggggcccgctaccgttatggccattggtaccgccgtgccgccaaactgcgttgatcaagctacttatcctgattactatttcagaattactaattctgaacataaggccgaattgaaagagaagtttcaaaggatgtgcgacaaatcacagataaagaagcgttatatgtacttgaacgaagaagtgttgaaggaaaatccaaatatgtgtgcctatatggctccttcattagatgccagacaagatattgttgtggttgaagttcccaagttgggcaaggaagcggcagtcaaagctattaaggaatggggacaaccaaaatcaaaaattacgcatttagtgttttgtaccacttctggcgtagatatgcctggtgccgactatcaattaacgaaattgcttggtttacgtccatcagtaaaaagattgatgatgtatcaacaaggttgctttgccggtggtacagttcttcgtcttgccaaggaccttgcagaaaacaataaaggggcaagggtgttggttgtatgttctgaaataacggccgtgacgtttagaggtcccactgatacccatttggattcattagtaggccaagctttatttggtgacggtgcagcagcaatcataatcggttccgatccgataccagaagtggaaaagcctttgtttgaattggttagcgcagcccaaaccatacttccagactctgaaggtgcaattgatggtcatttgagggaggtgggtctaacattccatcttttgaaggacgtgccgggacttatttctaagaatgtagaaaagtctttgactgaagcattcaaaccactgggaatttctgactggaattctttgttctggatcgctcacccaggtggccctgcgattctagatcaggtcgaggcaaaactttcactaaagcctgaaaaattgagggcgacgagacatgttttgtcagaatacggcaatatgtcatcagcttgcgtattgttcatattggatgaaatgagaagaaaatctaaagaggatggcctgaaaacgactggtgaaggtattgaatggggtgtcttgtttggtttcggtcctggcttgactgtcgagactgttgtgttgcatagtgttgctattaattga

SEQ ID NO: 104 - DNA, 1173 bp, Hypericum androsaemum
atggtgactgttgaagaagtaagaaaggctcaaagagctgaaggtcctgctactgttatggccatagggacagcggtcccaccaaactgtgttgatcaggcgacttatcctgattattatttcagaatcacgaattccgagcacaaagccgagctaaaagagaaatttcaaaggatgtgcgataaaagccagataaaaaagagatatatgtatctaaatgaagaagtcttaaaagagaacccgaacatgtgcgcttacatggcaccatccctagatgctagacaagatatcgtagtggttgaagttccaaagctgggtaaggaggcagcggtaaaagcaattaaggaatggggccaaccaaagtcaaagattactcacttagtattttgcactacttccggtgtagatatgcccggtgccgactatcaacttaccaaactacttggtttgcgtccaagcgttaaacgtctaatgatgtaccaacaaggatgctttgctggtggcaccgtgttaagattagcaaaagatctggccgagaataacaagggcgctagagttttagttgtatgttcagaaattacggctgtgactttcagaggccctacagacactcatcttgattcattagtgggccaagctttgttcggagacggagcagcagcaatcattatcggttcagatccaattccagaagtcgaaaaaccactgttcgaactagtttctgcagcccaaacaattttaccggattctgaaggcgctattgacggtcatttaagggaagtgggtttgactttccatttgttgaaagacgttccaggtctgatatccaaaaatgtggagaaatcattgaccgaagcatttaaaccattgggtatctctgattggaattcactattttggattgctcaccccggtggaccagcaatactggatcaagttgaagcgaaattgtcactgaagcctgaaaaattgagggctacgaggcatgtgttatccgaatacgggaatatgtctagcgcatgtgtgttgtttatacttgatgaaatgcgtaggaaatctaaggaagatggcttgaagactaccggtgaaggtattgaatggggtgtcttatttggatttggccctggtttgacagtggaaactgttgttcttcactcagtagctattaattaa

SEQ ID NO: 105 - protein, 1233 aa, Arabidopsis thaliana
MDLLLLEKSLIAVFVAVILATVISKLRGKKLKLPPGPIPIPIFGNWLQVGDDLNHRNLVDYAKKFGDLFLLRMGQRNLVVVSSPDLTKEVLLTQGVEFGSRTRNVVFDIFTGKGQDMVFTVYGEHWRKMRRIMTVPFFTNKVVQQNREGWEFEAASVVEDVKKNPDSATKGIVLRKRLQLMMYNNMFRIMFDRRFESEDDPLFLRLKALNGERSRLAQSFEYNYGDFIPILRPFLRGYLKICQDVKDRRIALFKKYFVDERKQIASSKPTGSEGLKCAIDHILEAEQKGEINEDNVLYIVENINVAAIETTLWSIEWGIAELVNHPEIQSKLRNELDTVLGPGVQVTEPDLHKLPYLQAVVKETLRLRMAIPLLVPHMNLHDAKLAGYDIPAESKILVNAWWLANNPNSWKKPEEFRPERFFEEESHVEANGNDFRYVPFGVGRRSCPGIILALPILGITIGRMVQNFELLPPPGQSKVDTSEKGGQFSLHILNHSIIVMKPRNCSAEAAAKEAAAKEAAAKASSSSSSSTSMIDLMAAIIKGEPVIVSDPANASAYESVAAELSSMLIENRQFAMIVTTSIAVLIGCIVMLVWRRSGSGNSKRVEPLKPLVIKPREEEIDDGRKKVTIFFGTQTGTAEGFAKALGEEAKARYEKTRFKIVDLDDYAADDDEYEEKLKKEDVAFFFLATYGDGEPTDNAARFYKWFTEGNDRGEWLKNLKYGVFGLGNRQYEHFNKVAKVVDDILVEQGAQRLVQVGLGDDDQCIEDDFTAWREALWPELDTILREEGDTAVATPYTAAVLEYRVSIHDSEDAKFNDINMANGNGYTVFDAQHPYKANVAVKRELHTPESDRSCIHLEFDIAGSGLTYETGDHVGVLCDNLSETVDEALRLLDMSPDTYFSLHAEKEDGTPISSSLPPPFPPCNLRTALTRYACLLSSPKKSALVALAAHASDPTEAERLKHLASPAGKDEYSKWVVESQRSLLEVMAEFPSAKPPLGVFFAGVAPRLQPRFYSISSSPKIAETRIHVTCALVYEKMPTGRIHKGVCSTWMKNAVPYEKSENCSSAPIFVRQSNFKLPSDSKVPIIMIGPGTGLAPFRGFLQERLALVESGVELGPSVLFFGCRNRRMDFIYEEELQRFVESGALAELSVAFSREGPTKEYVQHKMMDKASDIWNMISQGAYLYVCGDAKGMARDVHRSLHTIAQEQGSMDSTKAEGFVKNLQTSGRYLRDVW

SEQ ID NO: 106 - protein, 725 aa, Arabidopsis thaliana
MEINGAHKSNGGGVDAMLCGGDIKTKNMVINAEDPLNWGAAAEQMKGSHLDEVKRMVAEFRKPVVNLGGETLTIGQVAAISTIGNSVKVELSETARAGVNASSDWVMESMNKGTDSYGVTTGFGATSHRRTKNGVALQKELIRFLNAGIFGSTKETSHTLPHSATRAAMLVRINTLLQGFSGIRFEILEAITSFLNNNITPSLPLRGTITASGDLVPLSYIAGLLTGRPNSKATGPNGEALTAEEAFKLAGISSGFFDLQPKEGLALVNGTAVGSGMASMVLFETNVLSVLAEILSAVFAEVMSGKPEFTDHLTHRLKHHPGQIEAAAIMEHILDGSSYMKLAQKLHEMDPLQKPKQDRYALRTSPQWLGPQIEVIRYATKSIEREINSVNDNPLIDVSRNKAIHGGNFQGTPIGVSMDNTRLAIAAIGKLMFAQFSELVNDFYNNGLPSNLTASRNPSLDYGFKGAEIAMASYCSELQYLANPVTSHVQSAEQHNQDVNSLGLISSRKTSEAVDILKLMSTTFLVAICQAVDLRHLEENLRQTVKNTVSQVAKKVLTTGVNGELHPSRFCEKDLLKVVDREQVYTYADDPCSATYPLIQKLRQVIVDHALINGESEKNAVTSIFHKIGAFEEELKAVLPKEVEAARAAYDNGTSAIPNRIKECRSYPLYRFVREELGTELLTGEKVTSPGEEFDKVFTAICEGKIIDPMMECLNEWNGAPIPIC

SEQ ID NO: 107 - protein, 703 aa, Aspergillus niger
MLDKHIPDGHLETTSAHWRDLNQVVQNGELSIDGYSLSLADVVAVAKYGCQPRLTDKPETIDAINGSVIALAECLRDGHHIYGVNTGFGGSADSRTNQTTTLQSSLLQLLQSGILTASDTTNEGLQLNLQGQSSHSMPSEWVKATMLVRSNSVARGHSAVSLPAISAILRLIREDIVPVIPLRGTISASGDLMPLAYVVGAIEGSPGIYVRVKDGSEHQVVTAQKALQTIGAKGVTLGPKEGLGLVNGTAASGALAGLVLYEAHQLAVLAQAVTALTVEAIQGSTESFHPFIAQVRPHEGQIEAAENILSLLKGSLLARGSSTTQTRTGLVQDRYSLRTASQWIGPQLEDLLLADRQVQVELNSTSDNPLIDTGSKTFYTGGNFQATSITSAMEKTRLALQMFGKMLFVQCNEMIDPNLNNGLPTNLVADDPSLSFTMKGVDINMAAYMSELAYLANPVSSHVQTAEMQNQALNSLAFVSARYTMKAVDIVSMMGACALYVACQALDLRVLQLRFFQRVQGVAKEIAHGAFGKALEPFEIDQVADHLSEAIQNSWPSTSRLDLRDRCKRVAEMFIPVLFGALLQIIPQNRQTSDLFTAISACKMISVFKLEGVYREVFAEFCTSQPTADFLGTGTKEIYTFIRHDLRVPFHQGFVEHPSASQTDLPETINGRVKKTVGGWISVVYEALRNGTLSGTILNSFQQ

SEQ ID NO: 108 - protein, 716 aa, Rhodosporidium toruloides
MAPSLDSISHSFANGVASAKQAVNGASTNLAVAGSHLPTTQVTQVDIVEKMLAAPTDSTLELDGYSLNLGDVVSAARKGRPVRVKDSDEIRSKIDKSVEFLRSQLSMSVYGVTTGFGGSADTRTEDAISLQKALLEHQLCGVLPSSFDSFRLGRGLENSLPLEVVRGAMTIRVNSLTRGHSAVRLVVLEALTNFLNHGITPIVPLRGTISASGDLSPLSYIAAAISGHPDSKVHVVHEGKEKILYAREAMALFNLEPVVLGPKEGLGLVNGTAVSASMATLALHDAHMLSLLSQSLTAMTVEAMVGHAGSFHPFLHDVTRPHPTQIEVAGNIRKLLEGSRFAVHHEEEVKVKDDEGILRQDRYPLRTSPQWLGPLVSDLIHAHAVLTIEAGQSTTDNPLIDVENKTSHHGGNFQAAAVANTMEKTRLGLAQIGKLNFTQLTEMLNAGMNRGLPSCLAAEDPSLSYHCKGLDIAAAAYTSELGHLANPVTTHVQPAEMANQAVNSLALISARRTTESNDVLSLLLATHLYCVLQAIDLRAIEFEFKKQFGPAIVSLIDQHFGSAMTGSNLRDELVEKVNKTLAKRLEQTNSYDLVPRWHDAFSFAAGTVVEVLSSTSLSLAAVNAWKVAAAESAISLTRQVRETFWSAASTSSPALSYLSPRTQILYAFVREELGVKARRGDVFLGKQEVTIGSNVSKIYEAIKSGRINNVLLKMLA

SEQ ID NO: 109 - protein, 390 aa, Hypericum androsaemum; identical to SEQ ID NO: 49